European Patent Application EP 4 534 660 A1, published April 9, 2025. Title: Engineered Cas12f protein with expanded targetable range and uses thereof. Applicant: GenKOre Co., Ltd. The sequence listing filed with the application follows.

SEQUENCE LISTING (357 sequences)

SEQ ID NO: 1 - protein, 557 aa, unidentified
  source 1..557: note = CWCas12f
MGEKSSRRRRNGKSGAWTAAITSCVGGKMAKNTITKTLKLRIVRPYNSAEVEKIVADEKNNREKIALEKNKDKVKEACSKHLKVAAYCTTQVERNACLFCKARKLDDKFYQKLRGQFPDAVFWQEISEIFRQLQKQAAEIYNQSLIELYYEIFIKGKGIANASSVEHYLSDVCYTRAAELFKNAAIASGLRSKIKSNFRLKELKNMKSGLPTTKSDNFPIPLVKQKGGQYTGFEISNHNSDFIIKIPFGRWQVKKEIDKYRPWEKFDFEQVQKSPKPISLLLSTQRRKRNKGWSKDEGTEAEIKKVMNGDYQTSYIEVKRGSKIGEKSAWMLNLSIDVPKIDKGVDPSIIGGIDVGVKSPLVCAINNAFSRYSISDNDLFHFNKKMFARRRILLKKNRHKRAGHGAKNKLKPITILTEKSERFRKKLIERWACEIADFFIKNKVGTVQMENLESMKRKEDSYFNIRLRGFWPYAEMQNKIEFKLKQYGIEIRKVAPNNTSKTCSKCGHLNNYFNFEYRKKNKFPHFKCEKCNFKENADYNAALNISNPKLKSTKEEP

SEQ ID NO: 2 - protein, 555 aa, synthetic construct
  source 1..555: note = CWCas12f-v1
MEKRINKIRKKLSADNATKPVSRSGPMAKNTITKTLKLRIVRPYNSAEVEKIVADEKNNREKIALEKNKDKVKEACSKHLKVAAYCTTQVERNACLFCKARKLDDKFYQKLRGQFPDAVFWQEISEIFRQLQKQAAEIYNQSLIELYYEIFIKGKGIANASSVEHYLSDVCYTRAAELFKNAAIASGLRSKIKSNFRLKELKNMKSGLPTTKSDNFPIPLVKQKGGQYTGFEISNHNSDFIIKIPFGRWQVKKEIDKYRPWEKFDFEQVQKSPKPISLLLSTQRRKRNKGWSKDEGTEAEIKKVMNGDYQTSYIEVKRGSKIGEKSAWMLNLSIDVPKIDKGVDPSIIGGIDVGVKSPLVCAINNAFSRYSISDNDLFHFNKKMFARRRILLKKNRHKRAGHGAKNKLKPITILTEKSERFRKKLIERWACEIADFFIKNKVGTVQMENLESMKRKEDSYFNIRLRGFWPYAEMQNKIEFKLKQYGIEIRKVAPNNTSKTCSKCGHLNNYFNFEYRKKNKFPHFKCEKCNFKENADYNAALNISNPKLKSTKEEP

SEQ ID NO: 3 - protein, 557 aa, synthetic construct
  source 1..557: note = CWCas12f-v2
MAGGPGAGSAAPVSSTSSLPLAALNMRVMAKNTITKTLKLRIVRPYNSAEVEKIVADEKNNREKIALEKNKDKVKEACSKHLKVAAYCTTQVERNACLFCKARKLDDKFYQKLRGQFPDAVFWQEISEIFRQLQKQAAEIYNQSLIELYYEIFIKGKGIANASSVEHYLSDVCYTRAAELFKNAAIASGLRSKIKSNFRLKELKNMKSGLPTTKSDNFPIPLVKQKGGQYTGFEISNHNSDFIIKIPFGRWQVKKEIDKYRPWEKFDFEQVQKSPKPISLLLSTQRRKRNKGWSKDEGTEAEIKKVMNGDYQTSYIEVKRGSKIGEKSAWMLNLSIDVPKIDKGVDPSIIGGIDVGVKSPLVCAINNAFSRYSISDNDLFHFNKKMFARRRILLKKNRHKRAGHGAKNKLKPITILTEKSERFRKKLIERWACEIADFFIKNKVGTVQMENLESMKRKEDSYFNIRLRGFWPYAEMQNKIEFKLKQYGIEIRKVAPNNTSKTCSKCGHLNNYFNFEYRKKNKFPHFKCEKCNFKENADYNAALNISNPKLKSTKEEP

SEQ ID NO: 4 - protein, 555 aa, synthetic construct
  source 1..555: note = CWCas12f-v3
MAGGPGAGSAAPVSSTSSLPLAALNMMAKNTITKTLKLRIVRPYNSAEVEKIVADEKNNREKIALEKNKDKVKEACSKHLKVAAYCTTQVERNACLFCKARKLDDKFYQKLRGQFPDAVFWQEISEIFRQLQKQAAEIYNQSLIELYYEIFIKGKGIANASSVEHYLSDVCYTRAAELFKNAAIASGLRSKIKSNFRLKELKNMKSGLPTTKSDNFPIPLVKQKGGQYTGFEISNHNSDFIIKIPFGRWQVKKEIDKYRPWEKFDFEQVQKSPKPISLLLSTQRRKRNKGWSKDEGTEAEIKKVMNGDYQTSYIEVKRGSKIGEKSAWMLNLSIDVPKIDKGVDPSIIGGIDVGVKSPLVCAINNAFSRYSISDNDLFHFNKKMFARRRILLKKNRHKRAGHGAKNKLKPITILTEKSERFRKKLIERWACEIADFFIKNKVGTVQMENLESMKRKEDSYFNIRLRGFWPYAEMQNKIEFKLKQYGIEIRKVAPNNTSKTCSKCGHLNNYFNFEYRKKNKFPHFKCEKCNFKENADYNAALNISNPKLKSTKEEP

SEQ ID NO: 5 - protein, 529 aa, synthetic construct
  source 1..529: note = Un1Cas12f1
MAKNTITKTLKLRIVRPYNSAEVEKIVADEKNNREKIALEKNKDKVKEACSKHLKVAAYCTTQVERNACLFCKARKLDDKFYQKLRGQFPDAVFWQEISEIFRQLQKQAAEIYNQSLIELYYEIFIKGKGIANASSVEHYLSDVCYTRAAELFKNAAIASGLRSKIKSNFRLKELKNMKSGLPTTKSDNFPIPLVKQKGGQYTGFEISNHNSDFIIKIPFGRWQVKKEIDKYRPWEKFDFEQVQKSPKPISLLLSTQRRKRNKGWSKDEGTEAEIKKVMNGDYQTSYIEVKRGSKIGEKSAWMLNLSIDVPKIDKGVDPSIIGGIDVGVKSPLVCAINNAFSRYSISDNDLFHFNKKMFARRRILLKKNRHKRAGHGAKNKLKPITILTEKSERFRKKLIERWACEIADFFIKNKVGTVQMENLESMKRKEDSYFNIRLRGFWPYAEMQNKIEFKLKQYGIEIRKVAPNNTSKTCSKCGHLNNYFNFEYRKKNKFPHFKCEKCNFKENADYNAALNISNPKLKSTKEEP

SEQ ID NO: 6 - DNA, 1671 bp, synthetic construct
  source 1..1671: mol_type = other DNA; note = Human codon-optimized CWCas12f
atgggggagaaaagttcccgccgccgacggaatggaaaaagcggtgcgtggactgctgctataacaagctgtgttgggggtaagatggccaagaacacaattacaaagacactgaagctgaggatcgtgagaccatacaacagcgctgaggtcgagaagattgtggctgatgaaaagaacaacagggaaaagatcgccctcgagaagaacaaggataaggtgaaggaggcctgctctaagcacctgaaagtggccgcctactgcaccacacaggtggagaggaacgcctgtctgttttgtaaagctcggaagctggatgataagttttaccagaagctgcggggccagttccccgatgccgtcttttggcaggagattagcgagatcttcagacagctgcagaagcaggccgccgagatctacaaccagagcctgatcgagctctactacgagatcttcatcaagggcaagggcattgccaacgcctcctccgtggagcactacctgagcgacgtgtgctacacaagagccgccgagctctttaagaacgccgctatcgcttccgggctgaggagcaagattaagagtaacttccggctcaaggagctgaagaacatgaagagcggcctgcccactacaaagagcgacaacttcccaattccactggtgaagcagaaggggggccagtacacagggttcgagatttccaaccacaacagcgactttattattaagatcccctttggcaggtggcaggtcaagaaggagattgacaagtacaggccctgggagaagtttgatttcgagcaggtgcagaagagccccaagcctatttccctgctgctgtccacacagcggcggaagaggaacaaggggtggtctaaggatgaggggaccgaggccgagattaagaaagtgatgaacggcgactaccagacaagctacatcgaggtcaagcggggcagtaagattggcgagaagagcgcctggatgctgaacctgagcattgacgtgccaaagattgataagggcgtggatcccagcatcatcggagggatcgatgtgggggtcaagagccccctcgtgtgcgccatcaacaacgccttcagcaggtacagcatctccgataacgacctgttccactttaacaagaagatgttcgcccggcggaggattttgctcaagaagaaccggcacaagcgggccggacacggggccaagaacaagctcaagcccatcactatcctgaccgagaagagcgagaggttcaggaagaagctcatcgagagatgggcctgcgagatcgccgatttctttattaagaacaaggtcggaacagtgcagatggagaacctcgagagcatgaagaggaaggaggattcctacttcaacattcggctgagggggttctggccctacgctgagatgcagaacaagattgagtttaagctgaagcagtacgggattgagatccggaaggtggcccccaacaacaccagcaagacctgcagcaagtgcgggcacctcaacaactacttcaacttcgagtaccggaagaagaacaagttcccacacttcaagtgcgagaagtgcaactttaaggagaacgccgattacaacgccgccctgaacatcagcaaccctaagctgaagagcactaaggaggagccc

SEQ ID NO: 7 - DNA, 1666 bp, synthetic construct
  source 1..1666: mol_type = other DNA; note = Human codon-optimized CWCas12f-v1
atggaaaagagaatcaacaagatcaggaagaagctgagcgccgacaacgccaccaagcctgtgtctaggagtggcccccatggccaagaacacaattacaaagacactgaagctgaggatcgtgagaccatacaacagcgctgaggtcgagaagattgtggctgatgaaaagaacaacagggaaaagatcgccctcgagaagaacaaggataaggtgaaggaggcctgctctaagcacctgaaagtggccgcctactgcaccacacaggtggagaggaacgcctgtctgttttgtaaagctcggaagctggatgataagttttaccagaagctgcggggccagttccccgatgccgtcttttggcaggagattagcgagatcttcagacagctgcagaagcaggccgccgagatctacaaccagagcctgatcgagctctactacgagatcttcatcaagggcaagggcattgccaacgcctcctccgtggagcactacctgagcgacgtgtgctacacaagagccgccgagctctttaagaacgccgctatcgcttccgggctgaggagcaagattaagagtaacttccggctcaaggagctgaagaacatgaagagcggcctgcccactacaaagagcgacaacttcccaattccactggtgaagcagaaggggggccagtacacagggttcgagatttccaaccacaacagcgactttattattaagatcccctttggcaggtggcaggtcaagaaggagattgacaagtacaggccctgggagaagtttgatttcgagcaggtgcagaagagccccaagcctatttccctgctgctgtccacacagcggcggaagaggaacaaggggtggtctaaggatgaggggaccgaggccgagattaagaaagtgatgaacggcgactaccagacaagctacatcgaggtcaagcggggcagtaagattggcgagaagagcgcctggatgctgaacctgagcattgacgtgccaaagattgataagggcgtggatcccagcatcatcggagggatcgatgtgggggtcaagagccccctcgtgtgcgccatcaacaacgccttcagcaggtacagcatctccgataacgacctgttccactttaacaagaagatgttcgcccggcggaggattttgctcaagaagaaccggcacaagcgggccggacacggggccaagaacaagctcaagcccatcactatcctgaccgagaagagcgagaggttcaggaagaagctcatcgagagatgggcctgcgagatcgccgatttctttattaagaacaaggtcggaacagtgcagatggagaacctcgagagcatgaagaggaaggaggattcctacttcaacattcggctgagggggttctggccctacgctgagatgcagaacaagattgagtttaagctgaagcagtacgggattgagatccggaaggtggcccccaacaacaccagcaagacctgcagcaagtgcgggcacctcaacaactacttcaacttcgagtaccggaagaagaacaagttcccacacttcaagtgcgagaagtgcaactttaaggagaacgccgattacaacgccgccctgaacatcagcaaccctaagctgaagagcactaaggaggagccc

SEQ ID NO: 8 - DNA, 1671 bp, synthetic construct
  source 1..1671: mol_type = other DNA; note = Human codon-optimized CWCas12f-v2
atggctggcggaccaggcgcaggtagtgctgcgccagtttcttcaacttcctccctgcccctggctgcgcttaacatgcgcgtgatggccaagaacacaattacaaagacactgaagctgaggatcgtgagaccatacaacagcgctgaggtcgagaagattgtggctgatgaaaagaacaacagggaaaagatcgccctcgagaagaacaaggataaggtgaaggaggcctgctctaagcacctgaaagtggccgcctactgcaccacacaggtggagaggaacgcctgtctgttttgtaaagctcggaagctggatgataagttttaccagaagctgcggggccagttccccgatgccgtcttttggcaggagattagcgagatcttcagacagctgcagaagcaggccgccgagatctacaaccagagcctgatcgagctctactacgagatcttcatcaagggcaagggcattgccaacgcctcctccgtggagcactacctgagcgacgtgtgctacacaagagccgccgagctctttaagaacgccgctatcgcttccgggctgaggagcaagattaagagtaacttccggctcaaggagctgaagaacatgaagagcggcctgcccactacaaagagcgacaacttcccaattccactggtgaagcagaaggggggccagtacacagggttcgagatttccaaccacaacagcgactttattattaagatcccctttggcaggtggcaggtcaagaaggagattgacaagtacaggccctgggagaagtttgatttcgagcaggtgcagaagagccccaagcctatttccctgctgctgtccacacagcggcggaagaggaacaaggggtggtctaaggatgaggggaccgaggccgagattaagaaagtgatgaacggcgactaccagacaagctacatcgaggtcaagcggggcagtaagattggcgagaagagcgcctggatgctgaacctgagcattgacgtgccaaagattgataagggcgtggatcccagcatcatcggagggatcgatgtgggggtcaagagccccctcgtgtgcgccatcaacaacgccttcagcaggtacagcatctccgataacgacctgttccactttaacaagaagatgttcgcccggcggaggattttgctcaagaagaaccggcacaagcgggccggacacggggccaagaacaagctcaagcccatcactatcctgaccgagaagagcgagaggttcaggaagaagctcatcgagagatgggcctgcgagatcgccgatttctttattaagaacaaggtcggaacagtgcagatggagaacctcgagagcatgaagaggaaggaggattcctacttcaacattcggctgagggggttctggccctacgctgagatgcagaacaagattgagtttaagctgaagcagtacgggattgagatccggaaggtggcccccaacaacaccagcaagacctgcagcaagtgcgggcacctcaacaactacttcaacttcgagtaccggaagaagaacaagttcccacacttcaagtgcgagaagtgcaactttaaggagaacgccgattacaacgccgccctgaacatcagcaaccctaagctgaagagcactaaggaggagccc

SEQ ID NO: 9 - DNA, 1665 bp, synthetic construct
  source 1..1665: mol_type = other DNA; note = Human codon-optimized CWCas12f-v3
atggctggcggaccaggcgcaggtagtgctgcgccagtttcttcaacttcctccctgcccctggctgcgcttaacatgatggccaagaacacaattacaaagacactgaagctgaggatcgtgagaccatacaacagcgctgaggtcgagaagattgtggctgatgaaaagaacaacagggaaaagatcgccctcgagaagaacaaggataaggtgaaggaggcctgctctaagcacctgaaagtggccgcctactgcaccacacaggtggagaggaacgcctgtctgttttgtaaagctcggaagctggatgataagttttaccagaagctgcggggccagttccccgatgccgtcttttggcaggagattagcgagatcttcagacagctgcagaagcaggccgccgagatctacaaccagagcctgatcgagctctactacgagatcttcatcaagggcaagggcattgccaacgcctcctccgtggagcactacctgagcgacgtgtgctacacaagagccgccgagctctttaagaacgccgctatcgcttccgggctgaggagcaagattaagagtaacttccggctcaaggagctgaagaacatgaagagcggcctgcccactacaaagagcgacaacttcccaattccactggtgaagcagaaggggggccagtacacagggttcgagatttccaaccacaacagcgactttattattaagatcccctttggcaggtggcaggtcaagaaggagattgacaagtacaggccctgggagaagtttgatttcgagcaggtgcagaagagccccaagcctatttccctgctgctgtccacacagcggcggaagaggaacaaggggtggtctaaggatgaggggaccgaggccgagattaagaaagtgatgaacggcgactaccagacaagctacatcgaggtcaagcggggcagtaagattggcgagaagagcgcctggatgctgaacctgagcattgacgtgccaaagattgataagggcgtggatcccagcatcatcggagggatcgatgtgggggtcaagagccccctcgtgtgcgccatcaacaacgccttcagcaggtacagcatctccgataacgacctgttccactttaacaagaagatgttcgcccggcggaggattttgctcaagaagaaccggcacaagcgggccggacacggggccaagaacaagctcaagcccatcactatcctgaccgagaagagcgagaggttcaggaagaagctcatcgagagatgggcctgcgagatcgccgatttctttattaagaacaaggtcggaacagtgcagatggagaacctcgagagcatgaagaggaaggaggattcctacttcaacattcggctgagggggttctggccctacgctgagatgcagaacaagattgagtttaagctgaagcagtacgggattgagatccggaaggtggcccccaacaacaccagcaagacctgcagcaagtgcgggcacctcaacaactacttcaacttcgagtaccggaagaagaacaagttcccacacttcaagtgcgagaagtgcaactttaaggagaacgccgattacaacgccgccctgaacatcagcaaccctaagctgaagagcactaaggaggagccc

SEQ ID NO: 10 - DNA, 1587 bp, synthetic construct
  source 1..1587: mol_type = other DNA; note = Human codon-optimized Un1Cas12f1
atggccaagaacacaattacaaagacactgaagctgaggatcgtgagaccatacaacagcgctgaggtcgagaagattgtggctgatgaaaagaacaacagggaaaagatcgccctcgagaagaacaaggataaggtgaaggaggcctgctctaagcacctgaaagtggccgcctactgcaccacacaggtggagaggaacgcctgtctgttttgtaaagctcggaagctggatgataagttttaccagaagctgcggggccagttccccgatgccgtcttttggcaggagattagcgagatcttcagacagctgcagaagcaggccgccgagatctacaaccagagcctgatcgagctctactacgagatcttcatcaagggcaagggcattgccaacgcctcctccgtggagcactacctgagcgacgtgtgctacacaagagccgccgagctctttaagaacgccgctatcgcttccgggctgaggagcaagattaagagtaacttccggctcaaggagctgaagaacatgaagagcggcctgcccactacaaagagcgacaacttcccaattccactggtgaagcagaaggggggccagtacacagggttcgagatttccaaccacaacagcgactttattattaagatcccctttggcaggtggcaggtcaagaaggagattgacaagtacaggccctgggagaagtttgatttcgagcaggtgcagaagagccccaagcctatttccctgctgctgtccacacagcggcggaagaggaacaaggggtggtctaaggatgaggggaccgaggccgagattaagaaagtgatgaacggcgactaccagacaagctacatcgaggtcaagcggggcagtaagattggcgagaagagcgcctggatgctgaacctgagcattgacgtgccaaagattgataagggcgtggatcccagcatcatcggagggatcgatgtgggggtcaagagccccctcgtgtgcgccatcaacaacgccttcagcaggtacagcatctccgataacgacctgttccactttaacaagaagatgttcgcccggcggaggattttgctcaagaagaaccggcacaagcgggccggacacggggccaagaacaagctcaagcccatcactatcctgaccgagaagagcgagaggttcaggaagaagctcatcgagagatgggcctgcgagatcgccgatttctttattaagaacaaggtcggaacagtgcagatggagaacctcgagagcatgaagaggaaggaggattcctacttcaacattcggctgagggggttctggccctacgctgagatgcagaacaagattgagtttaagctgaagcagtacgggattgagatccggaaggtggcccccaacaacaccagcaagacctgcagcaagtgcgggcacctcaacaactacttcaacttcgagtaccggaagaagaacaagttcccacacttcaagtgcgagaagtgcaactttaaggagaacgccgattacaacgccgccctgaacatcagcaaccctaagctgaagagcactaaggaggagccc

SEQ ID NO: 11 - RNA, 161 nt, synthetic construct
  source 1..161: mol_type = other RNA; note = Wild-type tracrRNA for CWCas12f or Un1Cas12f1 gRNA
cttcactgataaagtggagaaccgcttcaccaaaagctgtcccttaggggattagaacttgagtgaaggtgggctgcttgcatcagcctaatgtcgagaagtgctttcttcggaaagtaaccctcgaaacaaattcatttttcctctccaattctgcacaa

SEQ ID NO: 12 - RNA, 37 nt, synthetic construct
  source 1..37: mol_type = other RNA; note = Wild-type crRNA for CWCas12f or Un1Cas12f1 gRNA
gttgcagaacccgaatagacgaatgaaggaatgcaac

SEQ ID NO: 13 - RNA, 222 nt, synthetic construct
  source 1..222: mol_type = other RNA; note = Canonical sgRNA for CWCas12f or Un1Cas12f1
  misc_feature 203..222: note = n is a, c, g or u
cttcactgataaagtggagaaccgcttcaccaaaagctgtcccttaggggattagaacttgagtgaaggtgggctgcttgcatcagcctaatgtcgagaagtgctttcttcggaaagtaaccctcgaaacaaattcatttttcctctccaattctgcacaagaaagttgcagaacccgaatagacgaatgaaggaatgcaacnnnnnnnnnnnnnnnnnnnn

SEQ ID NO: 14 - RNA, 20 nt, synthetic construct
  source 1..20: mol_type = other RNA; note = Xa of Formula (I)
cttcactgataaagtggaga

SEQ ID NO: 15 - RNA, 19 nt, synthetic construct
  source 1..19: mol_type = other RNA; note = Xa of Formula (I)
ttcactgataaagtggaga

SEQ ID NO: 16 - RNA, 18 nt, synthetic construct
  source 1..18: mol_type = other RNA; note = Xa of Formula (I)
tcactgataaagtggaga

SEQ ID NO: 17 - RNA, 17 nt, synthetic construct
  source 1..17: mol_type = other RNA; note = Xa of Formula (I)
cactgataaagtggaga

SEQ ID NO: 18 - RNA, 16 nt, synthetic construct
  source 1..16: mol_type = other RNA; note = Xa of Formula (I)
actgataaagtggaga

SEQ ID NO: 19 - RNA, 15 nt, synthetic construct
  source 1..15: mol_type = other RNA; note = Xa of Formula (I)
ctgataaagtggaga

SEQ ID NO: 20 - RNA, 14 nt, synthetic construct
  source 1..14: mol_type = other RNA; note = Xa of Formula (I)
tgataaagtggaga

SEQ ID NO: 21 - RNA, 13 nt, synthetic construct
  source 1..13: mol_type = other RNA; note = Xa of Formula (I)
gataaagtggaga

SEQ ID NO: 22 - RNA, 12 nt, synthetic construct
  source 1..12: mol_type = other RNA; note = Xa of Formula (I)
ataaagtggaga

SEQ ID NO: 23 - RNA, 11 nt, synthetic construct
  source 1..11: mol_type = other RNA; note = Xa of Formula (I)
taaagtggaga

SEQ ID NO: 24 - RNA, 10 nt, synthetic construct
  source 1..10: mol_type = other RNA; note = Xa of Formula (I)
aaagtggaga

SEQ ID NO: 25 - RNA, 13 nt, synthetic construct
  source 1..13: mol_type = other RNA; note = Xb1 of Formula (I)
caaaagctgtccc

SEQ ID NO: 26 - RNA, 12 nt, synthetic construct
  source 1..12: mol_type = other RNA; note = Xb1 of Formula (I)
caaaagctgtcc

SEQ ID NO: 27 - RNA, 11 nt, synthetic construct
  source 1..11: mol_type = other RNA; note = Xb1 of Formula (I)
caaaagctgtc

SEQ ID NO: 28 - RNA, 10 nt, synthetic construct
  source 1..10: mol_type = other RNA; note = Xb1 of Formula (I)
caaaagctgt

SEQ ID NO: 29 - RNA, 14 nt, synthetic construct
  source 1..14: mol_type = other RNA; note = Xb2 of Formula (I)
gggattagaacttg

SEQ ID NO: 30 - RNA, 13 nt, synthetic construct
  source 1..13: mol_type = other RNA; note = Xb2 of Formula (I)
ggattagaacttg

SEQ ID NO: 31 - RNA, 12 nt, synthetic construct
  source 1..12: mol_type = other RNA; note = Xb2 of Formula (I)
gattagaacttg

SEQ ID NO: 32 - RNA, 11 nt, synthetic construct
  source 1..11: mol_type = other RNA; note = Xb2 of Formula (I)
attagaacttg

SEQ ID NO: 33 - RNA, 10 nt, synthetic construct
  source 1..10: mol_type = other RNA; note = Xb2 of Formula (I)
ttagaacttg

SEQ ID NO: 34 - RNA, 31 nt, synthetic construct
  source 1..31: mol_type = other RNA; note = Xb1-UUAG-Xb2 of Formula (I)
caaaagctgtcccttaggggattagaacttg

SEQ ID NO: 35 - RNA, 25 nt, synthetic construct
  source 1..25: mol_type = other RNA; note = Xb1-UUAG-Xb2 of Formula (I)
caaaagctgtttagattagaacttg

SEQ ID NO: 36 - RNA, 20 nt, synthetic construct
  source 1..20: mol_type = other RNA; note = Xb1-UUAG-Xb2 of Formula (I)
caaaagctttagagaacttg

SEQ ID NO: 37 - RNA, 18 nt, synthetic construct
  source 1..18: mol_type = other RNA; note = Xb1-UUAG-Xb2 of Formula (I)
caaaagcttaggaacttg

SEQ ID NO: 38 - RNA, 10 nt, synthetic construct
  source 1..10: mol_type = other RNA; note = Xb1-UUAG-Xb2 of Formula (I)
caattagttg

SEQ ID NO: 39 - RNA, 28 nt, synthetic construct
  source 1..28: mol_type = other RNA; note = Xc1 of Formula (I)
ttcatttttcctctccaattctgcacaa

SEQ ID NO: 40 - RNA, 27 nt, synthetic construct
  source 1..27: mol_type = other RNA; note = Xc1 of Formula (I)
ttcatttttcctctccaattctgcaca

SEQ ID NO: 41 - RNA, 26 nt, synthetic construct
  source 1..26: mol_type = other RNA; note = Xc1 of Formula (I)
ttcatttttcctctccaattctgcac

SEQ ID NO: 42 - RNA, 25 nt, synthetic construct
  source 1..25: mol_type = other RNA; note = Xc1 of Formula (I)
ttcatttttcctctccaattctgca

SEQ ID NO: 43 - RNA, 24 nt, synthetic construct
  source 1..24: mol_type = other RNA; note = Xc1 of Formula (I)
ttcatttttcctctccaattctgc

SEQ ID NO: 44 - RNA, 23 nt, synthetic construct
  source 1..23: mol_type = other RNA; note = Xc1 of Formula (I)
ttcatttttcctctccaattctg

SEQ ID NO: 45 - RNA, 22 nt, synthetic construct
  source 1..22: mol_type = other RNA; note = Xc1 of Formula (I)
ttcatttttcctctccaattct

SEQ ID NO: 46 - RNA, 21 nt, synthetic construct
  source 1..21: mol_type = other RNA; note = Xc1 of Formula (I)
ttcatttttcctctccaattc

SEQ ID NO: 47 - RNA, 20 nt, synthetic construct
  source 1..20: mol_type = other RNA; note = Xc1 of Formula (I)
ttcatttttcctctccaatt

SEQ ID NO: 48 - RNA, 19 nt, synthetic construct
  source 1..19: mol_type = other RNA; note = Xc1 of Formula (I)
ttcatttttcctctccaat

SEQ ID NO: 49 - RNA, 18 nt, synthetic construct
  source 1..18: mol_type = other RNA; note = Xc1 of Formula (I)
ttcatttttcctctccaa

SEQ ID NO: 50 - RNA, 17 nt, synthetic construct
  source 1..17: mol_type = other RNA; note = Xc1 of Formula (I)
ttcatttttcctctcca

SEQ ID NO: 51 - RNA, 16 nt, synthetic construct
  source 1..16: mol_type = other RNA; note = Xc1 of Formula (I)
ttcatttttcctctcc

SEQ ID NO: 52 - RNA, 15 nt, synthetic construct
  source 1..15: mol_type = other RNA; note = Xc1 of Formula (I)
ttcatttttcctctc

SEQ ID NO: 53 - RNA, 14 nt, synthetic construct
  source 1..14: mol_type = other RNA; note = Xc1 of Formula (I)
ttcatttttcctct

SEQ ID NO: 54 - RNA, 13 nt, synthetic construct
  source 1..13: mol_type = other RNA; note = Xc1 of Formula (I)
ttcatttttcctc

SEQ ID NO: 55 - RNA, 12 nt, synthetic construct
  source 1..12: mol_type = other RNA; note = Xc1 of Formula (I)
ttcatttttcct

SEQ ID NO: 56 - RNA, 11 nt, synthetic construct
  source 1..11: mol_type = other RNA; note = Xc1 of Formula (I)
ttcatttttcc

SEQ ID NO: 57 - RNA, 10 nt, synthetic construct
  source 1..10: mol_type = other RNA; note = Xc1 of Formula (I)
ttcatttttc

SEQ ID NO: 58 - RNA, 27 nt, synthetic construct
  source 1..27: mol_type = other RNA; note = Xc2 of Formula (I)
gttgcagaacccgaatagacgaatgaa

SEQ ID NO: 59 - RNA, 26 nt, synthetic construct
  source 1..26: mol_type = other RNA; note = Xc2 of Formula (I)
ttgcagaacccgaatagacgaatgaa

SEQ ID NO: 60 - RNA, 25 nt, synthetic construct
  source 1..25: mol_type = other RNA; note = Xc2 of Formula (I)
tgcagaacccgaatagacgaatgaa

SEQ ID NO: 61 - RNA, 24 nt, synthetic construct
  source 1..24: mol_type = other RNA; note = Xc2 of Formula (I)
gcagaacccgaatagacgaatgaa

SEQ ID NO: 62 - RNA, 23 nt, synthetic construct
  source 1..23: mol_type = other RNA; note = Xc2 of Formula (I)
cagaacccgaatagacgaatgaa

SEQ ID NO: 63 - RNA, 22 nt, synthetic construct
  source 1..22: mol_type = other RNA; note = Xc2 of Formula (I)
agaacccgaatagacgaatgaa

SEQ ID NO: 64 - RNA, 21 nt, synthetic construct
  source 1..21: mol_type = other RNA; note = Xc2 of Formula (I)
gaacccgaatagacgaatgaa

SEQ ID NO: 65 - RNA, 20 nt, synthetic construct
  source 1..20: mol_type = other RNA; note = Xc2 of Formula (I)
aacccgaatagacgaatgaa

SEQ ID NO: 66 - RNA, 19 nt, synthetic construct
  source 1..19: mol_type = other RNA; note = Xc2 of Formula (I)
acccgaatagacgaatgaa

SEQ ID NO: 67 - RNA, 18 nt, synthetic construct
  source 1..18: mol_type = other RNA; note = Xc2 of Formula (I)
cccgaatagacgaatgaa

SEQ ID NO: 68 - RNA, 17 nt, synthetic construct
  source 1..17: mol_type = other RNA; note = Xc2 of Formula (I)
ccgaatagacgaatgaa

SEQ ID NO: 69 - RNA, 16 nt, synthetic construct
  source 1..16: mol_type = other RNA; note = Xc2 of Formula (I)
cgaatagacgaatgaa

SEQ ID NO: 70 - RNA, 15 nt, synthetic construct
  source 1..15: mol_type = other RNA; note = Xc2 of Formula (I)
gaatagacgaatgaa

SEQ ID NO: 71 - RNA, 14 nt, synthetic construct
  source 1..14: mol_type = other RNA; note = Xc2 of Formula (I)
aatagacgaatgaa

SEQ ID NO: 72 - RNA, 13 nt, synthetic construct
  source 1..13: mol_type = other RNA; note = Xc2 of Formula (I)
atagacgaatgaa

SEQ ID NO: 73 - RNA, 12 nt, synthetic construct
  source 1..12: mol_type = other RNA; note = Xc2 of Formula (I)
tagacgaatgaa

SEQ ID NO: 74 - RNA, 11 nt, synthetic construct
  source 1..11: mol_type = other RNA; note = Xc2 of Formula (I)
agacgaatgaa

SEQ ID NO: 75 - RNA, 10 nt, synthetic construct
  source 1..10: mol_type = other RNA; note = Xc2 of Formula (I)
gacgaatgaa

SEQ ID NO: 76 - RNA, 10 nt, synthetic construct
  source 1..10: mol_type = other RNA; note = Linker (Lk)
ttcgaaagaa

SEQ ID NO: 77 - RNA, 12 nt, synthetic construct
  source 1..12: mol_type = other RNA; note = Linker (Lk)
ttcagaaatgaa

SEQ ID NO: 78 - RNA, 14 nt, synthetic construct
  source 1..14: mol_type = other RNA; note = Linker (Lk)
ttcatgaaaatgaa

SEQ ID NO: 79 - RNA, 16 nt, synthetic construct
  source 1..16: mol_type = other RNA; note = Linker (Lk)
ttcattgaaaaatgaa

SEQ ID NO: 80 - RNA, 59 nt, synthetic construct
  source 1..59: mol_type = other RNA; note = Xc1-Lk-Xc2 of Formula (I)
ttcagtgctcctctccaattctgcacaagaaagttgcagaacccgaatagagcaatgaa

SEQ ID NO: 81 - RNA, 46 nt, synthetic construct
  source 1..46: mol_type = other RNA; note = Xc1-Lk-Xc2 of Formula (I)
ttcagtgctcctctccaattcgaaagaacccgaatagagcaatgaa

SEQ ID NO: 82 - RNA, 34 nt, synthetic construct
  source 1..34: mol_type = other RNA; note = Xc1-Lk-Xc2 of Formula (I)
ttcagtgctcctctcgaaagaatagagcaatgaa

SEQ ID NO: 83 - RNA, 22 nt, synthetic construct
  source 1..22: mol_type = other RNA; note = Xc1-Lk-Xc2 of Formula (I)
ttcagtgctgaaaagcaatgaa

SEQ ID NO: 84 - RNA, 18 nt, synthetic construct
  source 1..18: mol_type = other RNA; note = Xc1-Lk-Xc2 of Formula (I)
ttcatttgaaagaatgaa

SEQ ID NO: 85 - RNA, 14 nt, synthetic construct
  source 1..14: mol_type = other RNA; note = Xc1-Lk-Xc2 of Formula (I)
ttcatgaaaatgaa

SEQ ID NO: 86 - RNA, 10 nt, synthetic construct
  source 1..10: mol_type = other RNA; note = Xc1-Lk-Xc2 of Formula (I)
ttcgaaagaa

SEQ ID NO: 87 - RNA, 161 nt, synthetic construct
  source 1..161: mol_type = other RNA; note = Engineered tracrRNA for CWCas12f or Un1Cas12f1 gRNA (MS1)
cttcactgataaagtggagaaccgcttcaccaaaagctgtcccttaggggattagaacttgagtgaaggtgggctgcttgcatcagcctaatgtcgagaagtgctttcttcggaaagtaaccctcgaaacaaattcagtgctcctctccaattctgcacaa

SEQ ID NO: 88 - RNA, 154 nt, synthetic construct
  source 1..154: mol_type = other RNA; note = Engineered tracrRNA for CWCas12f or Un1Cas12f1 gRNA (MS1/MS3-1)
gataaagtggagaaccgcttcaccaaaagctgtcccttaggggattagaacttgagtgaaggtgggctgcttgcatcagcctaatgtcgagaagtgctttcttcggaaagtaaccctcgaaacaaattcagtgctcctctccaattctgcacaa

SEQ ID NO: 89 - RNA, 147 nt, synthetic construct
  source 1..147: mol_type = other RNA; note = Engineered tracrRNA for CWCas12f or Un1Cas12f1 gRNA (MS1/MS3-2)
tggagaaccgcttcaccaaaagctgtcccttaggggattagaacttgagtgaaggtgggctgcttgcatcagcctaatgtcgagaagtgctttcttcggaaagtaaccctcgaaacaaattcagtgctcctctccaattctgcacaa

SEQ ID NO: 90 - RNA, 141 nt, synthetic construct
  source 1..141: mol_type = other RNA; note = Engineered tracrRNA for CWCas12f or Un1Cas12f1 gRNA (MS1/MS3-3)
accgcttcaccaaaagctgtcccttaggggattagaacttgagtgaaggtgggctgcttgcatcagcctaatgtcgagaagtgctttcttcggaaagtaaccctcgaaacaaattcagtgctcctctccaattctgcacaa

SEQ ID NO: 91 - RNA, 154 nt, synthetic construct
  source 1..154: mol_type = other RNA; note = Engineered tracrRNA for CWCas12f or Un1Cas12f1 gRNA (MS1/MS4*-1)
cttcactgataaagtggagaaccgcttcaccaaaagctgtcccttaggggattagaacttgagtgaaggtgggctgcttgcatcagcctaatgtcgagaagtgctttcttcggaaagtaaccctcgaaacaaattcagtgctcctctccaattc

SEQ ID NO: 92 - RNA, 148 nt, synthetic construct
  source 1..148: mol_type = other RNA; note = Engineered tracrRNA for CWCas12f or Un1Cas12f1 gRNA (MS1/MS4*-2)
cttcactgataaagtggagaaccgcttcaccaaaagctgtcccttaggggattagaacttgagtgaaggtgggctgcttgcatcagcctaatgtcgagaagtgctttcttcggaaagtaaccctcgaaacaaattcagtgctcctctc

SEQ ID NO: 93 - RNA, 142 nt, synthetic construct
  source 1..142: mol_type = other RNA; note = Engineered tracrRNA for CWCas12f or Un1Cas12f1 gRNA (MS1/MS4*-3)
cttcactgataaagtggagaaccgcttcaccaaaagctgtcccttaggggattagaacttgagtgaaggtgggctgcttgcatcagcctaatgtcgagaagtgctttcttcggaaagtaaccctcgaaacaaattcagtgct

SEQ ID NO: 94 - RNA, 155 nt, synthetic construct
  source 1..155: mol_type = other RNA; note = Engineered tracrRNA for CWCas12f or Un1Cas12f1 gRNA (MS1/MS5-1)
cttcactgataaagtggagaaccgcttcaccaaaagctgtttagattagaacttgagtgaaggtgggctgcttgcatcagcctaatgtcgagaagtgctttcttcggaaagtaaccctcgaaacaaattcagtgctcctctccaattctgcacaa

SEQ ID NO: 95 - RNA, 148 nt, synthetic construct
  source 1..148: mol_type = other RNA; note = Engineered tracrRNA for CWCas12f or Un1Cas12f1 gRNA (MS1/MS5-2)
cttcactgataaagtggagaaccgcttcaccaaaagcttaggaacttgagtgaaggtgggctgcttgcatcagcctaatgtcgagaagtgctttcttcggaaagtaaccctcgaaacaaattcagtgctcctctccaattctgcacaa

SEQ ID NO: 96 - RNA, 140 nt, synthetic construct
  source 1..140: mol_type = other RNA; note = Engineered tracrRNA for CWCas12f or Un1Cas12f1 gRNA (MS1/MS5-3)
cttcactgataaagtggagaaccgcttcaccaattagttgagtgaaggtgggctgcttgcatcagcctaatgtcgagaagtgctttcttcggaaagtaaccctcgaaacaaattcagtgctcctctccaattctgcacaa

SEQ ID NO: 97 - RNA, 134 nt, synthetic construct
  source 1..134: mol_type = other RNA; note = Engineered tracrRNA for CWCas12f or Un1Cas12f1 gRNA (MS1/MS3-3/MS4*-1)
accgcttcaccaaaagctgtcccttaggggattagaacttgagtgaaggtgggctgcttgcatcagcctaatgtcgagaagtgctttcttcggaaagtaaccctcgaaacaaattcagtgctcctctccaattc

SEQ ID NO: 98 - RNA, 128 nt, synthetic construct
  source 1..128: mol_type = other RNA; note = Engineered tracrRNA for CWCas12f or Un1Cas12f1 gRNA (MS1/MS3-3/MS4*-2)
accgcttcaccaaaagctgtcccttaggggattagaacttgagtgaaggtgggctgcttgcatcagcctaatgtcgagaagtgctttcttcggaaagtaaccctcgaaacaaattcagtgctcctctc

SEQ ID NO: 99 - RNA, 122 nt, synthetic construct
  source 1..122: mol_type = other RNA; note = Engineered tracrRNA for CWCas12f or Un1Cas12f1 gRNA (MS1/MS3-3/MS4*-3)
accgcttcaccaaaagctgtcccttaggggattagaacttgagtgaaggtgggctgcttgcatcagcctaatgtcgagaagtgctttcttcggaaagtaaccctcgaaacaaattcagtgct

SEQ ID NO: 100 - RNA, 142 nt, synthetic construct
  source 1..142: mol_type = other RNA; note = Engineered tracrRNA for CWCas12f or Un1Cas12f1 gRNA (MS1/MS4*-2/MS5-1)
cttcactgataaagtggagaaccgcttcaccaaaagctgtttagattagaacttgagtgaaggtgggctgcttgcatcagcctaatgtcgagaagtgctttcttcggaaagtaaccctcgaaacaaattcagtgctcctctc

SEQ ID NO: 101 - RNA, 135 nt, synthetic construct
  source 1..135: mol_type = other RNA; note = Engineered tracrRNA for CWCas12f or Un1Cas12f1 gRNA (MS1/MS4*-2/MS5-2)
cttcactgataaagtggagaaccgcttcaccaaaagcttaggaacttgagtgaaggtgggctgcttgcatcagcctaatgtcgagaagtgctttcttcggaaagtaaccctcgaaacaaattcagtgctcctctc

SEQ ID NO: 102 - RNA, 127 nt, synthetic construct
  source 1..127: mol_type = other RNA; note = Engineered tracrRNA for CWCas12f or Un1Cas12f1 gRNA (MS1/MS4*-2/MS5-3)
cttcactgataaagtggagaaccgcttcaccaattagttgagtgaaggtgggctgcttgcatcagcctaatgtcgagaagtgctttcttcggaaagtaaccctcgaaacaaattcagtgctcctctc

SEQ ID NO: 103 - RNA, 135 nt, synthetic construct
  source 1..135: mol_type = other RNA; note = Engineered tracrRNA for CWCas12f or Un1Cas12f1 gRNA (MS1/MS3-3/MS5-1)
accgcttcaccaaaagctgtttagattagaacttgagtgaaggtgggctgcttgcatcagcctaatgtcgagaagtgctttcttcggaaagtaaccctcgaaacaaattcagtgctcctctccaattctgcacaa

SEQ ID NO: 104 - RNA, 128 nt, synthetic construct
  source 1..128: mol_type = other RNA; note = Engineered tracrRNA for CWCas12f or Un1Cas12f1 gRNA (MS1/MS3-3/MS5-2)
accgcttcaccaaaagcttaggaacttgagtgaaggtgggctgcttgcatcagcctaatgtcgagaagtgctttcttcggaaagtaaccctcgaaacaaattcagtgctcctctccaattctgcacaa

SEQ ID NO: 105 - RNA, 120 nt, synthetic construct
  source 1..120: mol_type = other RNA; note = Engineered tracrRNA for CWCas12f or Un1Cas12f1 gRNA (MS1/MS3-3/MS5-3)
accgcttcaccaattagttgagtgaaggtgggctgcttgcatcagcctaatgtcgagaagtgctttcttcggaaagtaaccctcgaaacaaattcagtgctcctctccaattctgcacaa

SEQ ID NO: 106 - RNA, 107 nt, synthetic construct
  source 1..107: mol_type = other RNA; note = Engineered tracrRNA for CWCas12f or Un1Cas12f1 gRNA (MS1/MS3-3/MS4*-2/MS5-3)
accgcttcaccaattagttgagtgaaggtgggctgcttgcatcagcctaatgtcgagaagtgctttcttcggaaagtaaccctcgaaacaaattcagtgctcctctc

SEQ ID NO: 107 - RNA, 140 nt, synthetic construct
  source 1..140: mol_type = other RNA; note = Engineered tracrRNA for CWCas12f or Un1Cas12f1 gRNA (MF)
cttcactgataaagtggagaaccgcttcaccaaaagctgtcccttaggggattagaacttgagtgaaggtgggctgcttgcatcagcctaatgtcgagaagtgctttcttcggaaagtaaccctcgaaacaaattcattt

SEQ ID NO: 108 - RNA, 133 nt, synthetic construct
  source 1..133: mol_type = other RNA; note = Engineered tracrRNA for CWCas12f or Un1Cas12f1 gRNA (MF/MS3-1)
gataaagtggagaaccgcttcaccaaaagctgtcccttaggggattagaacttgagtgaaggtgggctgcttgcatcagcctaatgtcgagaagtgctttcttcggaaagtaaccctcgaaacaaattcattt

SEQ ID NO: 109 - RNA, 126 nt, synthetic construct
  source 1..126: mol_type = other RNA; note = Engineered tracrRNA for CWCas12f or Un1Cas12f1 gRNA (MF/MS3-2)
tggagaaccgcttcaccaaaagctgtcccttaggggattagaacttgagtgaaggtgggctgcttgcatcagcctaatgtcgagaagtgctttcttcggaaagtaaccctcgaaacaaattcattt

SEQ ID NO: 110 - RNA, 120 nt, synthetic construct
  source 1..120: mol_type = other RNA; note = Engineered tracrRNA for CWCas12f or Un1Cas12f1 gRNA (MF/MS3-3)
accgcttcaccaaaagctgtcccttaggggattagaacttgagtgaaggtgggctgcttgcatcagcctaatgtcgagaagtgctttcttcggaaagtaaccctcgaaacaaattcattt

SEQ ID NO: 111 - RNA, 138 nt, synthetic construct
  source 1..138: mol_type = other RNA; note = Engineered tracrRNA for CWCas12f or Un1Cas12f1 gRNA (MF/MS4-1)
cttcactgataaagtggagaaccgcttcaccaaaagctgtcccttaggggattagaacttgagtgaaggtgggctgcttgcatcagcctaatgtcgagaagtgctttcttcggaaagtaaccctcgaaacaaattcat

SEQ ID NO: 112 - RNA, 136 nt, synthetic construct
  source 1..136: mol_type = other RNA; note = Engineered tracrRNA for CWCas12f or Un1Cas12f1 gRNA (MF/MS4-2)
cttcactgataaagtggagaaccgcttcaccaaaagctgtcccttaggggattagaacttgagtgaaggtgggctgcttgcatcagcctaatgtcgagaagtgctttcttcggaaagtaaccctcgaaacaaattc

SEQ ID NO: 113 - RNA, 133 nt, synthetic construct
  source 1..133: mol_type = other RNA; note = Engineered tracrRNA for CWCas12f or Un1Cas12f1 gRNA (MF/MS4-3)
cttcactgataaagtggagaaccgcttcaccaaaagctgtcccttaggggattagaacttgagtgaaggtgggctgcttgcatcagcctaatgtcgagaagtgctttcttcggaaagtaaccctcgaaacaaa

SEQ ID NO: 114 - RNA, 134 nt, synthetic construct
  source 1..134: mol_type = other RNA; note = Engineered tracrRNA for CWCas12f or Un1Cas12f1 gRNA (MF/MS5-1)
cttcactgataaagtggagaaccgcttcaccaaaagctgtttagattagaacttgagtgaaggtgggctgcttgcatcagcctaatgtcgagaagtgctttcttcggaaagtaaccctcgaaacaaattcattt

SEQ ID NO: 115 - RNA, 129 nt, synthetic construct
  source 1..129: mol_type = other RNA; note = Engineered tracrRNA for CWCas12f or Un1Cas12f1 gRNA (MF/MS5-2)
cttcactgataaagtggagaaccgcttcaccaaaagctttagagaacttgagtgaaggtgggctgcttgcatcagcctaatgtcgagaagtgctttcttcggaaagtaaccctcgaaacaaattcattt

SEQ ID NO: 116 - RNA, 119 nt, synthetic construct
  source 1..119: mol_type = other RNA; note = Engineered tracrRNA for CWCas12f or Un1Cas12f1 gRNA (MF/MS5-3)
cttcactgataaagtggagaaccgcttcaccaattagttgagtgaaggtgggctgcttgcatcagcctaatgtcgagaagtgctttcttcggaaagtaaccctcgaaacaaattcattt

SEQ ID NO: 117 - RNA, 113 nt, synthetic construct
  source 1..113: mol_type = other RNA; note = Engineered tracrRNA for CWCas12f or Un1Cas12f1 gRNA (MF/MS5)
cttcactgataaagtggagaaccgcttcacttagagtgaaggtgggctgcttgcatcagcctaatgtcgagaagtgctttcttcggaaagtaaccctcgaaacaaattcattt

SEQ ID NO: 118 - RNA, 118 nt, synthetic construct
  source 1..118: mol_type = other RNA; note = Engineered tracrRNA for CWCas12f or Un1Cas12f1 gRNA (MF/MS3-3/MS4-1)
accgcttcaccaaaagctgtcccttaggggattagaacttgagtgaaggtgggctgcttgcatcagcctaatgtcgagaagtgctttcttcggaaagtaaccctcgaaacaaattcat

SEQ ID NO: 119 - RNA, 116 nt, synthetic construct
  source 1..116: mol_type = other RNA; note = Engineered tracrRNA for CWCas12f or Un1Cas12f1 gRNA (MF/MS3-3/MS4-2)
accgcttcaccaaaagctgtcccttaggggattagaacttgagtgaaggtgggctgcttgcatcagcctaatgtcgagaagtgctttcttcggaaagtaaccctcgaaacaaattc

SEQ ID NO: 120 - RNA, 113 nt, synthetic construct
  source 1..113: mol_type = other RNA; note = Engineered tracrRNA for CWCas12f or Un1Cas12f1 gRNA (MF/MS3-3/MS4-3)
accgcttcaccaaaagctgtcccttaggggattagaacttgagtgaaggtgggctgcttgcatcagcctaatgtcgagaagtgctttcttcggaaagtaaccctcgaaacaaa

SEQ ID NO: 121 - RNA, 127 nt, synthetic construct
  source 1..127: mol_type = other RNA; note = Engineered tracrRNA for CWCas12f or Un1Cas12f1 gRNA (MF/MS4-3/MS5-1)
cttcactgataaagtggagaaccgcttcaccaaaagctgtttagattagaacttgagtgaaggtgggctgcttgcatcagcctaatgtcgagaagtgctttcttcggaaagtaaccctcgaaacaaa

SEQ ID NO: 122 - RNA, 122 nt, synthetic construct
  source 1..122: mol_type = other RNA; note = Engineered tracrRNA for CWCas12f or Un1Cas12f1 gRNA (MF/MS4-3/MS5-2)
cttcactgataaagtggagaaccgcttcaccaaaagctttagagaacttgagtgaaggtgggctgcttgcatcagcctaatgtcgagaagtgctttcttcggaaagtaaccctcgaaacaaa

SEQ ID NO: 123 - RNA, 112 nt, synthetic construct
  source 1..112: mol_type = other RNA; note = Engineered tracrRNA for CWCas12f or Un1Cas12f1 gRNA (MF/MS4-3/MS5-3)
cttcactgataaagtggagaaccgcttcaccaattagttgagtgaaggtgggctgcttgcatcagcctaatgtcgagaagtgctttcttcggaaagtaaccctcgaaacaaa

SEQ ID NO: 124 - RNA, 106 nt, synthetic construct
  source 1..106: mol_type = other RNA; note = Engineered tracrRNA for CWCas12f or Un1Cas12f1 gRNA (MF/MS4-3/MS5)
cttcactgataaagtggagaaccgcttcacttagagtgaaggtgggctgcttgcatcagcctaatgtcgagaagtgctttcttcggaaagtaaccctcgaaacaaa

SEQ ID NO: 125 - RNA, 114 nt, synthetic construct
  source 1..114: mol_type = other RNA; note = Engineered tracrRNA for TnpB or Cas12f1 gRNA (MF/MS3-3/MS5-1)
accgcttcaccaaaagctgtttagattagaacttgagtgaaggtgggctgcttgcatcagcctaatgtcgagaagtgctttcttcggaaagtaaccctcgaaacaaattcattt

SEQ ID NO: 126 - RNA, 109 nt, synthetic construct
  source 1..109: mol_type = other RNA; note = Engineered tracrRNA for CWCas12f or Un1Cas12f1 gRNA (MF/MS3-3/MS5-2)
accgcttcaccaaaagctttagagaacttgagtgaaggtgggctgcttgcatcagcctaatgtcgagaagtgctttcttcggaaagtaaccctcgaaacaaattcattt

SEQ ID NO: 127 - RNA, 99 nt, synthetic construct
  source 1..99: mol_type = other RNA; note = Engineered tracrRNA for CWCas12f or Un1Cas12f1 gRNA (MF/MS3-3/MS5-3)
accgcttcaccaattagttgagtgaaggtgggctgcttgcatcagcctaatgtcgagaagtgctttcttcggaaagtaaccctcgaaacaaattcattt

SEQ ID NO: 128 - RNA, 93 nt, synthetic construct
  source 1..93: mol_type = other RNA; note = Engineered tracrRNA for CWCas12f or Un1Cas12f1 gRNA (MF/MS3-3/MS5)
accgcttcacttagagtgaaggtgggctgcttgcatcagcctaatgtcgagaagtgctttcttcggaaagtaaccctcgaaacaaattcattt

SEQ ID NO: 129 - RNA, 92 nt, synthetic construct
  source 1..92: mol_type = other RNA; note = Engineered tracrRNA for CWCas12f or Un1Cas12f1 gRNA (MF/MS3-3/MS4-3/MS5-3)
accgcttcaccaattagttgagtgaaggtgggctgcttgcatcagcctaatgtcgagaagtgctttcttcggaaagtaaccctcgaaacaaa

SEQ ID NO: 130 - RNA, 91 nt, synthetic construct
  source 1..91: mol_type = other RNA; note = Engineered tracrRNA for CWCas12f or Un1Cas12f1 gRNA (MF/MS3-3/MS4-1/MS5)
accgcttcacttagagtgaaggtgggctgcttgcatcagcctaatgtcgagaagtgctttcttcggaaagtaaccctcgaaacaaattcat

SEQ ID NO: 131 - RNA, 89 nt, synthetic construct
  source 1..89: mol_type = other RNA; note = Engineered tracrRNA for CWCas12f or Un1Cas12f1 gRNA (MF/MS3-3/MS4-2/MS5)
accgcttcacttagagtgaaggtgggctgcttgcatcagcctaatgtcgagaagtgctttcttcggaaagtaaccctcgaaacaaattc

SEQ ID NO: 132 - RNA, 86 nt, synthetic construct
  source 1..86: mol_type = other RNA; note = Engineered tracrRNA for CWCas12f or Un1Cas12f1 gRNA (MF/MS3-3/MS4-3/MS5)
accgcttcacttagagtgaaggtgggctgcttgcatcagcctaatgtcgagaagtgctttcttcggaaagtaaccctcgaaacaaa

SEQ ID NO: 133 - RNA, 37 nt, synthetic construct
  source 1..37: mol_type = other RNA; note = Engineered crRNA for CWCas12f or Un1Cas12f1 gRNA (MS1)
gttgcagaacccgaatagagcaatgaaggaatgcaac

SEQ ID NO: 134 - RNA, 31 nt, synthetic construct
  source 1..31: mol_type = other RNA; note = Engineered crRNA for CWCas12f or Un1Cas12f1 gRNA (MS1/MS4*-1)
gaacccgaatagagcaatgaaggaatgcaac

SEQ ID NO: 135 - RNA, 25 nt, synthetic construct
  source 1..25: mol_type = other RNA; note = Engineered crRNA for CWCas12f or Un1Cas12f1 gRNA (MS1/MS4*-2)
gaatagagcaatgaaggaatgcaac

SEQ ID NO: 136 - RNA, 19 nt, synthetic construct
  source 1..19: mol_type = other RNA; note = Engineered crRNA for CWCas12f or Un1Cas12f1 gRNA (MS1/MS4*-3)
agcaatgaaggaatgcaac

SEQ ID NO: 137 - RNA, 17 nt, synthetic construct
  source 1..17: mol_type = other RNA; note = Engineered crRNA for CWCas12f or Un1Cas12f1 gRNA (MF)
gaatgaaggaatgcaac

SEQ ID NO: 138 - RNA, 15 nt, synthetic construct
  source 1..15: mol_type = other RNA; note = Engineered crRNA for CWCas12f or Un1Cas12f1 gRNA (MF/MS4-1)
atgaaggaatgcaac

SEQ ID NO: 139 - RNA, 13 nt, synthetic construct
  source 1..13: mol_type = other RNA; note = Engineered crRNA for CWCas12f or Un1Cas12f1 gRNA (MF/MS4-2)
gaaggaatgcaac

SEQ ID NO: 140 - RNA, 10 nt, synthetic construct
  source 1..10: mol_type = other RNA; note = Engineered crRNA for CWCas12f or Un1Cas12f1 gRNA (MF/MS4-3)
ggaatgcaac

SEQ ID NO: 141 - RNA, 68 nt, synthetic construct
  source 1..68: mol_type = other RNA; note = Engineered crRNA for CWCas12f or Un1Cas12f1 gRNA (MS1/MS2)
  misc_feature 38..57: note = n is a, c, g or u
gttgcagaacccgaatagagcaatgaaggaatgcaacnnnnnnnnnnnnnnnnnnnnttttatttttt

SEQ ID NO: 142 - RNA, 62 nt, synthetic construct
  source 1..62: mol_type = other RNA; note = Engineered crRNA for CWCas12f or Un1Cas12f1 gRNA (MS1/MS2/MS4*-1)
  misc_feature 32..51: note = n is a, c, g or u
gaacccgaatagagcaatgaaggaatgcaacnnnnnnnnnnnnnnnnnnnnttttatttttt

SEQ ID NO: 143 - RNA, 56 nt, synthetic construct
  source 1..56: mol_type = other RNA; note = Engineered crRNA for CWCas12f or Un1Cas12f1 gRNA (MS1/MS2/MS4*-2)
  misc_feature 26..45: note = n is a, c, g or u
gaatagagcaatgaaggaatgcaacnnnnnnnnnnnnnnnnnnnnttttatttttt

SEQ ID NO: 144 - RNA, 50 nt, synthetic construct
  source 1..50: mol_type = other RNA; note = Engineered crRNA for CWCas12f or Un1Cas12f1 gRNA (MS1/MS2/MS4*-3)
  misc_feature 20..39: note = n is a, c, g or u
agcaatgaaggaatgcaacnnnnnnnnnnnnnnnnnnnnttttatttttt

SEQ ID NO: 145 - RNA, 48 nt, synthetic construct
  source 1..48: mol_type = other RNA; note = Engineered crRNA for CWCas12f or Un1Cas12f1 gRNA (MF/MS2)
  misc_feature 18..37: note = n is a, c, g or u
gaatgaaggaatgcaacnnnnnnnnnnnnnnnnnnnnttttatttttt

SEQ ID NO: 146 - RNA, 46 nt, synthetic construct
  source 1..46: mol_type = other RNA; note = Engineered crRNA for CWCas12f or Un1Cas12f1 gRNA (MF/MS2/MS4-1)
  misc_feature 16..35: note = n is a, c, g or u
atgaaggaatgcaacnnnnnnnnnnnnnnnnnnnnttttatttttt

SEQ ID NO: 147 - RNA, 44 nt, synthetic construct
  source 1..44: mol_type = other RNA; note = Engineered crRNA for CWCas12f or Un1Cas12f1 gRNA (MF/MS2/MS4-2)
  misc_feature 14..33: note = n is a, c, g or u
gaaggaatgcaacnnnnnnnnnnnnnnnnnnnnttttatttttt

SEQ ID NO: 148 - RNA, 41 nt, synthetic construct
  source 1..41: mol_type = other RNA; note = Engineered crRNA for CWCas12f or Un1Cas12f1 gRNA (MF/MS2/MS4-3)
  misc_feature 11..30: note = n is a, c, g or u
ggaatgcaacnnnnnnnnnnnnnnnnnnnnttttatttttt

SEQ ID NO: 149 - RNA, 222 nt, synthetic construct
  source 1..222: mol_type = other RNA; note = Engineered sgRNA with modification of MS1 for CWCas12f or Un1Cas12f1
  misc_feature 203..222: note = n is a, c, g or u
cttcactgataaagtggagaaccgcttcaccaaaagctgtcccttaggggattagaacttgagtgaaggtgggctgcttgcatcagcctaatgtcgagaagtgctttcttcggaaagtaaccctcgaaacaaattcagtgctcctctccaattctgcacaagaaagttgcagaacccgaatagagcaatgaaggaatgcaacnnnnnnnnnnnnnnnnnnnn

SEQ ID NO: 150 - RNA, 233 nt, synthetic construct
  source 1..233: mol_type = other RNA; note = Engineered sgRNA with modification of MS1/MS2 for CWCas12f or Un1Cas12f1
  misc_feature 203..222: note = n is a, c, g or u
cttcactgataaagtggagaaccgcttcaccaaaagctgtcccttaggggattagaacttgagtgaaggtgggctgcttgcatcagcctaatgtcgagaagtgctttcttcggaaagtaaccctcgaaacaaattcagtgctcctctccaattctgcacaagaaagttgcagaacccgaatagagcaatgaaggaatgcaacnnnnnnnnnnnnnnnnnnnnttttatttttt

SEQ ID NO: 151 - RNA, 213 nt, synthetic construct
  source 1..213: mol_type = other RNA; note = Engineered sgRNA with modification of MS1/MS2/MS3 for CWCas12f or Un1Cas12f1
  misc_structure 183..202: note = n is a, c, g or u
accgcttcaccaaaagctgtcccttaggggattagaacttgagtgaaggtgggctgcttgcatcagcctaatgtcgagaagtgctttcttcggaaagtaaccctcgaaacaaattcagtgctcctctccaattctgcacaagaaagttgcagaacccgaatagagcaatgaaggaatgcaacnnnnnnnnnnnnnnnnnnnnttttatttttt

SEQ ID NO: 152 - RNA, 158 nt, synthetic construct
  source 1..158: mol_type = other RNA; note = Engineered sgRNA with modification of MS2/MS3/MS4 for CWCas12f or Un1Cas12f1
  misc_feature 128..147: note = n is a, c, g or u
accgcttcaccaaaagctgtcccttaggggattagaacttgagtgaaggtgggctgcttgcatcagcctaatgtcgagaagtgctttcttcggaaagtaaccctcgaaacaaagaaaggaatgcaacnnnnnnnnnnnnnnnnnnnnttttatttttt

SEQ ID NO: 153 - RNA, 131 nt, synthetic construct
  source 1..131: mol_type = other RNA; note = Engineered sgRNA with modification of MS2/MS3/MS4/MS5 for CWCas12f or Un1Cas12f1
  misc_feature 99..118: note = n is a, c, g or u
accgcttcacttagagtgaaggtgggctgcttgcatcagcctaatgtcgagaagtgctttcttcggaaagtaaccctcgaaacaaagaaaggaatgcaacnnnnnnnnnnnnnnnnnnnnttttatttttt

SEQ ID NO: 154 - RNA, 215 nt, synthetic construct
  source 1..215: mol_type = other RNA; note = Engineered sgRNA with modification of MS1/MS3-1 for CWCas12f or Un1Cas12f1
  misc_feature 196..215: note = n is a, c, g or u
gataaagtggagaaccgcttcaccaaaagctgtcccttaggggattagaacttgagtgaaggtgggctgcttgcatcagcctaatgtcgagaagtgctttcttcggaaagtaaccctcgaaacaaattcagtgctcctctccaattctgcacaagaaagttgcagaacccgaatagagcaatgaaggaatgcaacnnnnnnnnnnnnnnnnnnnn

SEQ ID NO: 155 - RNA, 208 nt, synthetic construct
  source 1..208: mol_type = other RNA; note = Engineered sgRNA with modification of MS1/MS3-2 for CWCas12f or Un1Cas12f1
  misc_feature 189..208: note = n is a, c, g or u
tggagaaccgcttcaccaaaagctgtcccttaggggattagaacttgagtgaaggtgggctgcttgcatcagcctaatgtcgagaagtgctttcttcggaaagtaaccctcgaaacaaattcagtgctcctctccaattctgcacaagaaagttgcagaacccgaatagagcaatgaaggaatgcaacnnnnnnnnnnnnnnnnnnnn

SEQ ID NO: 156 - RNA, 202 nt, synthetic construct
  source 1..202: mol_type = other RNA; note = Engineered sgRNA with modification of MS1/MS3-3 for CWCas12f or Un1Cas12f1
  misc_feature 183..202: note = n is a, c, g or u
accgcttcaccaaaagctgtcccttaggggattagaacttgagtgaaggtgggctgcttgcatcagcctaatgtcgagaagtgctttcttcggaaagtaaccctcgaaacaaattcagtgctcctctccaattctgcacaagaaagttgcagaacccgaatagagcaatgaaggaatgcaacnnnnnnnnnnnnnnnnnnnn

SEQ ID NO: 157 - RNA, 209 nt, synthetic construct
  source 1..209: mol_type = other RNA; note = Engineered sgRNA with modification of MS1/MS4*-1 for CWCas12f or Un1Cas12f1
  misc_feature 190..209: note = n is a, c, g or u
cttcactgataaagtggagaaccgcttcaccaaaagctgtcccttaggggattagaacttgagtgaaggtgggctgcttgcatcagcctaatgtcgagaagtgctttcttcggaaagtaaccctcgaaacaaattcagtgctcctctccaattcgaaagaacccgaatagagcaatgaaggaatgcaacnnnnnnnnnnnnnnnnnnnn

SEQ ID NO: 158 - RNA, 197 nt, synthetic construct
  source 1..197: mol_type = other RNA; note = Engineered sgRNA with modification of MS1/MS4*-2 for CWCas12f or Un1Cas12f1
  misc_feature 178..197: note = n is a, c, g or u
cttcactgataaagtggagaaccgcttcaccaaaagctgtcccttaggggattagaacttgagtgaaggtgggctgcttgcatcagcctaatgtcgagaagtgctttcttcggaaagtaaccctcgaaacaaattcagtgctcctctcgaaagaatagagcaatgaaggaatgcaacnnnnnnnnnnnnnnnnnnnn

SEQ ID NO: 159 - RNA, 185 nt, synthetic construct
  source 1..185: mol_type = other RNA; note = Engineered sgRNA with modification of MS1/MS4*-3 for CWCas12f or Un1Cas12f1
  misc_feature 166..185: note = n is a, c, g or u
cttcactgataaagtggagaaccgcttcaccaaaagctgtcccttaggggattagaacttgagtgaaggtgggctgcttgcatcagcctaatgtcgagaagtgctttcttcggaaagtaaccctcgaaacaaattcagtgctgaaaagcaatgaaggaatgcaacnnnnnnnnnnnnnnnnnnnn

SEQ ID NO: 160 - RNA, 216 nt, synthetic construct
  source 1..216: mol_type = other RNA; note = Engineered sgRNA with modification of MS1/MS5-1 for CWCas12f or Un1Cas12f1
  misc_feature 197..216: note = n is a, c, g or u
cttcactgataaagtggagaaccgcttcaccaaaagctgtttagattagaacttgagtgaaggtgggctgcttgcatcagcctaatgtcgagaagtgctttcttcggaaagtaaccctcgaaacaaattcagtgctcctctccaattctgcacaagaaagttgcagaacccgaatagagcaatgaaggaatgcaacnnnnnnnnnnnnnnnnnnnn

SEQ ID NO: 161 - RNA, 209 nt, synthetic construct
  source 1..209: mol_type = other RNA; note = Engineered sgRNA with modification of MS1/MS5-2 for CWCas12f or Un1Cas12f1
  misc_feature 190..209: note = n is a, c, g or u
cttcactgataaagtggagaaccgcttcaccaaaagcttaggaacttgagtgaaggtgggctgcttgcatcagcctaatgtcgagaagtgctttcttcggaaagtaaccctcgaaacaaattcagtgctcctctccaattctgcacaagaaagttgcagaacccgaatagagcaatgaaggaatgcaacnnnnnnnnnnnnnnnnnnnn

SEQ ID NO: 162 - RNA, 201 nt, synthetic construct
  source 1..201: mol_type = other RNA; note = Engineered sgRNA with modification of MS1/MS5-3 for CWCas12f or Un1Cas12f1
  misc_feature 182..201: note = n is a, c, g or u
cttcactgataaagtggagaaccgcttcaccaattagttgagtgaaggtgggctgcttgcatcagcctaatgtcgagaagtgctttcttcggaaagtaaccctcgaaacaaattcagtgctcctctccaattctgcacaagaaagttgcagaacccgaatagagcaatgaaggaatgcaacnnnnnnnnnnnnnnnnnnnn

SEQ ID NO: 163 - RNA, 206 nt, synthetic construct
  source 1..206: mol_type = other RNA; note = Engineered sgRNA with modification of MS1/MS2/MS4*-2 for CWCas12f or Un1Cas12f1
  misc_feature 178..197: note = n is a, c, g or u
cttcactgataaagtggagaaccgcttcaccaaaagctgtcccttaggggattagaacttgagtgaaggtgggctgcttgcatcagcctaatgtcgagaagtgctttcttcggaaagtaaccctcgaaacaaattcagtgctcctctcgaaagaatagagcaatgaaggaatgcaacnnnnnnnnnnnnnnnnnnnnttttatttt

SEQ ID NO: 164 - RNA, 177 nt, synthetic construct
  source 1..177: mol_type = other RNA; note = Engineered sgRNA with modification of MS1/MS3-3/MS4*-2 for CWCas12f or Un1Cas12f1
  misc_feature 158..177: note = n is a, c, g or u
accgcttcaccaaaagctgtcccttaggggattagaacttgagtgaaggtgggctgcttgcatcagcctaatgtcgagaagtgctttcttcggaaagtaaccctcgaaacaaattcagtgctcctctcgaaagaatagagcaatgaaggaatgcaacnnnnnnnnnnnnnnnnnnnn

SEQ ID NO: 165 - RNA, 210 nt, synthetic construct
  source 1..210: mol_type = other RNA; note = Engineered sgRNA with modification of MS1/MS2/MS5-3 for CWCas12f or Un1Cas12f1
  misc_feature 182..201: note = n is a, c, g or u
cttcactgataaagtggagaaccgcttcaccaattagttgagtgaaggtgggctgcttgcatcagcctaatgtcgagaagtgctttcttcggaaagtaaccctcgaaacaaattcagtgctcctctccaattctgcacaagaaagttgcagaacccgaatagagcaatgaaggaatgcaacnnnnnnnnnnnnnnnnnnnnttttatttt

SEQ ID NO: 166 - RNA, 181 nt, synthetic construct
  source 1..181: mol_type = other RNA; note = Engineered sgRNA with modification of MS1/MS3-3/MS5-3 for CWCas12f or Un1Cas12f1
  misc_feature 162..181: note = n is a, c, g or u
accgcttcaccaattagttgagtgaaggtgggctgcttgcatcagcctaatgtcgagaagtgctttcttcggaaagtaaccctcgaaacaaattcagtgctcctctccaattctgcacaagaaagttgcagaacccgaatagagcaatgaaggaatgcaacnnnnnnnnnnnnnnnnnnnn

SEQ ID NO: 167 - RNA, 176 nt, synthetic construct
  source 1..176: mol_type = other RNA; note = Engineered sgRNA with modification of MS1/MS4*-2/MS5-3 for CWCas12f or Un1Cas12f1
  misc_feature 157..176: note = n is a, c, g or u
cttcactgataaagtggagaaccgcttcaccaattagttgagtgaaggtgggctgcttgcatcagcctaatgtcgagaagtgctttcttcggaaagtaaccctcgaaacaaattcagtgctcctctcgaaagaatagagcaatgaaggaatgcaacnnnnnnnnnnnnnnnnnnnn

SEQ ID NO: 168 - RNA, 186 nt, synthetic construct
  source 1..186: mol_type = other RNA; note = Engineered sgRNA with modification of MS1/MS2/MS3-3/MS4*-2 for CWCas12f or Un1Cas12f1
  misc_feature 158..177: note = n is a, c, g or u
accgcttcaccaaaagctgtcccttaggggattagaacttgagtgaaggtgggctgcttgcatcagcctaatgtcgagaagtgctttcttcggaaagtaaccctcgaaacaaattcagtgctcctctcgaaagaatagagcaatgaaggaatgcaacnnnnnnnnnnnnnnnnnnnnttttatttt

SEQ ID NO: 169 - RNA, 190 nt, synthetic construct
  source 1..190: mol_type = other RNA; note = Engineered sgRNA with modification of MS1/MS2/MS3-3/MS5-3 for CWCas12f or Un1Cas12f1
  misc_feature 162..181: note = n is a, c, g or u
accgcttcaccaattagttgagtgaaggtgggctgcttgcatcagcctaatgtcgagaagtgctttcttcggaaagtaaccctcgaaacaaattcagtgctcctctccaattctgcacaagaaagttgcagaacccgaatagagcaatgaaggaatgcaacnnnnnnnnnnnnnnnnnnnnttttatttt

SEQ ID NO: 170 - RNA, 185 nt, synthetic construct
  source 1..185: mol_type = other RNA; note = Engineered sgRNA with modification of MS1/MS2/MS4*-2/MS5-3 for CWCas12f or Un1Cas12f1
  misc_feature 157..176: note = n is a, c, g or u
cttcactgataaagtggagaaccgcttcaccaattagttgagtgaaggtgggctgcttgcatcagcctaatgtcgagaagtgctttcttcggaaagtaaccctcgaaacaaattcagtgctcctctcgaaagaatagagcaatgaaggaatgcaacnnnnnnnnnnnnnnnnnnnnttttatttt

SEQ ID NO: 171 - RNA, 156 nt, synthetic construct
  source 1..156: mol_type = other RNA; note = Engineered sgRNA with modification of MS1/MS3-3/MS4*-2/MS5-3 for CWCas12f or Un1Cas12f1
  misc_feature 137..156: note = n is a, c, g or u
accgcttcaccaattagttgagtgaaggtgggctgcttgcatcagcctaatgtcgagaagtgctttcttcggaaagtaaccctcgaaacaaattcagtgctcctctcgaaagaatagagcaatgaaggaatgcaacnnnnnnnnnnnnnnnnnnnn

SEQ ID NO: 172 - RNA, 165 nt, synthetic construct
  source 1..165: mol_type = other RNA; note = Engineered sgRNA with modification of MS1/MS2/MS3-3/MS4*-2/MS5-3 for CWCas12f or Un1Cas12f1
  misc_feature 137..156: note = n is a, c, g or u
accgcttcaccaattagttgagtgaaggtgggctgcttgcatcagcctaatgtcgagaagtgctttcttcggaaagtaaccctcgaaacaaattcagtgctcctctcgaaagaatagagcaatgaaggaatgcaacnnnnnnnnnnnnnnnnnnnnttttatttt

SEQ ID NO: 173 - RNA, 181 nt, synthetic construct
  source 1..181: mol_type = other RNA; note = Mature form sgRNA for CWCas12f or Un1Cas12f1
  misc_feature 162..181: note = n is a, c, g or u
cttcactgataaagtggagaaccgcttcaccaaaagctgtcccttaggggattagaacttgagtgaaggtgggctgcttgcatcagcctaatgtcgagaagtgctttcttcggaaagtaaccctcgaaacaaattcatttgaaagaatgaaggaatgcaacnnnnnnnnnnnnnnnnnnnn

SEQ ID NO: 174 - RNA, 174 nt, synthetic construct
  source 1..174: mol_type = other RNA; note = Mature form sgRNA with modification of MS3-1 for CWCas12f or Un1Cas12f1
  misc_feature 155..174: note = n is a, c, g or u
gataaagtggagaaccgcttcaccaaaagctgtcccttaggggattagaacttgagtgaaggtgggctgcttgcatcagcctaatgtcgagaagtgctttcttcggaaagtaaccctcgaaacaaattcatttgaaagaatgaaggaatgcaacnnnnnnnnnnnnnnnnnnnn

SEQ ID NO: 175 - RNA, 167 nt, synthetic construct
  source 1..167: mol_type = other RNA; note = Mature form sgRNA with modification of MS3-2 for CWCas12f or Un1Cas12f1
  misc_feature 148..167: note = n is a, c, g or u
tggagaaccgcttcaccaaaagctgtcccttaggggattagaacttgagtgaaggtgggctgcttgcatcagcctaatgtcgagaagtgctttcttcggaaagtaaccctcgaaacaaattcatttgaaagaatgaaggaatgcaacnnnnnnnnnnnnnnnnnnnn

SEQ ID NO: 176 - RNA, 161 nt, synthetic construct
  source 1..161: mol_type = other RNA; note = Mature form sgRNA with modification of MS3-3 for CWCas12f or Un1Cas12f1
  misc_feature 142..161: note = n is a, c, g or u
accgcttcaccaaaagctgtcccttaggggattagaacttgagtgaaggtgggctgcttgcatcagcctaatgtcgagaagtgctttcttcggaaagtaaccctcgaaacaaattcatttgaaagaatgaaggaatgcaacnnnnnnnnnnnnnnnnnnnn

SEQ ID NO: 177 - RNA, 177 nt, synthetic construct
  source 1..177: mol_type = other RNA; note = Mature form sgRNA with modification of MS4-1 for CWCas12f or Un1Cas12f1
  misc_feature 158..177: note = n is a, c, g or u
cttcactgataaagtggagaaccgcttcaccaaaagctgtcccttaggggattagaacttgagtgaaggtgggctgcttgcatcagcctaatgtcgagaagtgctttcttcggaaagtaaccctcgaaacaaattcatgaaaatgaaggaatgcaacnnnnnnnnnnnnnnnnnnnn

SEQ ID NO: 178 - RNA, 173 nt, synthetic construct
  source 1..173: mol_type = other RNA; note = Mature form sgRNA with modification of MS4-2 for CWCas12f or Un1Cas12f1
  misc_feature 154..173: note = n is a, c, g or u
cttcactgataaagtggagaaccgcttcaccaaaagctgtcccttaggggattagaacttgagtgaaggtgggctgcttgcatcagcctaatgtcgagaagtgctttcttcggaaagtaaccctcgaaacaaattcgaaagaaggaatgcaacnnnnnnnnnnnnnnnnnnnn

SEQ ID NO: 179 - RNA, 167 nt, synthetic construct
  source 1..167: mol_type = other RNA; note = Mature form sgRNA with modification of MS4-3 for CWCas12f or Un1Cas12f1
  misc_feature 148..167: note = n is a, c, g or u
cttcactgataaagtggagaaccgcttcaccaaaagctgtcccttaggggattagaacttgagtgaaggtgggctgcttgcatcagcctaatgtcgagaagtgctttcttcggaaagtaaccctcgaaacaaagaaaggaatgcaacnnnnnnnnnnnnnnnnnnnn

SEQ ID NO: 180 - RNA, 175 nt, synthetic construct
  source 1..175: mol_type = other RNA; note = Mature form sgRNA with modification of MS5-1 for CWCas12f or Un1Cas12f1
  misc_feature 156..175: note = n is a, c, g or u
cttcactgataaagtggagaaccgcttcaccaaaagctgtttagattagaacttgagtgaaggtgggctgcttgcatcagcctaatgtcgagaagtgctttcttcggaaagtaaccctcgaaacaaattcatttgaaagaatgaaggaatgcaacnnnnnnnnnnnnnnnnnnnn

SEQ ID NO: 181 - RNA, 170 nt, synthetic construct
  source 1..170: mol_type = other RNA; note = Mature form sgRNA with modification of MS5-2 for CWCas12f or Un1Cas12f1
  misc_feature 151..170: note = n is a, c, g or u
cttcactgataaagtggagaaccgcttcaccaaaagctttagagaacttgagtgaaggtgggctgcttgcatcagcctaatgtcgagaagtgctttcttcggaaagtaaccctcgaaacaaattcatttgaaagaatgaaggaatgcaacnnnnnnnnnnnnnnnnnnnn

SEQ ID NO: 182 - RNA, 160 nt, synthetic construct
  source 1..160: mol_type = other RNA; note = Mature form sgRNA with modification of MS5-3 for CWCas12f or Un1Cas12f1
  misc_feature 141..160: note = n is a, c, g or u
cttcactgataaagtggagaaccgcttcaccaattagttgagtgaaggtgggctgcttgcatcagcctaatgtcgagaagtgctttcttcggaaagtaaccctcgaaacaaattcatttgaaagaatgaaggaatgcaacnnnnnnnnnnnnnnnnnnnn

SEQ ID NO: 183 - RNA, 147 nt, synthetic construct
  source 1..147: mol_type = other RNA; note = Mature form sgRNA with modification of MS3-3/MS4-3 for CWCas12f or Un1Cas12f1
  misc_feature 128..147: note = n is a, c, g or u
accgcttcaccaaaagctgtcccttaggggattagaacttgagtgaaggtgggctgcttgcatcagcctaatgtcgagaagtgctttcttcggaaagtaaccctcgaaacaaagaaaggaatgcaacnnnnnnnnnnnnnnnnnnnn

SEQ ID NO: 184 - RNA, 140 nt, synthetic construct
  source 1..140: mol_type = other RNA; note = Mature form sgRNA with modification of MS3-3/MS5-3 for CWCas12f or Un1Cas12f1
  misc_feature 121..140: note = n is a, c, g or u
accgcttcaccaattagttgagtgaaggtgggctgcttgcatcagcctaatgtcgagaagtgctttcttcggaaagtaaccctcgaaacaaattcatttgaaagaatgaaggaatgcaacnnnnnnnnnnnnnnnnnnnn

SEQ ID NO: 185 - RNA, 146 nt, synthetic construct
  source 1..146: mol_type = other RNA; note = Mature form sgRNA with modification of MS4-3/MS5-3 for CWCas12f or Un1Cas12f1
  misc_feature 127..146: note = n is a, c, g or u
cttcactgataaagtggagaaccgcttcaccaattagttgagtgaaggtgggctgcttgcatcagcctaatgtcgagaagtgctttcttcggaaagtaaccctcgaaacaaagaaaggaatgcaacnnnnnnnnnnnnnnnnnnnn

SEQ ID NO: 186 - RNA, 126 nt, synthetic construct
  source 1..126: mol_type = other RNA; note = Mature form sgRNA with modification of MS3-3/MS4-3/MS5-3 for CWCas12f or Un1Cas12f1
  misc_feature 107..126: note = n is a, c, g or u
accgcttcaccaattagttgagtgaaggtgggctgcttgcatcagcctaatgtcgagaagtgctttcttcggaaagtaaccctcgaaacaaagaaaggaatgcaacnnnnnnnnnnnnnnnnnnnn

SEQ ID NO: 187 - RNA, 10 nt, synthetic construct
  source 1..10: mol_type = other RNA; note = The additional sequence for CWCas12f or Un1Cas12f1 gRNA
ataaaggtga

SEQ ID NO: 188 - RNA, 37 nt, synthetic construct
  source 1..37: mol_type = other RNA; note = The additional sequence for CWCas12f or Un1Cas12f1 gRNA
ctgatgagtccgtgaggacgaaacgagtaagctcgtc

SEQ ID NO: 189 - RNA, 37 nt, synthetic construct
  source 1..37: mol_type = other RNA; note = The additional sequence for CWCas12f or Un1Cas12f1 gRNA
ctgctcgaatgagcaaagcaggagtgcctgagtagtc

SEQ ID NO: 190 - protein, 249 aa, synthetic construct
  source 1..249: note = N-term 249aa extension
MVSKGEELFTGVVPILVELDGDVNGHKFSVSGEGEGDATYGKLTLKFICTTGKLPVPWPTLVTTLTYGVQCFSRYPDHMKQHDFFKSAMPEGYVQERTIFFKDDGNYKTRAEVKFEGDTLVNRIELKGIDFKEDGNILGHKLEYNYNSHNVYIMADKQKNGIKVNFKIRHNIEDGSVQLADHYQQNTPIGDGPVLLPDNHYLSTQSALSKDPNEKRDHMVLLEFVTAAGITLGMDELYKSGLRSRAQAL

SEQ ID NO: 191 - protein, 248 aa, synthetic construct
  source 1..248: note = C-term 248aa extension
RARDPPVATMVSKGEELFTGVVPILVELDGDVNGHKFSVSGEGEGDATYGKLTLKFICTTGKLPVPWPTLVTTLTYGVQCFSRYPDHMKQHDFFKSAMPEGYVQERTIFFKDDGNYKTRAEVKFEGDTLVNRIELKGIDFKEDGNILGHKLEYNYNSHNVYIMADKQKNGIKVNFKIRHNIEDGSVQLADHYQQNTPIGDGPVLLPDNHYLSTQSALSKDPNEKRDHMVLLEFVTAAGITLGMDELYK

SEQ ID NO: 192 - DNA, 20 bp, synthetic construct
  source 1..20: mol_type = other DNA; note = PAM library-protospacer
cacacacacagtgggctacc

SEQ ID NO: 193 - DNA, 34 bp, synthetic construct
  source 1..34: mol_type = other DNA; note = PAM library-adaptor DNA
agatcggaagagcacacgtctgaactccagtcac

SEQ ID NO: 194 - DNA, 17 bp, synthetic construct
  source 1..17: mol_type = other DNA; note = PAM library-primer (forward)
gtaaaacgacggccagt

SEQ ID NO: 195 - DNA, 13 bp, synthetic construct
  source 1..13: mol_type = other DNA; note = PAM library-primer (reverse)
gtgactggagttc

SEQ ID NO: 196 - DNA, 100 bp, synthetic construct
  source 1..100: mol_type = other DNA; note = PAM modifying oligonucleotide (donor DNA)
  misc_feature 47..50: note = n is a, c, g or t
aggctgttgtcaaatgtctgataatcctgcactgtcctcttcacatnnnngagggagacacaagttgatagggagttctgtgtgtctaagggaggcggtg

SEQ ID NO: 197 - DNA, 2910 bp, synthetic construct
  source 1..2910: mol_type = other DNA; note = TaRGET-ABE-N1
atgtccgaagtcgagttttcccatgagtactggatgagacacgcattgactctcgcaaagagggcttgggatgaacgcgaggtgcccgtgggggcagtactcgtgcataacaatcgcgtaatcggcgaaggttggaataggccgatcggacgccacgaccccactgcacatgcggaaatcatggcccttcgacagggagggcttgtgatgcagaattatcgacttatcgatgcgacgctgtacgtcacgcttgaaccttgcgtaatgtgcgcgggagctatgattcactcccgcattggacgagttgtattcggtgcccgcgacgccaagacgggtgccgcaggttcactgatggacgtgctgcatcacccaggcatgaaccaccgggtagaaatcacagaaggcatattggcggacgaatgtgcggcgctgttgtccgacttttttcgcatgcggaggcaggagatcaaggcccagaaaaaagcacaatcctctactgactctggtggttcttctggtggttctagcggcagcgagactcccgggacctcagagtccgccacacccgaaagttcaggtggatcttcaggtggatcttcggaagtggaattttcgcacgagtattggatgaggcacgctttaactctcgctaagagagcacgagacgaacgggaagtgccggttggggctgtcctcgtactcaataatcgagttatcggagaaggctggaacagggcaatcggactccacgatcccacagctcatgccgagataatggcgcttcgacaaggaggcctagtcatgcaaaattatcgtcttattgacgcgaccctctacgtgacctttgagccatgcgttatgtgtgcgggtgcaatgatacattcccggataggacgtgtagtatttggagttcgcaacgcgaagaccggtgcggctggttctctcatggatgtcctgcactaccctgggatgaatcaccgcgttgaaatcactgaaggcattttggccgatgaatgcgcggccctgttatgttacttttttcgcatgcccaggcaggtctttaacgcacagaagaaagcccaatcgtccactgattctggtggctcttcaggtggatcaagcgggagtgagacaccagggacctcggagtccgctacaccggagagttcaggcggttcatcaggtggatctatgggggagaaaagttcccgccgccgacggaatggaaaaagcggtgcgtggactgctgctataacaagctgtgttgggggtaagatggccaagaacacaattacaaagacactgaagctgaggatcgtgagaccatacaacagcgctgaggtcgagaagattgtggctgatgaaaagaacaacagggaaaagatcgccctcgagaagaacaaggataaggtgaaggaggcctgctctaagcacctgaaagtggccgcctactgcaccacacaggtggagaggaacgcctgtctgttttgtaaagctcggaagctggatgataagttttaccagaagctgcggggccagttccccgatgccgtcttttggcaggagattagcgagatcttcagacagctgcagaagcaggccgccgagatctacaaccagagcctgatcgagctctactacgagatcttcatcaagggcaagggcattgccaacgcctcctccgtggagcactacctgagcgacgtgtgctacacaagagccgccgagctctttaagaacgccgctatcgcttccgggctgaggagcaagattaagagtaacttccggctcaaggagctgaagaacatgaagagcggcctgcccactacaaagagcgacaacttcccaattccactggtgaagcagaaggggggccagtacacagggttcgagatttccaaccacaacagcgactttattattaagatcccctttggcaggtggcaggtcaagaaggagattgacaagtacaggccctgggagaagtttgatttcgagcaggtgcagaagagccccaagcctatttccctgctgctgtccacacagcggcggaagaggaacaaggggtggtctaaggatgaggggaccgaggccgagattaagaaagtgatgaacggcgactaccagacaagctacatcgaggtcaagcggggcagtaagattggcgagaagagcgcctggatgctgaacctgagcattgacgtgccaaagattgataagggcgtggatcccagcatcatcggagggatcgctgtgggggtcaagagccccctcgtgtgcgccatcaacaacgccttcagcaggtacagcatctccgataacgacctgttccactttaacaagaagatgttcgcccggcggaggattttgctcaagaagaaccggcacaagcgggccggacacggggccaagaacaagctcaagcccatcactatcctgaccgagaagagcgagaggttcaggaagaagctcatcgagagatgggcctgcgagatcgccgatttctttattaagaacaaggtcggaacagtgcagatggagaacctcgagagcatgaagaggaaggaggattcctacttcaacattcggctgagggggttctggccctacgctgagatgcagaacaagattgagtttaagctgaagcagtacgggattgagatccggaaggtggcccccaacaacaccagcaagacctgcagcaagtgcgggcacctcaacaactacttcaacttcgagtaccggaagaagaacaagttcccacacttcaagtgcgagaagtgcaactttaaggagaacgccgattacaacgccgccctgaacatcagcaaccctaagctgaagagcactaaggaggagcccaaaaggccggcggccacgaaaaaggccggccaggcaaaaaagaaaaag

SEQ ID NO: 198 - DNA, 2910 bp, synthetic construct
  source 1..2910: mol_type = other DNA; note = TaRGET-ABE-N2
atgtccgaagtcgagttttcccatgagtactggatgagacacgcattgactctcgcaaagagggctcgagatgaacgcgaggtgcccgtgggggcagtactcgtgctcaacaatcgcgtaatcggcgaaggttggaatagggcaatcggactccacgaccccactgcacatgcggaaatcatggcccttcgacagggagggcttgtgatgcagaattatcgacttatcgatgcgacgctgtacgtcacgtttgaaccttgcgtaatgtgcgcgggagctatgattcactcccgcattggacgagttgtattcggtgttcgcaacgccaagacgggtgccgcaggttcactgatggacgtgctgcattacccaggcatgaaccaccgggtagaaatcacagaaggcatattggcggacgaatgtgcggcgctgttgtgttacttttttcgcatgcccaggcaggtctttaacgcccagaaaaaagcacaatcctctactgactctggtggttcttctggtggttctagcggcagcgagactcccgggacctcagagtccgccacacccgaaagttctggtggttcttctggtggttcttccgaagtcgagttttcccatgagtactggatgagacacgcattgactctcgcaaagagggcttgggatgaacgcgaggtgcccgtgggggcagtactcgtgcataacaatcgcgtaatcggcgaaggttggaataggccgatcggacgccacgaccccactgcacatgcggaaatcatggcccttcgacagggagggcttgtgatgcagaattatcgacttatcgatgcgacgctgtacgtcacgcttgaaccttgcgtaatgtgcgcgggagctatgattcactcccgcattggacgagttgtattcggtgcccgcgacgccaagacgggtgccgcaggttcactgatggacgtgctgcatcacccaggcatgaaccaccgggtagaaatcacagaaggcatattggcggacgaatgtgcggcgctgttgtccgacttttttcgcatgcggaggcaggagatcaaggcccagaaaaaagcacaatcctctactgactctggtggttcttctggtggttctagcggcagcgagactcccgggacctcagagtccgccacacccgaaagttctggtggttcttctggtggttctatgggggagaaaagttcccgccgccgacggaatggaaaaagcggtgcgtggactgctgctataacaagctgtgttgggggtaagatggccaagaacacaattacaaagacactgaagctgaggatcgtgagaccatacaacagcgctgaggtcgagaagattgtggctgatgaaaagaacaacagggaaaagatcgccctcgagaagaacaaggataaggtgaaggaggcctgctctaagcacctgaaagtggccgcctactgcaccacacaggtggagaggaacgcctgtctgttttgtaaagctcggaagctggatgataagttttaccagaagctgcggggccagttccccgatgccgtcttttggcaggagattagcgagatcttcagacagctgcagaagcaggccgccgagatctacaaccagagcctgatcgagctctactacgagatcttcatcaagggcaagggcattgccaacgcctcctccgtggagcactacctgagcgacgtgtgctacacaagagccgccgagctctttaagaacgccgctatcgcttccgggctgaggagcaagattaagagtaacttccggctcaaggagctgaagaacatgaagagcggcctgcccactacaaagagcgacaacttcccaattccactggtgaagcagaaggggggccagtacacagggttcgagatttccaaccacaacagcgactttattattaagatcccctttggcaggtggcaggtcaagaaggagattgacaagtacaggccctgggagaagtttgatttcgagcaggtgcagaagagccccaagcctatttccctgctgctgtccacacagcggcggaagaggaacaaggggtggtctaaggatgaggggaccgaggccgagattaagaaagtgatgaacggcgactaccagacaagctacatcgaggtcaagcggggcagtaagattggcgagaagagcgcctggatgctgaacctgagcattgacgtgccaaagattgataagggcgtggatcccagcatcatcggagggatcgctgtgggggtcaagagccccctcgtgtgcgccatcaacaacgccttcagcaggtacagcatctccgataacgacctgttccactttaacaagaagatgttcgcccggcggaggattttgctcaagaagaaccggcacaagcgggccggacacggggccaagaacaagctcaagcccatcactatcctgaccgagaagagcgagaggttcaggaagaagctcatcgagagatgggcctgcgagatcgccgatttctttattaagaacaaggtcggaacagtgcagatggagaacctcgagagcatgaagaggaaggaggattcctacttcaacattcggctgagggggttctggccctacgctgagatgcagaacaagattgagtttaagctgaagcagtacgggattgagatccggaaggtggcccccaacaacaccagcaagacctgcagcaagtgcgggcacctcaacaactacttcaacttcgagtaccggaagaagaacaagttcccacacttcaagtgcgagaagtgcaactttaaggagaacgccgattacaacgccgccctgaacatcagcaaccctaagctgaagagcactaaggaggagcccaaaaggccggcggccacgaaaaaggccggccaggcaaaaaagaaaaag

SEQ ID NO: 199 - DNA, 2907 bp, synthetic construct
  source 1..2907: mol_type = other DNA; note = TaRGET-ABE-C1
atgggggagaaaagttcccgccgccgacggaatggaaaaagcggtgcgtggactgctgctataacaagctgtgttgggggtaagatggccaagaacacaattacaaagacactgaagctgaggatcgtgagaccatacaacagcgctgaggtcgagaagattgtggctgatgaaaagaacaacagggaaaagatcgccctcgagaagaacaaggataaggtgaaggaggcctgctctaagcacctgaaagtggccgcctactgcaccacacaggtggagaggaacgcctgtctgttttgtaaagctcggaagctggatgataagttttaccagaagctgcggggccagttccccgatgccgtcttttggcaggagattagcgagatcttcagacagctgcagaagcaggccgccgagatctacaaccagagcctgatcgagctctactacgagatcttcatcaagggcaagggcattgccaacgcctcctccgtggagcactacctgagcgacgtgtgctacacaagagccgccgagctctttaagaacgccgctatcgcttccgggctgaggagcaagattaagagtaacttccggctcaaggagctgaagaacatgaagagcggcctgcccactacaaagagcgacaacttcccaattccactggtgaagcagaaggggggccagtacacagggttcgagatttccaaccacaacagcgactttattattaagatcccctttggcaggtggcaggtcaagaaggagattgacaagtacaggccctgggagaagtttgatttcgagcaggtgcagaagagccccaagcctatttccctgctgctgtccacacagcggcggaagaggaacaaggggtggtctaaggatgaggggaccgaggccgagattaagaaagtgatgaacggcgactaccagacaagctacatcgaggtcaagcggggcagtaagattggcgagaagagcgcctggatgctgaacctgagcattgacgtgccaaagattgataagggcgtggatcccagcatcatcggagggatcgctgtgggggtcaagagccccctcgtgtgcgccatcaacaacgccttcagcaggtacagcatctccgataacgacctgttccactttaacaagaagatgttcgcccggcggaggattttgctcaagaagaaccggcacaagcgggccggacacggggccaagaacaagctcaagcccatcactatcctgaccgagaagagcgagaggttcaggaagaagctcatcgagagatgggcctgcgagatcgccgatttctttattaagaacaaggtcggaacagtgcagatggagaacctcgagagcatgaagaggaaggaggattcctacttcaacattcggctgagggggttctggccctacgctgagatgcagaacaagattgagtttaagctgaagcagtacgggattgagatccggaaggtggcccccaacaacaccagcaagacctgcagcaagtgcgggcacctcaacaactacttcaacttcgagtaccggaagaagaacaagttcccacacttcaagtgcgagaagtgcaactttaaggagaacgccgattacaacgccgccctgaacatcagcaaccctaagctgaagagcactaaggaggagccctctggaggatctagcggaggatcctctggcagcgagacaccaggaacaagcgagtcagcaacaccagagagcagtggcggcagcagcggcggcagctcggaagtggaattttcgcacgagtattggatgaggcacgctttaactctcgctaagagagcacgagacgaacgggaagtgccggttggggctgtcctcgtactcaataatcgagttatcggagaaggctggaacagggcaatcggactccacgatcccacagctcatgccgagataatggcgcttcgacaaggaggcctagtcatgcaaaattatcgtcttattgacgcgaccctctacgtgacctttgagccatgcgttatgtgtgcgggtgcaatgatacattcccggataggacgtgtagtatttggagttcgcaacgcgaagaccggtgcggctggttctctcatggatgtcctgcactaccctgggatgaatcaccgcgttgaaatcactgaaggcattttggccgatgaatgcgcggccctgttatgttacttttttcgcatgcccaggcaggtctttaacgcacagaagaaagcccaatcgtccactgattctggtggttcttctggtggttctagcggcagcgagactcccgggacctcagagtccgccacacccgaaagttcaggtggatcttcaggtggatcttccgaagtcgagttttcccatgagtactggatgagacacgcattgactctcgcaaagagggcttgggatgaacgcgaggtgcccgtgggggcagtactcgtgcataacaatcgcgtaatcggcgaaggttggaataggccgatcggacgccacgaccccactgcacatgcggaaatcatggcccttcgacagggagggcttgtgatgcagaattatcgacttatcgatgcgacgctgtacgtcacgcttgaaccttgcgtaatgtgcgcgggagctatgattcactcccgcattggacgagttgtattcggtgcccgcgacgccaagacgggtgccgcaggttcactgatggacgtgctgcatcacccaggcatgaaccaccgggtagaaatcacagaaggcatattggcggacgaatgtgcggcgctgttgtccgacttttttcgcatgcggaggcaggagatcaaggcccagaaaaaagcacaatcctctactgacaaaaggccggcggccacgaaaaaggccggccaggcaaaaaagaaaaag

SEQ ID NO: 200 - DNA, 2907 bp, synthetic construct
  source 1..2907: mol_type = other DNA; note = TaRGET-ABE-C2
atgggggagaaaagttcccgccgccgacggaatggaaaaagcggtgcgtggactgctgctataacaagctgtgttgggggtaagatggccaagaacacaattacaaagacactgaagctgaggatcgtgagaccatacaacagcgctgaggtcgagaagattgtggctgatgaaaagaacaacagggaaaagatcgccctcgagaagaacaaggataaggtgaaggaggcctgctctaagcacctgaaagtggccgcctactgcaccacacaggtggagaggaacgcctgtctgttttgtaaagctcggaagctggatgataagttttaccagaagctgcggggccagttccccgatgccgtcttttggcaggagattagcgagatcttcagacagctgcagaagcaggccgccgagatctacaaccagagcctgatcgagctctactacgagatcttcatcaagggcaagggcattgccaacgcctcctccgtggagcactacctgagcgacgtgtgctacacaagagccgccgagctctttaagaacgccgctatcgcttccgggctgaggagcaagattaagagtaacttccggctcaaggagctgaagaacatgaagagcggcctgcccactacaaagagcgacaacttcccaattccactggtgaagcagaaggggggccagtacacagggttcgagatttccaaccacaacagcgactttattattaagatcccctttggcaggtggcaggtcaagaaggagattgacaagtacaggccctgggagaagtttgatttcgagcaggtgcagaagagccccaagcctatttccctgctgctgtccacacagcggcggaagaggaacaaggggtggtctaaggatgaggggaccgaggccgagattaagaaagtgatgaacggcgactaccagacaagctacatcgaggtcaagcggggcagtaagattggcgagaagagcgcctggatgctgaacctgagcattgacgtgccaaagattgataagggcgtggatcccagcatcatcggagggatcgctgtgggggtcaagagccccctcgtgtgcgccatcaacaacgccttcagcaggtacagcatctccgataacgacctgttccactttaacaagaagatgttcgcccggcggaggattttgctcaagaagaaccggcacaagcgggccggacacggggccaagaacaagctcaagcccatcactatcctgaccgagaagagcgagaggttcaggaagaagctcatcgagagatgggcctgcgagatcgccgatttctttattaagaacaaggtcggaacagtgcagatggagaacctcgagagcatgaagaggaaggaggattcctacttcaacattcggctgagggggttctggccctacgctgagatgcagaacaagattgagtttaagctgaagcagtacgggattgagatccggaaggtggcccccaacaacaccagcaagacctgcagcaagtgcgggcacctcaacaactacttcaacttcgagtaccggaagaagaacaagttcccacacttcaagtgcgagaagtgcaactttaaggagaacgccgattacaacgccgccctgaacatcagcaaccctaagctgaagagcactaaggaggagccctctggaggatctagcggaggatcctctggcagcgagacaccaggaacaagcgagtcagcaacaccagagagcagtggcggcagcagcggcggcagctccgaagtcgagttttcccatgagtactggatgagacacgcattgactctcgcaaagagggcttgggatgaacgcgaggtgcccgtgggggcagtactcgtgcataacaatcgcgtaatcggcgaaggttggaataggccgatcggacgccacgaccccactgcacatgcggaaatcatggcccttcgacagggagggcttgtgatgcagaattatcgacttatcgatgcgacgctgtacgtcacgcttgaaccttgcgtaatgtgcgcgggagctatgattcactcccgcattggacgagttgtattcggtgcccgcgacgccaagacgggtgccgcaggttcactgatggacgtgctgcatcacccaggcatgaaccaccgggtagaaatcacagaaggcatattggcggacgaatgtgcggcgctgttgtccgacttttttcgcatgcggaggcaggagatcaaggcccagaaaaaagcacaatcctctactgactctggtggttcttctggtggttctagcggcagcgagactcccgggacctcagagtccgccacacccgaaagttcaggtggatcttcaggtggatcttcggaagtggaattttcgcacgagtattggatgaggcacgctttaactctcgctaagagagcacgagacgaacgggaagtgccggttggggctgtcctcgtactcaataatcgagttatcggagaaggctggaacagggcaatcggactccacgatcccacagctcatgccgagataatggcgcttcgacaaggaggcctagtcatgcaaaattatcgtcttattgacgcgaccctctacgtgacctttgagccatgcgttatgtgtgcgggtgcaatgatacattcccggataggacgtgtagtatttggagttcgcaacgcgaagaccggtgcggctggttctctcatggatgtcctgcactaccctgggatgaatcaccgcgttgaaatcactgaaggcattttggccgatgaatgcgcggccctgttatgttacttttttcgcatgcccaggcaggtctttaacgcacagaagaaagcccaatcgtccactgataaaaggccggcggccacgaaaaaggccggccaggcaaaaaagaaaaag

SEQ ID NO: 201 - protein, 970 aa, synthetic construct
  source 1..970: note = TaRGET-ABE-N1
MSEVEFSHEYWMRHALTLAKRAWDEREVPVGAVLVHNNRVIGEGWNRPIGRHDPTAHAEIMALRQGGLVMQNYRLIDATLYVTLEPCVMCAGAMIHSRIGRVVFGARDAKTGAAGSLMDVLHHPGMNHRVEITEGILADECAALLSDFFRMRRQEIKAQKKAQSSTDSGGSSGGSSGSETPGTSESATPESSGGSSGGSSEVEFSHEYWMRHALTLAKRARDEREVPVGAVLVLNNRVIGEGWNRAIGLHDPTAHAEIMALRQGGLVMQNYRLIDATLYVTFEPCVMCAGAMIHSRIGRVVFGVRNAKTGAAGSLMDVLHYPGMNHRVEITEGILADECAALLCYFFRMPRQVFNAQKKAQSSTDSGGSSGGSSGSETPGTSESATPESSGGSSGGSMGEKSSRRRRNGKSGAWTAAITSCVGGKMAKNTITKTLKLRIVRPYNSAEVEKIVADEKNNREKIALEKNKDKVKEACSKHLKVAAYCTTQVERNACLFCKARKLDDKFYQKLRGQFPDAVFWQEISEIFRQLQKQAAEIYNQSLIELYYEIFIKGKGIANASSVEHYLSDVCYTRAAELFKNAAIASGLRSKIKSNFRLKELKNMKSGLPTTKSDNFPIPLVKQKGGQYTGFEISNHNSDFIIKIPFGRWQVKKEIDKYRPWEKFDFEQVQKSPKPISLLLSTQRRKRNKGWSKDEGTEAEIKKVMNGDYQTSYIEVKRGSKIGEKSAWMLNLSIDVPKIDKGVDPSIIGGIAVGVKSPLVCAINNAFSRYSISDNDLFHFNKKMFARRRILLKKNRHKRAGHGAKNKLKPITILTEKSERFRKKLIERWACEIADFFIKNKVGTVQMENLESMKRKEDSYFNIRLRGFWPYAEMQNKIEFKLKQYGIEIRKVAPNNTSKTCSKCGHLNNYFNFEYRKKNKFPHFKCEKCNFKENADYNAALNISNPKLKSTKEEPKRPAATKKAGQAKKKK

SEQ ID NO: 202 - protein, 970 aa, synthetic construct
  source 1..970: note = TaRGET-ABE-N2
MSEVEFSHEYWMRHALTLAKRARDEREVPVGAVLVLNNRVIGEGWNRAIGLHDPTAHAEIMALRQGGLVMQNYRLIDATLYVTFEPCVMCAGAMIHSRIGRVVFGVRNAKTGAAGSLMDVLHYPGMNHRVEITEGILADECAALLCYFFRMPRQVFNAQKKAQSSTDSGGSSGGSSGSETPGTSESATPESSGGSSGGSSEVEFSHEYWMRHALTLAKRAWDEREVPVGAVLVHNNRVIGEGWNRPIGRHDPTAHAEIMALRQGGLVMQNYRLIDATLYVTLEPCVMCAGAMIHSRIGRVVFGARDAKTGAAGSLMDVLHHPGMNHRVEITEGILADECAALLSDFFRMRRQEIKAQKKAQSSTDSGGSSGGSSGSETPGTSESATPESSGGSSGGSMGEKSSRRRRNGKSGAWTAAITSCVGGKMAKNTITKTLKLRIVRPYNSAEVEKIVADEKNNREKIALEKNKDKVKEACSKHLKVAAYCTTQVERNACLFCKARKLDDKFYQKLRGQFPDAVFWQEISEIFRQLQKQAAEIYNQSLIELYYEIFIKGKGIANASSVEHYLSDVCYTRAAELFKNAAIASGLRSKIKSNFRLKELKNMKSGLPTTKSDNFPIPLVKQKGGQYTGFEISNHNSDFIIKIPFGRWQVKKEIDKYRPWEKFDFEQVQKSPKPISLLLSTQRRKRNKGWSKDEGTEAEIKKVMNGDYQTSYIEVKRGSKIGEKSAWMLNLSIDVPKIDKGVDPSIIGGIAVGVKSPLVCAINNAFSRYSISDNDLFHFNKKMFARRRILLKKNRHKRAGHGAKNKLKPITILTEKSERFRKKLIERWACEIADFFIKNKVGTVQMENLESMKRKEDSYFNIRLRGFWPYAEMQNKIEFKLKQYGIEIRKVAPNNTSKTCSKCGHLNNYFNFEYRKKNKFPHFKCEKCNFKENADYNAALNISNPKLKSTKEEPKRPAATKKAGQAKKKK

SEQ ID NO: 203 - protein, 969 aa, synthetic construct
  source 1..969: note = TaRGET-ABE-C1
MGEKSSRRRRNGKSGAWTAAITSCVGGKMAKNTITKTLKLRIVRPYNSAEVEKIVADEKNNREKIALEKNKDKVKEACSKHLKVAAYCTTQVERNACLFCKARKLDDKFYQKLRGQFPDAVFWQEISEIFRQLQKQAAEIYNQSLIELYYEIFIKGKGIANASSVEHYLSDVCYTRAAELFKNAAIASGLRSKIKSNFRLKELKNMKSGLPTTKSDNFPIPLVKQKGGQYTGFEISNHNSDFIIKIPFGRWQVKKEIDKYRPWEKFDFEQVQKSPKPISLLLSTQRRKRNKGWSKDEGTEAEIKKVMNGDYQTSYIEVKRGSKIGEKSAWMLNLSIDVPKIDKGVDPSIIGGIAVGVKSPLVCAINNAFSRYSISDNDLFHFNKKMFARRRILLKKNRHKRAGHGAKNKLKPITILTEKSERFRKKLIERWACEIADFFIKNKVGTVQMENLESMKRKEDSYFNIRLRGFWPYAEMQNKIEFKLKQYGIEIRKVAPNNTSKTCSKCGHLNNYFNFEYRKKNKFPHFKCEKCNFKENADYNAALNISNPKLKSTKEEPSGGSSGGSSGSETPGTSESATPESSGGSSGGSSEVEFSHEYWMRHALTLAKRARDEREVPVGAVLVLNNRVIGEGWNRAIGLHDPTAHAEIMALRQGGLVMQNYRLIDATLYVTFEPCVMCAGAMIHSRIGRVVFGVRNAKTGAAGSLMDVLHYPGMNHRVEITEGILADECAALLCYFFRMPRQVFNAQKKAQSSTDSGGSSGGSSGSETPGTSESATPESSGGSSGGSSEVEFSHEYWMRHALTLAKRAWDEREVPVGAVLVHNNRVIGEGWNRPIGRHDPTAHAEIMALRQGGLVMQNYRLIDATLYVTLEPCVMCAGAMIHSRIGRVVFGARDAKTGAAGSLMDVLHHPGMNHRVEITEGILADECAALLSDFFRMRRQEIKAQKKAQSSTDKRPAATKKAGQAKKKK

SEQ ID NO: 204 - protein, 969 aa, synthetic construct
  source 1..969: note = TaRGET-ABE-C2
MGEKSSRRRRNGKSGAWTAAITSCVGGKMAKNTITKTLKLRIVRPYNSAEVEKIVADEKNNREKIALEKNKDKVKEACSKHLKVAAYCTTQVERNACLFCKARKLDDKFYQKLRGQFPDAVFWQEISEIFRQLQKQAAEIYNQSLIELYYEIFIKGKGIANASSVEHYLSDVCYTRAAELFKNAAIASGLRSKIKSNFRLKELKNMKSGLPTTKSDNFPIPLVKQKGGQYTGFEISNHNSDFIIKIPFGRWQVKKEIDKYRPWEKFDFEQVQKSPKPISLLLSTQRRKRNKGWSKDEGTEAEIKKVMNGDYQTSYIEVKRGSKIGEKSAWMLNLSIDVPKIDKGVDPSIIGGIAVGVKSPLVCAINNAFSRYSISDNDLFHFNKKMFARRRILLKKNRHKRAGHGAKNKLKPITILTEKSERFRKKLIERWACEIADFFIKNKVGTVQMENLESMKRKEDSYFNIRLRGFWPYAEMQNKIEFKLKQYGIEIRKVAPNNTSKTCSKCGHLNNYFNFEYRKKNKFPHFKCEKCNFKENADYNAALNISNPKLKSTKEEPSGGSSGGSSGSETPGTSESATPESSGGSSGGSSEVEFSHEYWMRHALTLAKRAWDEREVPVGAVLVHNNRVIGEGWNRPIGRHDPTAHAEIMALRQGGLVMQNYRLIDATLYVTLEPCVMCAGAMIHSRIGRVVFGARDAKTGAAGSLMDVLHHPGMNHRVEITEGILADECAALLSDFFRMRRQEIKAQKKAQSSTDSGGSSGGSSGSETPGTSESATPESSGGSSGGSSEVEFSHEYWMRHALTLAKRARDEREVPVGAVLVLNNRVIGEGWNRAIGLHDPTAHAEIMALRQGGLVMQNYRLIDATLYVTFEPCVMCAGAMIHSRIGRVVFGVRNAKTGAAGSLMDVLHYPGMNHRVEITEGILADECAALLCYFFRMPRQVFNAQKKAQSSTDKRPAATKKAGQAKKKK

SEQ ID NO: 205 - DNA, 2907 bp, synthetic construct
  source 1..2907: mol_type = other DNA; note = TaRGET-ABE-C3.0
atgggggagaaaagttcccgccgccgacggaatggaaaaagcggtgcgtggactgctgctataacaagctgtgttgggggtaagatggccaagaacacaattacaaagacactgaagctgaggatcgtgagaccatacaacagcgctgaggtcgagaagattgtggctgatgaaaagaacaacagggaaaagatcgccctcgagaagaacaaggataaggtgaaggaggcctgctctaagcacctgaaagtggccgcctactgcaccacacaggtggagaggaacgcctgtctgttttgtaaagctcggaagctggatgataagttttaccagaagctgcggggccagttccccgatgccgtcttttggcaggagattagcgagatcttcagacagctgcagaagcaggccgccgagatctacaaccagagcctgatcgagctctactacgagatcttcatcaagggcaagggcattgccaacgcctcctccgtggagcactacctgagcgacgtgtgctacacaagagccgccgagctctttaagaacgccgctatcgcttccgggctgaggagcaagattaagagtaacttccggctcaaggagctgaagaacatgaagagcggcctgcccactacaaagagcgacaacttcccaattccactggtgaagcagaaggggggccagtacacagggttcgagatttccaaccacaacagcgactttattattaagatcccctttggcaggtggcaggtcaagaaggagattgacaagtacaggccctgggagaagtttgatttcgagcaggtgcagaagagccccaagcctatttccctgctgctgtccacacagcggcggaagaggaacaaggggtggtctaaggatgaggggaccgaggccgagattaagaaagtgatgaacggcgactaccagacaagctacatcgaggtcaagcggggcagtaagattggcgagaagagcgcctggatgctgaacctgagcattgacgtgccaaagattgataagggcgtggatcccagcatcatcggagggatcgctgtgggggtcaagagccccctcgtgtgcgccatcaacaacgccttcagcaggtacagcatctccgataacgacctgttccactttaacaagaagatgttcgcccggcggaggattttgctcaagaagaaccggcacaagcgggccggacacggggccaagaacaagctcaagcccatcactatcctgaccgagaagagcgagaggttcaggaagaagctcatcgagagatgggcctgcgagatcgccgatttctttattaagaacaaggtcggaacagtgcagatggagaacctcgagagcatgaagaggaaggaggattcctacttcaacattcggctgagggggttctggccctacgctgagatgcagaacaagattgagtttaagctgaagcagtacgggattgagatccggaaggtggcccccaacaacaccagcaagacctgcagcaagtgcgggcacctcaacaactacttcaacttcgagtaccggaagaagaacaagttcccacacttcaagtgcgagaagtgcaactttaaggagaacgccgattacaacgccgccctgaacatcagcaaccctaagctgaagagcactaaggaggagccctctggaggatctagcggaggatcctctggcagcgagacaccaggaacaagcgagtcagcaacaccagagagcagtggcggcagcagcggcggcagctccgaagtcgagttttcccatgagtactggatgagacacgcattgactctcgcaaagagggcttgggatgaacgcgaggtgcccgtgggggcagtactcgtgcataacaatcgcgtaatcggcgaaggttggaataggccgatcggacgccacgaccccactgcacatgcggaaatcatggcccttcgacagggagggcttgtgatgcagaattatcgacttatcgatgcgacgctgtacgtcacgcttgaaccttgcgtaatgtgcgcgggagctatgattcactcccgcattggacgagttgtattcggtgcccgcgacgccaagacgggtgccgcaggttcactgatggacgtgctgcatcacccaggcatgaaccaccgggtagaaatcacagaaggcatattggcggacgaatgtgcggcgctgttgtccgacttttttcgcatgcggaggcaggagatcaaggcccagaaaaaagcacaatcctctactgactctggtggttcttctggtggttctagcggcagcgagactcccgggacctcagagtccgccacacccgaaagttcaggtggatcttcaggtggatcttcggaagtggaattttcgcacgagtattggatgaggcacgctttaactctcgctaagagagcacgagacgaacgggaagtgccggttggggctgtcctcgtactcaataatcgagttatcggagaaggctggaacagggcaatcggactccacgatcccacagctcatgccgagataatggcgcttcgacaaggaggcctagtcatgcaaaattatcgtcttattgacgcgaccctctacgtgacctttgagccatgcgttatgtgtgcgggtgcaatgatacattcccggataggacgtgtagtatttggatggcgccaggcgaagaccggtgcggctggttctctcatggatgtcctgcactaccctgggatgaatcaccgcgttgaaatcactgaaggcattttggccgatgaatgcgcggccctgttatgttacttttttcgcatgcccaggcaggtctttaacgcacagaagaaagcccaatcgtccactgataaaaggccggcggccacgaaaaaggccggccaggcaaaaaagaaaaag

SEQ ID NO: 206 - protein, 969 aa, synthetic construct
  source 1..969: note = TaRGET-ABE-C3.0
MGEKSSRRRRNGKSGAWTAAITSCVGGKMAKNTITKTLKLRIVRPYNSAEVEKIVADEKNNREKIALEKNKDKVKEACSKHLKVAAYCTTQVERNACLFCKARKLDDKFYQKLRGQFPDAVFWQEISEIFRQLQKQAAEIYNQSLIELYYEIFIKGKGIANASSVEHYLSDVCYTRAAELFKNAAIASGLRSKIKSNFRLKELKNMKSGLPTTKSDNFPIPLVKQKGGQYTGFEISNHNSDFIIKIPFGRWQVKKEIDKYRPWEKFDFEQVQKSPKPISLLLSTQRRKRNKGWSKDEGTEAEIKKVMNGDYQTSYIEVKRGSKIGEKSAWMLNLSIDVPKIDKGVDPSIIGGIAVGVKSPLVCAINNAFSRYSISDNDLFHFNKKMFARRRILLKKNRHKRAGHGAKNKLKPITILTEKSERFRKKLIERWACEIADFFIKNKVGTVQMENLESMKRKEDSYFNIRLRGFWPYAEMQNKIEFKLKQYGIEIRKVAPNNTSKTCSKCGHLNNYFNFEYRKKNKFPHFKCEKCNFKENADYNAALNISNPKLKSTKEEPSGGSSGGSSGSETPGTSESATPESSGGSSGGSSEVEFSHEYWMRHALTLAKRAWDEREVPVGAVLVHNNRVIGEGWNRPIGRHDPTAHAEIMALRQGGLVMQNYRLIDATLYVTLEPCVMCAGAMIHSRIGRVVFGARDAKTGAAGSLMDVLHHPGMNHRVEITEGILADECAALLSDFFRMRRQEIKAQKKAQSSTDSGGSSGGSSGSETPGTSESATPESSGGSSGGSSEVEFSHEYWMRHALTLAKRARDEREVPVGAVLVLNNRVIGEGWNRAIGLHDPTAHAEIMALRQGGLVMQNYRLIDATLYVTFEPCVMCAGAMIHSRIGRVVFGWRQAKTGAAGSLMDVLHYPGMNHRVEITEGILADECAALLCYFFRMPRQVFNAQKKAQSSTDKRPAATKKAGQAKKKK

SEQ ID NO: 207 - DNA, 2907 bp, synthetic construct
  source 1..2907: mol_type = other DNA; note = TaRGET-ABE-C3.1
atgggggagaaaagttcccgccgccgacggaatggaaaaagcggtgcgtggactgctgctataacaagctgtgttgggggtaagatggccaagaacacaattacaaagacactgaagctgaggatcgtgagaccatacaacagcgctgaggtcgagaagattgtggctgatgaaaagaacaacagggaaaagatcgccctcgagaagaacaaggataaggtgaaggaggcctgctctaagcacctgaaagtggccgcctactgcaccacacaggtggagaggaacgcctgtctgttttgtaaagctcggaagctggatgataagttttaccagaagctgcggggccagttccccgatgccgtcttttggcaggagattagcgagatcttcagacagctgcagaagcaggccgccgagatctacaaccagagcctgatcgagctctactacgagatcttcatcaagggcaagggcattgccaacgcctcctccgtggagcactacctgagcgacgtgtgctacacaagagccgccgagctctttaagaacgccgctatcgcttccgggctgaggagcaagattaagagtaacttccggctcaaggagctgaagaacatgaagagcggcctgcccactacaaagagcgacaacttcccaattccactggtgaagcagaaggggggccagtacacagggttcgagatttccaaccacaacagcgactttattattaagatcccctttggcaggtggcaggtcaagaaggagattgacaagtacaggccctgggagaagtttgatttcgagcaggtgcagaagagccccaagcctatttccctgctgctgtccacacagcggcggaagaggaacaaggggtggtctaaggatgaggggaccgaggccgagattaagaaagtgatgaacggcgactaccagacaagctacatcgaggtcaagcggggcagtaagattggcgagaagagcgcctggatgctgaacctgagcattgacgtgccaaagattgataagggcgtggatcccagcatcatcggagggatcgctgtgggggtcaagagccccctcgtgtgcgccatcaacaacgccttcagcaggtacagcatctccgataacgacctgttccactttaacaagaagatgttcgcccggcggaggattttgctcaagaagaaccggcacaagcgggccggacacggggccaagaacaagctcaagcccatcactatcctgaccgagaagagcgagaggttcaggaagaagctcatcgagagatgggcctgcgagatcgccgatttctttattaagaacaaggtcggaacagtgcagatggagaacctcgagagcatgaagaggaaggaggattcctacttcaacattcggctgagggggttctggccctacgctgagatgcagaacaagattgagtttaagctgaagcagtacgggattgagatccggaaggtggcccccaacaacaccagcaagacctgcagcaagtgcgggcacctcaacaactacttcaacttcgagtaccggaagaagaacaagttcccacacttcaagtgcgagaagtgcaactttaaggagaacgccgattacaacgccgccctgaacatcagcaaccctaagctgaagagcactaaggaggagccctctggaggatctagcggaggatcctctggcagcgagacaccaggaacaagcgagtcagcaacaccagagagcagtggcggcagcagcggcggcagctccgaagtcgagttttcccatgagtactggatgagacacgcattgactctcgcaaagagggcttgggatgaacgcgaggtgcccgtgggggcagtactcgtgcataacaatcgcgtaatcggcgaaggttggaataggccgatcggacgccacgaccccactgcacatgcggaaatcatggcccttcgacagggagggcttgtgatgcagaattatcgacttatcgatgcgacgctgtacgtcacgcttgaaccttgcgtaatgtgcgcgggagctatgattcactcccgcattggacgagttgtattcggtgcccgcgacgccaagacgggtgccgcaggttcactgatggacgtgctgcatcacccaggcatgaaccaccgggtagaaatcacagaaggcatattggcggacgaatgtgcggcgctgttgtccgacttttttcgcatgcggaggcaggagatcaaggcccagaaaaaagcacaatcctctactgactctggtggttcttctggtggttctagcggcagcgagactcccgggacctcagagtccgccacacccgaaagttcaggtggatcttcaggtggatcttctgaggtggagttttcccacgagtactggatgagacatgccctgaccctggccaagagggcacgggatgagagggaggtgcctgtgggagccgtgctggtgctgaacaatagagtgatcggcgagggctggaacagagccatcggcctgcacgacccaacagcccatgccgaaattatggccctgagacagggcggcctggtcatgcagaactacagactgattgacgccaccctgtacgtgacattcgagccttgcgtgatgtgcgccggcgccatgatccactctaggatcggccgcgtggtgtttggatggagacagtctaaaagaggcgccgcaggctccctgatgaacgtgctgaactaccccggcatgaatcaccgcgtcgaaattaccgagggaatcctggcagatgaatgtgccgccctgctgtgcgatttctatcggatgcctagacaggtgttcaatgctcagaagaaggcccagagctccatcaacaaaaggccggcggccacgaaaaaggccggccaggcaaaaaagaaaaag

SEQ ID NO: 208 - protein, 969 aa, synthetic construct
  source 1..969: note = TaRGET-ABE-C3.1
MGEKSSRRRRNGKSGAWTAAITSCVGGKMAKNTITKTLKLRIVRPYNSAEVEKIVADEKNNREKIALEKNKDKVKEACSKHLKVAAYCTTQVERNACLFCKARKLDDKFYQKLRGQFPDAVFWQEISEIFRQLQKQAAEIYNQSLIELYYEIFIKGKGIANASSVEHYLSDVCYTRAAELFKNAAIASGLRSKIKSNFRLKELKNMKSGLPTTKSDNFPIPLVKQKGGQYTGFEISNHNSDFIIKIPFGRWQVKKEIDKYRPWEKFDFEQVQKSPKPISLLLSTQRRKRNKGWSKDEGTEAEIKKVMNGDYQTSYIEVKRGSKIGEKSAWMLNLSIDVPKIDKGVDPSIIGGIAVGVKSPLVCAINNAFSRYSISDNDLFHFNKKMFARRRILLKKNRHKRAGHGAKNKLKPITILTEKSERFRKKLIERWACEIADFFIKNKVGTVQMENLESMKRKEDSYFNIRLRGFWPYAEMQNKIEFKLKQYGIEIRKVAPNNTSKTCSKCGHLNNYFNFEYRKKNKFPHFKCEKCNFKENADYNAALNISNPKLKSTKEEPSGGSSGGSSGSETPGTSESATPESSGGSSGGSSEVEFSHEYWMRHALTLAKRAWDEREVPVGAVLVHNNRVIGEGWNRPIGRHDPTAHAEIMALRQGGLVMQNYRLIDATLYVTLEPCVMCAGAMIHSRIGRVVFGARDAKTGAAGSLMDVLHHPGMNHRVEITEGILADECAALLSDFFRMRRQEIKAQKKAQSSTDSGGSSGGSSGSETPGTSESATPESSGGSSGGSSEVEFSHEYWMRHALTLAKRARDEREVPVGAVLVLNNRVIGEGWNRAIGLHDPTAHAEIMALRQGGLVMQNYRLIDATLYVTFEPCVMCAGAMIHSRIGRVVFGWRQSKRGAAGSLMNVLNYPGMNHRVEITEGILADECAALLCDFYRMPRQVFNAQKKAQSSINKRPAATKKAGQAKKKK

SEQ ID NO: 209 - DNA, 498 bp, synthetic construct
  source 1..498: mol_type = other DNA; note = Wild type Tad for TaRGET-ABE system
tccgaagtcgagttttcccatgagtactggatgagacacgcattgactctcgcaaagagggcttgggatgaacgcgaggtgcccgtgggggcagtactcgtgcataacaatcgcgtaatcggcgaaggttggaataggccgatcggacgccacgaccccactgcacatgcggaaatcatggcccttcgacagggagggcttgtgatgcagaattatcgacttatcgatgcgacgctgtacgtcacgcttgaaccttgcgtaatgtgcgcgggagctatgattcactcccgcattggacgagttgtattcggtgcccgcgacgccaagacgggtgccgcaggttcactgatggacgtgctgcatcacccaggcatgaaccaccgggtagaaatcacagaaggcatattggcggacgaatgtgcggcgctgttgtccgacttttttcgcatgcggaggcaggagatcaaggcccagaaaaaagcacaatcctctactgac

SEQ ID NO: 210 - protein, 166 aa, synthetic construct
  source 1..166: note = Wild type Tad for TaRGET-ABE system
SEVEFSHEYWMRHALTLAKRAWDEREVPVGAVLVHNNRVIGEGWNRPIGRHDPTAHAEIMALRQGGLVMQNYRLIDATLYVTLEPCVMCAGAMIHSRIGRVVFGARDAKTGAAGSLMDVLHHPGMNHRVEITEGILADECAALLSDFFRMRRQEIKAQKKAQSSTD

SEQ ID NO: 211 - DNA, 498 bp, synthetic construct
  source 1..498: mol_type = other DNA; note = mutant Tad(C1 and C2) for TaRGET-ABE system
tcggaagtggaattttcgcacgagtattggatgaggcacgctttaactctcgctaagagagcacgagacgaacgggaagtgccggttggggctgtcctcgtactcaataatcgagttatcggagaaggctggaacagggcaatcggactccacgatcccacagctcatgccgagataatggcgcttcgacaaggaggcctagtcatgcaaaattatcgtcttattgacgcgaccctctacgtgacctttgagccatgcgttatgtgtgcgggtgcaatgatacattcccggataggacgtgtagtatttggagttcgcaacgcgaagaccggtgcggctggttctctcatggatgtcctgcactaccctgggatgaatcaccgcgttgaaatcactgaaggcattttggccgatgaatgcgcggccctgttatgttacttttttcgcatgcccaggcaggtctttaacgcacagaagaaagcccaatcgtccactgat

SEQ ID NO: 212 - protein, 166 aa, synthetic construct
  source 1..166: note = mutant Tad(C1 and C2) for TaRGET-ABE system
SEVEFSHEYWMRHALTLAKRARDEREVPVGAVLVLNNRVIGEGWNRAIGLHDPTAHAEIMALRQGGLVMQNYRLIDATLYVTFEPCVMCAGAMIHSRIGRVVFGVRNAKTGAAGSLMDVLHYPGMNHRVEITEGILADECAALLCYFFRMPRQVFNAQKKAQSSTD

SEQ ID NO: 213 - DNA, 498 bp, synthetic construct
  source 1..498: mol_type = other DNA; note = mutant Tad(C3.0) for TaRGET-ABE system
tcggaagtggaattttcgcacgagtattggatgaggcacgctttaactctcgctaagagagcacgagacgaacgggaagtgccggttggggctgtcctcgtactcaataatcgagttatcggagaaggctggaacagggcaatcggactccacgatcccacagctcatgccgagataatggcgcttcgacaaggaggcctagtcatgcaaaattatcgtcttattgacgcgaccctctacgtgacctttgagccatgcgttatgtgtgcgggtgcaatgatacattcccggataggacgtgtagtatttggatggcgccaggcgaagaccggtgcggctggttctctcatggatgtcctgcactaccctgggatgaatcaccgcgttgaaatcactgaaggcattttggccgatgaatgcgcggccctgttatgttacttttttcgcatgcccaggcaggtctttaacgcacagaagaaagcccaatcgtccactgat

SEQ ID NO: 214 - protein, 166 aa, synthetic construct
  source 1..166: note = mutant Tad(C3.0) for TaRGET-ABE system
SEVEFSHEYWMRHALTLAKRARDEREVPVGAVLVLNNRVIGEGWNRAIGLHDPTAHAEIMALRQGGLVMQNYRLIDATLYVTFEPCVMCAGAMIHSRIGRVVFGWRQAKTGAAGSLMDVLHYPGMNHRVEITEGILADECAALLCYFFRMPRQVFNAQKKAQSSTD

SEQ ID NO: 215 - DNA, 498 bp, synthetic construct
  source 1..498: mol_type = other DNA; note = mutant Tad(C3.1) for TaRGET-ABE system
tctgaggtggagttttcccacgagtactggatgagacatgccctgaccctggccaagagggcacgggatgagagggaggtgcctgtgggagccgtgctggtgctgaacaatagagtgatcggcgagggctggaacagagccatcggcctgcacgacccaacagcccatgccgaaattatggccctgagacagggcggcctggtcatgcagaactacagactgattgacgccaccctgtacgtgacattcgagccttgcgtgatgtgcgccggcgccatgatccactctaggatcggccgcgtggtgtttggatggagacagtctaaaagaggcgccgcaggctccctgatgaacgtgctgaactaccccggcatgaatcaccgcgtcgaaattaccgagggaatcctggcagatgaatgtgccgccctgctgtgcgatttctatcggatgcctagacaggtgttcaatgctcagaagaaggcccagagctccatcaac

SEQ ID NO: 216 - protein, 166 aa, synthetic construct
  source 1..166: note = mutant Tad(C3.1) for TaRGET-ABE system
SEVEFSHEYWMRHALTLAKRARDEREVPVGAVLVLNNRVIGEGWNRAIGLHDPTAHAEIMALRQGGLVMQNYRLIDATLYVTFEPCVMCAGAMIHSRIGRVVFGWRQSKRGAAGSLMNVLNYPGMNHRVEITEGILADECAALLCDFYRMPRQVFNAQKKAQSSIN

SEQ ID NO: 217 - DNA, 48 bp, synthetic construct
  source 1..48: mol_type = other DNA; note = NLS for TaRGET-ABE system
aaaaggccggcggccacgaaaaaggccggccaggcaaaaaagaaaaag

SEQ ID NO: 218 - protein, 16 aa, synthetic construct
  source 1..16: note = NLS for TaRGET-ABE system
KRPAATKKAGQAKKKK

SEQ ID NO: 219 - DNA, 96 bp, synthetic construct
  source 1..96: mol_type = other DNA; note = linker 1 for TaRGET-ABE system
tctggaggatctagcggaggatcctctggcagcgagacaccaggaacaagcgagtcagcaacaccagagagcagtggcggcagcagcggcggcagc

SEQ ID NO: 220 - protein, 32 aa, synthetic construct
  source 1..32: note = linker 1 for TaRGET-ABE system
SGGSSGGSSGSETPGTSESATPESSGGSSGGS

SEQ ID NO: 221 - DNA, 96 bp, synthetic construct
  source 1..96: mol_type = other DNA; note = linker 2 for TaRGET-ABE system
tctggtggttcttctggtggttctagcggcagcgagactcccgggacctcagagtccgccacacccgaaagttcaggtggatcttcaggtggatct

SEQ ID NO: 222 - protein, 32 aa, synthetic construct; identical to SEQ ID NO: 220
  source 1..32: note = linker 2 for TaRGET-ABE system

SEQ ID NO: 223 - protein, 557 aa, synthetic construct
  source 1..557: note = Engineered CWCas12f (D354A)
MGEKSSRRRRNGKSGAWTAAITSCVGGKMAKNTITKTLKLRIVRPYNSAEVEKIVADEKNNREKIALEKNKDKVKEACSKHLKVAAYCTTQVERNACLFCKARKLDDKFYQKLRGQFPDAVFWQEISEIFRQLQKQAAEIYNQSLIELYYEIFIKGKGIANASSVEHYLSDVCYTRAAELFKNAAIASGLRSKIKSNFRLKELKNMKSGLPTTKSDNFPIPLVKQKGGQYTGFEISNHNSDFIIKIPFGRWQVKKEIDKYRPWEKFDFEQVQKSPKPISLLLSTQRRKRNKGWSKDEGTEAEIKKVMNGDYQTSYIEVKRGSKIGEKSAWMLNLSIDVPKIDKGVDPSIIGGIAVGVKSPLVCAINNAFSRYSISDNDLFHFNKKMFARRRILLKKNRHKRAGHGAKNKLKPITILTEKSERFRKKLIERWACEIADFFIKNKVGTVQMENLESMKRKEDSYFNIRLRGFWPYAEMQNKIEFKLKQYGIEIRKVAPNNTSKTCSKCGHLNNYFNFEYRKKNKFPHFKCEKCNFKENADYNAALNISNPKLKSTKEEP

SEQ ID NO: 224 - protein, 557 aa, synthetic construct
  source 1..557: note = Engineered CWCas12f (E450A)
MGEKSSRRRRNGKSGAWTAAITSCVGGKMAKNTITKTLKLRIVRPYNSAEVEKIVADEKNNREKIALEKNKDKVKEACSKHLKVAAYCTTQVERNACLFCKARKLDDKFYQKLRGQFPDAVFWQEISEIFRQLQKQAAEIYNQSLIELYYEIFIKGKGIANASSVEHYLSDVCYTRAAELFKNAAIASGLRSKIKSNFRLKELKNMKSGLPTTKSDNFPIPLVKQKGGQYTGFEISNHNSDFIIKIPFGRWQVKKEIDKYRPWEKFDFEQVQKSPKPISLLLSTQRRKRNKGWSKDEGTEAEIKKVMNGDYQTSYIEVKRGSKIGEKSAWMLNLSIDVPKIDKGVDPSIIGGIDVGVKSPLVCAINNAFSRYSISDNDLFHFNKKMFARRRILLKKNRHKRAGHGAKNKLKPITILTEKSERFRKKLIERWACEIADFFIKNKVGTVQMANLESMKRKEDSYFNIRLRGFWPYAEMQNKIEFKLKQYGIEIRKVAPNNTSKTCSKCGHLNNYFNFEYRKKNKFPHFKCEKCNFKENADYNAALNISNPKLKSTKEEP

SEQ ID NO: 225 - protein, 557 aa, synthetic construct
  source 1..557: note = Engineered CWCas12f (R518A)
MGEKSSRRRRNGKSGAWTAAITSCVGGKMAKNTITKTLKLRIVRPYNSAEVEKIVADEKNNREKIALEKNKDKVKEACSKHLKVAAYCTTQVERNACLFCKARKLDDKFYQKLRGQFPDAVFWQEISEIFRQLQKQAAEIYNQSLIELYYEIFIKGKGIANASSVEHYLSDVCYTRAAELFKNAAIASGLRSKIKSNFRLKELKNMKSGLPTTKSDNFPIPLVKQKGGQYTGFEISNHNSDFIIKIPFGRWQVKKEIDKYRPWEKFDFEQVQKSPKPISLLLSTQRRKRNKGWSKDEGTEAEIKKVMNGDYQTSYIEVKRGSKIGEKSAWMLNLSIDVPKIDKGVDPSIIGGIDVGVKSPLVCAINNAFSRYSISDNDLFHFNKKMFARRRILLKKNRHKRAGHGAKNKLKPITILTEKSERFRKKLIERWACEIADFFIKNKVGTVQMENLESMKRKEDSYFNIRLRGFWPYAEMQNKIEFKLKQYGIEIRKVAPNNTSKTCSKCGHLNNYFNFEYAKKNKFPHFKCEKCNFKENADYNAALNISNPKLKSTKEEP

SEQ ID NO: 226 - protein, 557 aa, synthetic construct
  source 1..557: note = Engineered CWCas12f (D538A)
MGEKSSRRRRNGKSGAWTAAITSCVGGKMAKNTITKTLKLRIVRPYNSAEVEKIVADEKNNREKIALEKNKDKVKEACSKHLKVAAYCTTQVERNACLFCKARKLDDKFYQKLRGQFPDAVFWQEISEIFRQLQKQAAEIYNQSLIELYYEIFIKGKGIANASSVEHYLSDVCYTRAAELFKNAAIASGLRSKIKSNFRLKELKNMKSGLPTTKSDNFPIPLVKQKGGQYTGFEISNHNSDFIIKIPFGRWQVKKEIDKYRPWEKFDFEQVQKSPKPISLLLSTQRRKRNKGWSKDEGTEAEIKKVMNGDYQTSYIEVKRGSKIGEKSAWMLNLSIDVPKIDKGVDPSIIGGIDVGVKSPLVCAINNAFSRYSISDNDLFHFNKKMFARRRILLKKNRHKRAGHGAKNKLKPITILTEKSERFRKKLIERWACEIADFFIKNKVGTVQMENLESMKRKEDSYFNIRLRGFWPYAEMQNKIEFKLKQYGIEIRKVAPNNTSKTCSKCGHLNNYFNFEYRKKNKFPHFKCEKCNFKENAAYNAALNISNPKLKSTKEEP

SEQ ID NO: 227 - protein, 557 aa, synthetic construct
  source 1..557: note = Engineered CWCas12f (I159W)
MGEKSSRRRRNGKSGAWTAAITSCVGGKMAKNTITKTLKLRIVRPYNSAEVEKIVADEKNNREKIALEKNKDKVKEACSKHLKVAAYCTTQVERNACLFCKARKLDDKFYQKLRGQFPDAVFWQEISEIFRQLQKQAAEIYNQSLIELYYEIFIKGKGWANASSVEHYLSDVCYTRAAELFKNAAIASGLRSKIKSNFRLKELKNMKSGLPTTKSDNFPIPLVKQKGGQYTGFEISNHNSDFIIKIPFGRWQVKKEIDKYRPWEKFDFEQVQKSPKPISLLLSTQRRKRNKGWSKDEGTEAEIKKVMNGDYQTSYIEVKRGSKIGEKSAWMLNLSIDVPKIDKGVDPSIIGGIDVGVKSPLVCAINNAFSRYSISDNDLFHFNKKMFARRRILLKKNRHKRAGHGAKNKLKPITILTEKSERFRKKLIERWACEIADFFIKNKVGTVQMENLESMKRKEDSYFNIRLRGFWPYAEMQNKIEFKLKQYGIEIRKVAPNNTSKTCSKCGHLNNYFNFEYRKKNKFPHFKCEKCNFKENADYNAALNISNPKLKSTKEEP

SEQ ID NO: 228 - protein, 557 aa, synthetic construct
  source 1..557: note = Engineered CWCas12f (S164Y)
MGEKSSRRRRNGKSGAWTAAITSCVGGKMAKNTITKTLKLRIVRPYNSAEVEKIVADEKNNREKIALEKNKDKVKEACSKHLKVAAYCTTQVERNACLFCKARKLDDKFYQKLRGQFPDAVFWQEISEIFRQLQKQAAEIYNQSLIELYYEIFIKGKGIANASYVEHYLSDVCYTRAAELFKNAAIASGLRSKIKSNFRLKELKNMKSGLPTTKSDNFPIPLVKQKGGQYTGFEISNHNSDFIIKIPFGRWQVKKEIDKYRPWEKFDFEQVQKSPKPISLLLSTQRRKRNKGWSKDEGTEAEIKKVMNGDYQTSYIEVKRGSKIGEKSAWMLNLSIDVPKIDKGVDPSIIGGIDVGVKSPLVCAINNAFSRYSISDNDLFHFNKKMFARRRILLKKNRHKRAGHGAKNKLKPITILTEKSERFRKKLIERWACEIADFFIKNKVGTVQMENLESMKRKEDSYFNIRLRGFWPYAEMQNKIEFKLKQYGIEIRKVAPNNTSKTCSKCGHLNNYFNFEYRKKNKFPHFKCEKCNFKENADYNAALNISNPKLKSTKEEP

SEQ ID NO: 229 - protein, 557 aa, synthetic construct
  source 1..557: note = Engineered CWCas12f (I159W/S164Y)
MGEKSSRRRRNGKSGAWTAAITSCVGGKMAKNTITKTLKLRIVRPYNSAEVEKIVADEKNNREKIALEKNKDKVKEACSKHLKVAAYCTTQVERNACLFCKARKLDDKFYQKLRGQFPDAVFWQEISEIFRQLQKQAAEIYNQSLIELYYEIFIKGKGWANASYVEHYLSDVCYTRAAELFKNAAIASGLRSKIKSNFRLKELKNMKSGLPTTKSDNFPIPLVKQKGGQYTGFEISNHNSDFIIKIPFGRWQVKKEIDKYRPWEKFDFEQVQKSPKPISLLLSTQRRKRNKGWSKDEGTEAEIKKVMNGDYQTSYIEVKRGSKIGEKSAWMLNLSIDVPKIDKGVDPSIIGGIDVGVKSPLVCAINNAFSRYSISDNDLFHFNKKMFARRRILLKKNRHKRAGHGAKNKLKPITILTEKSERFRKKLIERWACEIADFFIKNKVGTVQMENLESMKRKEDSYFNIRLRGFWPYAEMQNKIEFKLKQYGIEIRKVAPNNTSKTCSKCGHLNNYFNFEYRKKNKFPHFKCEKCNFKENADYNAALNISNPKLKSTKEEP

SEQ ID NO: 230 - protein, 557 aa, synthetic construct
  source 1..557: note = Engineered CWCas12f (S170C)
MGEKSSRRRRNGKSGAWTAAITSCVGGKMAKNTITKTLKLRIVRPYNSAEVEKIVADEKNNREKIALEKNKDKVKEACSKHLKVAAYCTTQVERNACLFCKARKLDDKFYQKLRGQFPDAVFWQEISEIFRQLQKQAAEIYNQSLIELYYEIFIKGKGIANASSVEHYLCDVCYTRAAELFKNAAIASGLRSKIKSNFRLKELKNMKSGLPTTKSDNFPIPLVKQKGGQYTGFEISNHNSDFIIKIPFGRWQVKKEIDKYRPWEKFDFEQVQKSPKPISLLLSTQRRKRNKGWSKDEGTEAEIKKVMNGDYQTSYIEVKRGSKIGEKSAWMLNLSIDVPKIDKGVDPSIIGGIDVGVKSPLVCAINNAFSRYSISDNDLFHFNKKMFARRRILLKKNRHKRAGHGAKNKLKPITILTEKSERFRKKLIERWACEIADFFIKNKVGTVQMENLESMKRKEDSYFNIRLRGFWPYAEMQNKIEFKLKQYGIEIRKVAPNNTSKTCSKCGHLNNYFNFEYRKKNKFPHFKCEKCNFKENADYNAALNISNPKLKSTKEEP

SEQ ID NO: 231 - protein, 557 aa, synthetic construct
  source 1..557: note = Engineered CWCas12f (S170T)
MGEKSSRRRRNGKSGAWTAAITSCVGGKMAKNTITKTLKLRIVRPYNSAEVEKIVADEKNNREKIALEKNKDKVKEACSKHLKVAAYCTTQVERNACLFCKARKLDDKFYQKLRGQFPDAVFWQEISEIFRQLQKQAAEIYNQSLIELYYEIFIKGKGIANASSVEHYLTDVCYTRAAELFKNAAIASGLRSKIKSNFRLKELKNMKSGLPTTKSDNFPIPLVKQKGGQYTGFEISNHNSDFIIKIPFGRWQVKKEIDKYRPWEKFDFEQVQKSPKPISLLLSTQRRKRNKGWSKDEGTEAEIKKVMNGDYQTSYIEVKRGSKIGEKSAWMLNLSIDVPKIDKGVDPSIIGGIDVGVKSPLVCAINNAFSRYSISDNDLFHFNKKMFARRRILLKKNRHKRAGHGAKNKLKPITILTEKSERFRKKLIERWACEIADFFIKNKVGTVQMENLESMKRKEDSYFNIRLRGFWPYAEMQNKIEFKLKQYGIEIRKVAPNNTSKTCSKCGHLNNYFNFEYRKKNKFPHFKCEKCNFKENADYNAALNISNPKLKSTKEEP

SEQ ID NO: 232 - protein, 557 aa, synthetic construct
  source 1..557: note = Engineered CWCas12f (S170Y)
MGEKSSRRRRNGKSGAWTAAITSCVGGKMAKNTITKTLKLRIVRPYNSAEVEKIVADEKNNREKIALEKNKDKVKEACSKHLKVAAYCTTQVERNACLFCKARKLDDKFYQKLRGQFPDAVFWQEISEIFRQLQKQAAEIYNQSLIELYYEIFIKGKGIANASSVEHYLYDVCYTRAAELFKNAAIASGLRSKIKSNFRLKELKNMKSGLPTTKSDNFPIPLVKQKGGQYTGFEISNHNSDFIIKIPFGRWQVKKEIDKYRPWEKFDFEQVQKSPKPISLLLSTQRRKRNKGWSKDEGTEAEIKKVMNGDYQTSYIEVKRGSKIGEKSAWMLNLSIDVPKIDKGVDPSIIGGIDVGVKSPLVCAINNAFSRYSISDNDLFHFNKKMFARRRILLKKNRHKRAGHGAKNKLKPITILTEKSERFRKKLIERWACEIADFFIKNKVGTVQMENLESMKRKEDSYFNIRLRGFWPYAEMQNKIEFKLKQYGIEIRKVAPNNTSKTCSKCGHLNNYFNFEYRKKNKFPHFKCEKCNFKENADYNAALNISNPKLKSTKEEP

SEQ ID NO: 233 - protein, 557 aa, synthetic construct
  source 1..557: note = Engineered CWCas12f (Y174H)
MGEKSSRRRRNGKSGAWTAAITSCVGGKMAKNTITKTLKLRIVRPYNSAEVEKIVADEKNNREKIALEKNKDKVKEACSKHLKVAAYCTTQVERNACLFCKARKLDDKFYQKLRGQFPDAVFWQEISEIFRQLQKQAAEIYNQSLIELYYEIFIKGKGIANASSVEHYLSDVCHTRAAELFKNAAIASGLRSKIKSNFRLKELKNMKSGLPTTKSDNFPIPLVKQKGGQYTGFEISNHNSDFIIKIPFGRWQVKKEIDKYRPWEKFDFEQVQKSPKPISLLLSTQRRKRNKGWSKDEGTEAEIKKVMNGDYQTSYIEVKRGSKIGEKSAWMLNLSIDVPKIDKGVDPSIIGGIDVGVKSPLVCAINNAFSRYSISDNDLFHFNKKMFARRRILLKKNRHKRAGHGAKNKLKPITILTEKSERFRKKLIERWACEIADFFIKNKVGTVQMENLESMKRKEDSYFNIRLRGFWPYAEMQNKIEFKLKQYGIEIRKVAPNNTSKTCSKCGHLNNYFNFEYRKKNKFPHFKCEKCNFKENADYNAALNISNPKLKSTKEEP

SEQ ID NO: 234 - protein, 557 aa, synthetic construct
  source 1..557: note = Engineered CWCas12f (Y174K)
MGEKSSRRRRNGKSGAWTAAITSCVGGKMAKNTITKTLKLRIVRPYNSAEVEKIVADEKNNREKIALEKNKDKVKEACSKHLKVAAYCTTQVERNACLFCKARKLDDKFYQKLRGQFPDAVFWQEISEIFRQLQKQAAEIYNQSLIELYYEIFIKGKGIANASSVEHYLSDVCKTRAAELFKNAAIASGLRSKIKSNFRLKELKNMKSGLPTTKSDNFPIPLVKQKGGQYTGFEISNHNSDFIIKIPFGRWQVKKEIDKYRPWEKFDFEQVQKSPKPISLLLSTQRRKRNKGWSKDEGTEAEIKKVMNGDYQTSYIEVKRGSKIGEKSAWMLNLSIDVPKIDKGVDPSIIGGIDVGVKSPLVCAINNAFSRYSISDNDLFHFNKKMFARRRILLKKNRHKRAGHGAKNKLKPITILTEKSERFRKKLIERWACEIADFFIKNKVGTVQMENLESMKRKEDSYFNIRLRGFWPYAEMQNKIEFKLKQYGIEIRKVAPNNTSKTCSKCGHLNNYFNFEYRKKNKFPHFKCEKCNFKENADYNAALNISNPKLKSTKEEP

SEQ ID NO: 235 - protein, 557 aa, synthetic construct
  source 1..557: note = Engineered CWCas12f (Y174T)
MGEKSSRRRRNGKSGAWTAAITSCVGGKMAKNTITKTLKLRIVRPYNSAEVEKIVADEKNNREKIALEKNKDKVKEACSKHLKVAAYCTTQVERNACLFCKARKLDDKFYQKLRGQFPDAVFWQEISEIFRQLQKQAAEIYNQSLIELYYEIFIKGKGIANASSVEHYLSDVCTTRAAELFKNAAIASGLRSKIKSNFRLKELKNMKSGLPTTKSDNFPIPLVKQKGGQYTGFEISNHNSDFIIKIPFGRWQVKKEIDKYRPWEKFDFEQVQKSPKPISLLLSTQRRKRNKGWSKDEGTEAEIKKVMNGDYQTSYIEVKRGSKIGEKSAWMLNLSIDVPKIDKGVDPSIIGGIDVGVKSPLVCAINNAFSRYSISDNDLFHFNKKMFARRRILLKKNRHKRAGHGAKNKLKPITILTEKSERFRKKLIERWACEIADFFIKNKVGTVQMENLESMKRKEDSYFNIRLRGFWPYAEMQNKIEFKLKQYGIEIRKVAPNNTSKTCSKCGHLNNYFNFEYRKKNKFPHFKCEKCNFKENADYNAALNISNPKLKSTKEEP

SEQ ID NO: 236 - protein, 557 aa, synthetic construct
  source 1..557: note = Engineered CWCas12f (A184G)
MGEKSSRRRRNGKSGAWTAAITSCVGGKMAKNTITKTLKLRIVRPYNSAEVEKIVADEKNNREKIALEKNKDKVKEACSKHLKVAAYCTTQVERNACLFCKARKLDDKFYQKLRGQFPDAVFWQEISEIFRQLQKQAAEIYNQSLIELYYEIFIKGKGIANASSVEHYLSDVCYTRAAELFKNGAIASGLRSKIKSNFRLKELKNMKSGLPTTKSDNFPIPLVKQKGGQYTGFEISNHNSDFIIKIPFGRWQVKKEIDKYRPWEKFDFEQVQKSPKPISLLLSTQRRKRNKGWSKDEGTEAEIKKVMNGDYQTSYIEVKRGSKIGEKSAWMLNLSIDVPKIDKGVDPSIIGGIDVGVKSPLVCAINNAFSRYSISDNDLFHFNKKMFARRRILLKKNRHKRAGHGAKNKLKPITILTEKSERFRKKLIERWACEIADFFIKNKVGTVQMENLESMKRKEDSYFNIRLRGFWPYAEMQNKIEFKLKQYGIEIRKVAPNNTSKTCSKCGHLNNYFNFEYRKKNKFPHFKCEKCNFKENADYNAALNISNPKLKSTKEEP

SEQ ID NO: 237 - protein, 557 aa, synthetic construct
  source 1..557: note = Engineered CWCas12f (A184H)
MGEKSSRRRRNGKSGAWTAAITSCVGGKMAKNTITKTLKLRIVRPYNSAEVEKIVADEKNNREKIALEKNKDKVKEACSKHLKVAAYCTTQVERNACLFCKARKLDDKFYQKLRGQFPDAVFWQEISEIFRQLQKQAAEIYNQSLIELYYEIFIKGKGIANASSVEHYLSDVCYTRAAELFKNHAIASGLRSKIKSNFRLKELKNMKSGLPTTKSDNFPIPLVKQKGGQYTGFEISNHNSDFIIKIPFGRWQVKKEIDKYRPWEKFDFEQVQKSPKPISLLLSTQRRKRNKGWSKDEGTEAEIKKVMNGDYQTSYIEVKRGSKIGEKSAWMLNLSIDVPKIDKGVDPSIIGGIDVGVKSPLVCAINNAFSRYSISDNDLFHFNKKMFARRRILLKKNRHKRAGHGAKNKLKPITILTEKSERFRKKLIERWACEIADFFIKNKVGTVQMENLESMKRKEDSYFNIRLRGFWPYAEMQNKIEFKLKQYGIEIRKVAPNNTSKTCSKCGHLNNYFNFEYRKKNKFPHFKCEKCNFKENADYNAALNISNPKLKSTKEEP

SEQ ID NO: 238 - protein, 557 aa, synthetic construct
  source 1..557: note = Engineered CWCas12f (A184N)
MGEKSSRRRRNGKSGAWTAAITSCVGGKMAKNTITKTLKLRIVRPYNSAEVEKIVADEKNNREKIALEKNKDKVKEACSKHLKVAAYCTTQVERNACLFCKARKLDDKFYQKLRGQFPDAVFWQEISEIFRQLQKQAAEIYNQSLIELYYEIFIKGKGIANASSVEHYLSDVCYTRAAELFKNNAIASGLRSKIKSNFRLKELKNMKSGLPTTKSDNFPIPLVKQKGGQYTGFEISNHNSDFIIKIPFGRWQVKKEIDKYRPWEKFDFEQVQKSPKPISLLLSTQRRKRNKGWSKDEGTEAEIKKVMNGDYQTSYIEVKRGSKIGEKSAWMLNLSIDVPKIDKGVDPSIIGGIDVGVKSPLVCAINNAFSRYSISDNDLFHFNKKMFARRRILLKKNRHKRAGHGAKNKLKPITILTEKSERFRKKLIERWACEIADFFIKNKVGTVQMENLESMKRKEDSYFNIRLRGFWPYAEMQNKIEFKLKQYGIEIRKVAPNNTSKTCSKCGHLNNYFNFEYRKKNKFPHFKCEKCNFKENADYNAALNISNPKLKSTKEEP

SEQ ID NO: 239 - protein, 557 aa, synthetic construct
  source 1..557: note = Engineered CWCas12f (A184R)
MGEKSSRRRRNGKSGAWTAAITSCVGGKMAKNTITKTLKLRIVRPYNSAEVEKIVADEKNNREKIALEKNKDKVKEACSKHLKVAAYCTTQVERNACLFCKARKLDDKFYQKLRGQFPDAVFWQEISEIFRQLQKQAAEIYNQSLIELYYEIFIKGKGIANASSVEHYLSDVCYTRAAELFKNRAIASGLRSKIKSNFRLKELKNMKSGLPTTKSDNFPIPLVKQKGGQYTGFEISNHNSDFIIKIPFGRWQVKKEIDKYRPWEKFDFEQVQKSPKPISLLLSTQRRKRNKGWSKDEGTEAEIKKVMNGDYQTSYIEVKRGSKIGEKSAWMLNLSIDVPKIDKGVDPSIIGGIDVGVKSPLVCAINNAFSRYSISDNDLFHFNKKMFARRRILLKKNRHKRAGHGAKNKLKPITILTEKSERFRKKLIERWACEIADFFIKNKVGTVQMENLESMKRKEDSYFNIRLRGFWPYAEMQNKIEFKLKQYGIEIRKVAPNNTSKTCSKCGHLNNYFNFEYRKKNKFPHFKCEKCNFKENADYNAALNISNPKLKSTKEEP

SEQ ID NO: 240 - protein, 557 aa, synthetic construct
  source 1..557: note = Engineered CWCas12f (A184S)
MGEKSSRRRRNGKSGAWTAAITSCVGGKMAKNTITKTLKLRIVRPYNSAEVEKIVADEKNNREKIALEKNKDKVKEACSKHLKVAAYCTTQVERNACLFCKARKLDDKFYQKLRGQFPDAVFWQEISEIFRQLQKQAAEIYNQSLIELYYEIFIKGKGIANASSVEHYLSDVCYTRAAELFKNSAIASGLRSKIKSNFRLKELKNMKSGLPTTKSDNFPIPLVKQKGGQYTGFEISNHNSDFIIKIPFGRWQVKKEIDKYRPWEKFDFEQVQKSPKPISLLLSTQRRKRNKGWSKDEGTEAEIKKVMNGDYQTSYIEVKRGSKIGEKSAWMLNLSIDVPKIDKGVDPSIIGGIDVGVKSPLVCAINNAFSRYSISDNDLFHFNKKMFARRRILLKKNRHKRAGHGAKNKLKPITILTEKSERFRKKLIERWACEIADFFIKNKVGTVQMENLESMKRKEDSYFNIRLRGFWPYAEMQNKIEFKLKQYGIEIRKVAPNNTSKTCSKCGHLNNYFNFEYRKKNKFPHFKCEKCNFKENADYNAALNISNPKLKSTKEEP

SEQ ID NO: 241 - protein, 557 aa, synthetic construct
  source 1..557: note = Engineered CWCas12f (A184W)
MGEKSSRRRRNGKSGAWTAAITSCVGGKMAKNTITKTLKLRIVRPYNSAEVEKIVADEKNNREKIALEKNKDKVKEACSKHLKVAAYCTTQVERNACLFCKARKLDDKFYQKLRGQFPDAVFWQEISEIFRQLQKQAAEIYNQSLIELYYEIFIKGKGIANASSVEHYLSDVCYTRAAELFKNWAIASGLRSKIKSNFRLKELKNMKSGLPTTKSDNFPIPLVKQKGGQYTGFEISNHNSDFIIKIPFGRWQVKKEIDKYRPWEKFDFEQVQKSPKPISLLLSTQRRKRNKGWSKDEGTEAEIKKVMNGDYQTSYIEVKRGSKIGEKSAWMLNLSIDVPKIDKGVDPSIIGGIDVGVKSPLVCAINNAFSRYSISDNDLFHFNKKMFARRRILLKKNRHKRAGHGAKNKLKPITILTEKSERFRKKLIERWACEIADFFIKNKVGTVQMENLESMKRKEDSYFNIRLRGFWPYAEMQNKIEFKLKQYGIEIRKVAPNNTSKTCSKCGHLNNYFNFEYRKKNKFPHFKCEKCNFKENADYNAALNISNPKLKSTKEEP

SEQ ID NO: 242 - protein, 557 aa, synthetic construct
  source 1..557: note = Engineered CWCas12f (S188H)
MGEKSSRRRRNGKSGAWTAAITSCVGGKMAKNTITKTLKLRIVRPYNSAEVEKIVADEKNNREKIALEKNKDKVKEACSKHLKVAAYCTTQVERNACLFCKARKLDDKFYQKLRGQFPDAVFWQEISEIFRQLQKQAAEIYNQSLIELYYEIFIKGKGIANASSVEHYLSDVCYTRAAELFKNAAIAHGLRSKIKSNFRLKELKNMKSGLPTTKSDNFPIPLVKQKGGQYTGFEISNHNSDFIIKIPFGRWQVKKEIDKYRPWEKFDFEQVQKSPKPISLLLSTQRRKRNKGWSKDEGTEAEIKKVMNGDYQTSYIEVKRGSKIGEKSAWMLNLSIDVPKIDKGVDPSIIGGIDVGVKSPLVCAINNAFSRYSISDNDLFHFNKKMFARRRILLKKNRHKRAGHGAKNKLKPITILTEKSERFRKKLIERWACEIADFFIKNKVGTVQMENLESMKRKEDSYFNIRLRGFWPYAEMQNKIEFKLKQYGIEIRKVAPNNTSKTCSKCGHLNNYFNFEYRKKNKFPHFKCEKCNFKENADYNAALNISNPKLKSTKEEP

SEQ ID NO: 243 - protein, 557 aa, synthetic construct
  source 1..557: note = Engineered CWCas12f (S188K)
MGEKSSRRRRNGKSGAWTAAITSCVGGKMAKNTITKTLKLRIVRPYNSAEVEKIVADEKNNREKIALEKNKDKVKEACSKHLKVAAYCTTQVERNACLFCKARKLDDKFYQKLRGQFPDAVFWQEISEIFRQLQKQAAEIYNQSLIELYYEIFIKGKGIANASSVEHYLSDVCYTRAAELFKNAAIAKGLRSKIKSNFRLKELKNMKSGLPTTKSDNFPIPLVKQKGGQYTGFEISNHNSDFIIKIPFGRWQVKKEIDKYRPWEKFDFEQVQKSPKPISLLLSTQRRKRNKGWSKDEGTEAEIKKVMNGDYQTSYIEVKRGSKIGEKSAWMLNLSIDVPKIDKGVDPSIIGGIDVGVKSPLVCAINNAFSRYSISDNDLFHFNKKMFARRRILLKKNRHKRAGHGAKNKLKPITILTEKSERFRKKLIERWACEIADFFIKNKVGTVQMENLESMKRKEDSYFNIRLRGFWPYAEMQNKIEFKLKQYGIEIRKVAPNNTSKTCSKCGHLNNYFNFEYRKKNKFPHFKCEKCNFKENADYNAALNISNPKLKSTKEEP

SEQ ID NO: 244 - protein, 557 aa, synthetic construct
  source 1..557: note = Engineered CWCas12f (S188N)
MGEKSSRRRRNGKSGAWTAAITSCVGGKMAKNTITKTLKLRIVRPYNSAEVEKIVADEKNNREKIALEKNKDKVKEACSKHLKVAAYCTTQVERNACLFCKARKLDDKFYQKLRGQFPDAVFWQEISEIFRQLQKQAAEIYNQSLIELYYEIFIKGKGIANASSVEHYLSDVCYTRAAELFKNAAIANGLRSKIKSNFRLKELKNMKSGLPTTKSDNFPIPLVKQKGGQYTGFEISNHNSDFIIKIPFGRWQVKKEIDKYRPWEKFDFEQVQKSPKPISLLLSTQRRKRNKGWSKDEGTEAEIKKVMNGDYQTSYIEVKRGSKIGEKSAWMLNLSIDVPKIDKGVDPSIIGGIDVGVKSPLVCAINNAFSRYSISDNDLFHFNKKMFARRRILLKKNRHKRAGHGAKNKLKPITILTEKSERFRKKLIERWACEIADFFIKNKVGTVQMENLESMKRKEDSYFNIRLRGFWPYAEMQNKIEFKLKQYGIEIRKVAPNNTSKTCSKCGHLNNYFNFEYRKKNKFPHFKCEKCNFKENADYNAALNISNPKLKSTKEEP

SEQ ID NO: 245 - protein, 557 aa, synthetic construct
  source 1..557: note = Engineered CWCas12f (S188Q)
MGEKSSRRRRNGKSGAWTAAITSCVGGKMAKNTITKTLKLRIVRPYNSAEVEKIVADEKNNREKIALEKNKDKVKEACSKHLKVAAYCTTQVERNACLFCKARKLDDKFYQKLRGQFPDAVFWQEISEIFRQLQKQAAEIYNQSLIELYYEIFIKGKGIANASSVEHYLSDVCYTRAAELFKNAAIAQGLRSKIKSNFRLKELKNMKSGLPTTKSDNFPIPLVKQKGGQYTGFEISNHNSDFIIKIPFGRWQVKKEIDKYRPWEKFDFEQVQKSPKPISLLLSTQRRKRNKGWSKDEGTEAEIKKVMNGDYQTSYIEVKRGSKIGEKSAWMLNLSIDVPKIDKGVDPSIIGGIDVGVKSPLVCAINNAFSRYSISDNDLFHFNKKMFARRRILLKKNRHKRAGHGAKNKLKPITILTEKSERFRKKLIERWACEIADFFIKNKVGTVQMENLESMKRKEDSYFNIRLRGFWPYAEMQNKIEFKLKQYGIEIRKVAPNNTSKTCSKCGHLNNYFNFEYRKKNKFPHFKCEKCNFKENADYNAALNISNPKLKSTKEEP

SEQ ID NO: 246 - protein, 557 aa, synthetic construct
  source 1..557: note = Engineered CWCas12f (S188R)
MGEKSSRRRRNGKSGAWTAAITSCVGGKMAKNTITKTLKLRIVRPYNSAEVEKIVADEKNNREKIALEKNKDKVKEACSKHLKVAAYCTTQVERNACLFCKARKLDDKFYQKLRGQFPDAVFWQEISEIFRQLQKQAAEIYNQSLIELYYEIFIKGKGIANASSVEHYLSDVCYTRAAELFKNAAIARGLRSKIKSNFRLKELKNMKSGLPTTKSDNFPIPLVKQKGGQYTGFEISNHNSDFIIKIPFGRWQVKKEIDKYRPWEKFDFEQVQKSPKPISLLLSTQRRKRNKGWSKDEGTEAEIKKVMNGDYQTSYIEVKRGSKIGEKSAWMLNLSIDVPKIDKGVDPSIIGGIDVGVKSPLVCAINNAFSRYSISDNDLFHFNKKMFARRRILLKKNRHKRAGHGAKNKLKPITILTEKSERFRKKLIERWACEIADFFIKNKVGTVQMENLESMKRKEDSYFNIRLRGFWPYAEMQNKIEFKLKQYGIEIRKVAPNNTSKTCSKCGHLNNYFNFEYRKKNKFPHFKCEKCNFKENADYNAALNISNPKLKSTKEEP

SEQ ID NO: 247 - protein, 557 aa, synthetic construct
  source 1..557: note = Engineered CWCas12f (R191K)
MGEKSSRRRRNGKSGAWTAAITSCVGGKMAKNTITKTLKLRIVRPYNSAEVEKIVADEKNNREKIALEKNKDKVKEACSKHLKVAAYCTTQVERNACLFCKARKLDDKFYQKLRGQFPDAVFWQEISEIFRQLQKQAAEIYNQSLIELYYEIFIKGKGIANASSVEHYLSDVCYTRAAELFKNAAIASGLKSKIKSNFRLKELKNMKSGLPTTKSDNFPIPLVKQKGGQYTGFEISNHNSDFIIKIPFGRWQVKKEIDKYRPWEKFDFEQVQKSPKPISLLLSTQRRKRNKGWSKDEGTEAEIKKVMNGDYQTSYIEVKRGSKIGEKSAWMLNLSIDVPKIDKGVDPSIIGGIDVGVKSPLVCAINNAFSRYSISDNDLFHFNKKMFARRRILLKKNRHKRAGHGAKNKLKPITILTEKSERFRKKLIERWACEIADFFIKNKVGTVQMENLESMKRKEDSYFNIRLRGFWPYAEMQNKIEFKLKQYGIEIRKVAPNNTSKTCSKCGHLNNYFNFEYRKKNKFPHFKCEKCNFKENADYNAALNISNPKLKSTKEEP

SEQ ID NO: 248 - protein, 557 aa, synthetic construct
  source 1..557: note = Engineered CWCas12f (R191Q)
MGEKSSRRRRNGKSGAWTAAITSCVGGKMAKNTITKTLKLRIVRPYNSAEVEKIVADEKNNREKIALEKNKDKVKEACSKHLKVAAYCTTQVERNACLFCKARKLDDKFYQKLRGQFPDAVFWQEISEIFRQLQKQAAEIYNQSLIELYYEIFIKGKGIANASSVEHYLSDVCYTRAAELFKNAAIASGLQSKIKSNFRLKELKNMKSGLPTTKSDNFPIPLVKQKGGQYTGFEISNHNSDFIIKIPFGRWQVKKEIDKYRPWEKFDFEQVQKSPKPISLLLSTQRRKRNKGWSKDEGTEAEIKKVMNGDYQTSYIEVKRGSKIGEKSAWMLNLSIDVPKIDKGVDPSIIGGIDVGVKSPLVCAINNAFSRYSISDNDLFHFNKKMFARRRILLKKNRHKRAGHGAKNKLKPITILTEKSERFRKKLIERWACEIADFFIKNKVGTVQMENLESMKRKEDSYFNIRLRGFWPYAEMQNKIEFKLKQYGIEIRKVAPNNTSKTCSKCGHLNNYFNFEYRKKNKFPHFKCEKCNFKENADYNAALNISNPKLKSTKEEP

SEQ ID NO: 249 - protein, 557 aa, synthetic construct
  source 1..557: note = Engineered CWCas12f (R191W)
MGEKSSRRRRNGKSGAWTAAITSCVGGKMAKNTITKTLKLRIVRPYNSAEVEKIVADEKNNREKIALEKNKDKVKEACSKHLKVAAYCTTQVERNACLFCKARKLDDKFYQKLRGQFPDAVFWQEISEIFRQLQKQAAEIYNQSLIELYYEIFIKGKGIANASSVEHYLSDVCYTRAAELFKNAAIASGLWSKIKSNFRLKELKNMKSGLPTTKSDNFPIPLVKQKGGQYTGFEISNHNSDFIIKIPFGRWQVKKEIDKYRPWEKFDFEQVQKSPKPISLLLSTQRRKRNKGWSKDEGTEAEIKKVMNGDYQTSYIEVKRGSKIGEKSAWMLNLSIDVPKIDKGVDPSIIGGIDVGVKSPLVCAINNAFSRYSISDNDLFHFNKKMFARRRILLKKNRHKRAGHGAKNKLKPITILTEKSERFRKKLIERWACEIADFFIKNKVGTVQMENLESMKRKEDSYFNIRLRGFWPYAEMQNKIEFKLKQYGIEIRKVAPNNTSKTCSKCGHLNNYFNFEYRKKNKFPHFKCEKCNFKENADYNAALNISNPKLKSTKEEP

SEQ ID NO: 250 - protein, 557 aa, synthetic construct
  source 1..557: note = Engineered CWCas12f (Q225F)
MGEKSSRRRRNGKSGAWTAAITSCVGGKMAKNTITKTLKLRIVRPYNSAEVEKIVADEKNNREKIALEKNKDKVKEACSKHLKVAAYCTTQVERNACLFCKARKLDDKFYQKLRGQFPDAVFWQEISEIFRQLQKQAAEIYNQSLIELYYEIFIKGKGIANASSVEHYLSDVCYTRAAELFKNAAIASGLRSKIKSNFRLKELKNMKSGLPTTKSDNFPIPLVKFKGGQYTGFEISNHNSDFIIKIPFGRWQVKKEIDKYRPWEKFDFEQVQKSPKPISLLLSTQRRKRNKGWSKDEGTEAEIKKVMNGDYQTSYIEVKRGSKIGEKSAWMLNLSIDVPKIDKGVDPSIIGGIDVGVKSPLVCAINNAFSRYSISDNDLFHFNKKMFARRRILLKKNRHKRAGHGAKNKLKPITILTEKSERFRKKLIERWACEIADFFIKNKVGTVQMENLESMKRKEDSYFNIRLRGFWPYAEMQNKIEFKLKQYGIEIRKVAPNNTSKTCSKCGHLNNYFNFEYRKKNKFPHFKCEKCNFKENADYNAALNISNPKLKSTKEEP

SEQ ID NO: 251 - protein, 557 aa, synthetic construct
  source 1..557: note = Engineered CWCas12f (Q225R)
MGEKSSRRRRNGKSGAWTAAITSCVGGKMAKNTITKTLKLRIVRPYNSAEVEKIVADEKNNREKIALEKNKDKVKEACSKHLKVAAYCTTQVERNACLFCKARKLDDKFYQKLRGQFPDAVFWQEISEIFRQLQKQAAEIYNQSLIELYYEIFIKGKGIANASSVEHYLSDVCYTRAAELFKNAAIASGLRSKIKSNFRLKELKNMKSGLPTTKSDNFPIPLVKRKGGQYTGFEISNHNSDFIIKIPFGRWQVKKEIDKYRPWEKFDFEQVQKSPKPISLLLSTQRRKRNKGWSKDEGTEAEIKKVMNGDYQTSYIEVKRGSKIGEKSAWMLNLSIDVPKIDKGVDPSIIGGIDVGVKSPLVCAINNAFSRYSISDNDLFHFNKKMFARRRILLKKNRHKRAGHGAKNKLKPITILTEKSERFRKKLIERWACEIADFFIKNKVGTVQMENLESMKRKEDSYFNIRLRGFWPYAEMQNKIEFKLKQYGIEIRKVAPNNTSKTCSKCGHLNNYFNFEYRKKNKFPHFKCEKCNFKENADYNAALNISNPKLKSTKEEP

SEQ ID NO: 252 - protein, 557 aa, synthetic construct
  source 1..557: note = Engineered CWCas12f (Q225T)
MGEKSSRRRRNGKSGAWTAAITSCVGGKMAKNTITKTLKLRIVRPYNSAEVEKIVADEKNNREKIALEKNKDKVKEACSKHLKVAAYCTTQVERNACLFCKARKLDDKFYQKLRGQFPDAVFWQEISEIFRQLQKQAAEIYNQSLIELYYEIFIKGKGIANASSVEHYLSDVCYTRAAELFKNAAIASGLRSKIKSNFRLKELKNMKSGLPTTKSDNFPIPLVKTKGGQYTGFEISNHNSDFIIKIPFGRWQVKKEIDKYRPWEKFDFEQVQKSPKPISLLLSTQRRKRNKGWSKDEGTEAEIKKVMNGDYQTSYIEVKRGSKIGEKSAWMLNLSIDVPKIDKGVDPSIIGGIDVGVKSPLVCAINNAFSRYSISDNDLFHFNKKMFARRRILLKKNRHKRAGHGAKNKLKPITILTEKSERFRKKLIERWACEIADFFIKNKVGTVQMENLESMKRKEDSYFNIRLRGFWPYAEMQNKIEFKLKQYGIEIRKVAPNNTSKTCSKCGHLNNYFNFEYRKKNKFPHFKCEKCNFKENADYNAALNISNPKLKSTKEEP

SEQ ID NO: 253 - protein, 557 aa, synthetic construct
  source 1..557: note = Engineered CWCas12f (Y230C)
MGEKSSRRRRNGKSGAWTAAITSCVGGKMAKNTITKTLKLRIVRPYNSAEVEKIVADEKNNREKIALEKNKDKVKEACSKHLKVAAYCTTQVERNACLFCKARKLDDKFYQKLRGQFPDAVFWQEISEIFRQLQKQAAEIYNQSLIELYYEIFIKGKGIANASSVEHYLSDVCYTRAAELFKNAAIASGLRSKIKSNFRLKELKNMKSGLPTTKSDNFPIPLVKQKGGQCTGFEISNHNSDFIIKIPFGRWQVKKEIDKYRPWEKFDFEQVQKSPKPISLLLSTQRRKRNKGWSKDEGTEAEIKKVMNGDYQTSYIEVKRGSKIGEKSAWMLNLSIDVPKIDKGVDPSIIGGIDVGVKSPLVCAINNAFSRYSISDNDLFHFNKKMFARRRILLKKNRHKRAGHGAKNKLKPITILTEKSERFRKKLIERWACEIADFFIKNKVGTVQMENLESMKRKEDSYFNIRLRGFWPYAEMQNKIEFKLKQYGIEIRKVAPNNTSKTCSKCGHLNNYFNFEYRKKNKFPHFKCEKCNFKENADYNAALNISNPKLKSTKEEP

SEQ ID NO: 254 - protein, 557 aa, synthetic construct
  source 1..557: note = Engineered CWCas12f (Y230H)
MGEKSSRRRRNGKSGAWTAAITSCVGGKMAKNTITKTLKLRIVRPYNSAEVEKIVADEKNNREKIALEKNKDKVKEACSKHLKVAAYCTTQVERNACLFCKARKLDDKFYQKLRGQFPDAVFWQEISEIFRQLQKQAAEIYNQSLIELYYEIFIKGKGIANASSVEHYLSDVCYTRAAELFKNAAIASGLRSKIKSNFRLKELKNMKSGLPTTKSDNFPIPLVKQKGGQHTGFEISNHNSDFIIKIPFGRWQVKKEIDKYRPWEKFDFEQVQKSPKPISLLLSTQRRKRNKGWSKDEGTEAEIKKVMNGDYQTSYIEVKRGSKIGEKSAWMLNLSIDVPKIDKGVDPSIIGGIDVGVKSPLVCAINNAFSRYSISDNDLFHFNKKMFARRRILLKKNRHKRAGHGAKNKLKPITILTEKSERFRKKLIERWACEIADFFIKNKVGTVQMENLESMKRKEDSYFNIRLRGFWPYAEMQNKIEFKLKQYGIEIRKVAPNNTSKTCSKCGHLNNYFNFEYRKKNKFPHFKCEKCNFKENADYNAALNISNPKLKSTKEEP

SEQ ID NO: 255 - protein, 557 aa, synthetic construct
  source 1..557: note = Engineered CWCas12f (Y230K)
MGEKSSRRRRNGKSGAWTAAITSCVGGKMAKNTITKTLKLRIVRPYNSAEVEKIVADEKNNREKIALEKNKDKVKEACSKHLKVAAYCTTQVERNACLFCKARKLDDKFYQKLRGQFPDAVFWQEISEIFRQLQKQAAEIYNQSLIELYYEIFIKGKGIANASSVEHYLSDVCYTRAAELFKNAAIASGLRSKIKSNFRLKELKNMKSGLPTTKSDNFPIPLVKQKGGQKTGFEISNHNSDFIIKIPFGRWQVKKEIDKYRPWEKFDFEQVQKSPKPISLLLSTQRRKRNKGWSKDEGTEAEIKKVMNGDYQTSYIEVKRGSKIGEKSAWMLNLSIDVPKIDKGVDPSIIGGIDVGVKSPLVCAINNAFSRYSISDNDLFHFNKKMFARRRILLKKNRHKRAGHGAKNKLKPITILTEKSERFRKKLIERWACEIADFFIKNKVGTVQMENLESMKRKEDSYFNIRLRGFWPYAEMQNKIEFKLKQYGIEIRKVAPNNTSKTCSKCGHLNNYFNFEYRKKNKFPHFKCEKCNFKENADYNAALNISNPKLKSTKEEP

SEQ ID NO: 256 - protein, 557 aa, synthetic construct
  source 1..557: note = Engineered CWCas12f (Y230R)
MGEKSSRRRRNGKSGAWTAAITSCVGGKMAKNTITKTLKLRIVRPYNSAEVEKIVADEKNNREKIALEKNKDKVKEACSKHLKVAAYCTTQVERNACLFCKARKLDDKFYQKLRGQFPDAVFWQEISEIFRQLQKQAAEIYNQSLIELYYEIFIKGKGIANASSVEHYLSDVCYTRAAELFKNAAIASGLRSKIKSNFRLKELKNMKSGLPTTKSDNFPIPLVKQKGGQRTGFEISNHNSDFIIKIPFGRWQVKKEIDKYRPWEKFDFEQVQKSPKPISLLLSTQRRKRNKGWSKDEGTEAEIKKVMNGDYQTSYIEVKRGSKIGEKSAWMLNLSIDVPKIDKGVDPSIIGGIDVGVKSPLVCAINNAFSRYSISDNDLFHFNKKMFARRRILLKKNRHKRAGHGAKNKLKPITILTEKSERFRKKLIERWACEIADFFIKNKVGTVQMENLESMKRKEDSYFNIRLRGFWPYAEMQNKIEFKLKQYGIEIRKVAPNNTSKTCSKCGHLNNYFNFEYRKKNKFPHFKCEKCNFKENADYNAALNISNPKLKSTKEEP

SEQ ID NO: 257 - protein, 557 aa, synthetic construct
  source 1..557: note = Engineered CWCas12f (Y230S)
MGEKSSRRRRNGKSGAWTAAITSCVGGKMAKNTITKTLKLRIVRPYNSAEVEKIVADEKNNREKIALEKNKDKVKEACSKHLKVAAYCTTQVERNACLFCKARKLDDKFYQKLRGQFPDAVFWQEISEIFRQLQKQAAEIYNQSLIELYYEIFIKGKGIANASSVEHYLSDVCYTRAAELFKNAAIASGLRSKIKSNFRLKELKNMKSGLPTTKSDNFPIPLVKQKGGQSTGFEISNHNSDFIIKIPFGRWQVKKEIDKYRPWEKFDFEQVQKSPKPISLLLSTQRRKRNKGWSKDEGTEAEIKKVMNGDYQTSYIEVKRGSKIGEKSAWMLNLSIDVPKIDKGVDPSIIGGIDVGVKSPLVCAINNAFSRYSISDNDLFHFNKKMFARRRILLKKNRHKRAGHGAKNKLKPITILTEKSERFRKKLIERWACEIADFFIKNKVGTVQMENLESMKRKEDSYFNIRLRGFWPYAEMQNKIEFKLKQYGIEIRKVAPNNTSKTCSKCGHLNNYFNFEYRKKNKFPHFKCEKCNFKENADYNAALNISNPKLKSTKEEP

SEQ ID NO: 258 - protein, 557 aa, synthetic construct
  source 1..557: note = Engineered CWCas12f (Y230T)
MGEKSSRRRRNGKSGAWTAAITSCVGGKMAKNTITKTLKLRIVRPYNSAEVEKIVADEKNNREKIALEKNKDKVKEACSKHLKVAAYCTTQVERNACLFCKARKLDDKFYQKLRGQFPDAVFWQEISEIFRQLQKQAAEIYNQSLIELYYEIFIKGKGIANASSVEHYLSDVCYTRAAELFKNAAIASGLRSKIKSNFRLKELKNMKSGLPTTKSDNFPIPLVKQKGGQTTGFEISNHNSDFIIKIPFGRWQVKKEIDKYRPWEKFDFEQVQKSPKPISLLLSTQRRKRNKGWSKDEGTEAEIKKVMNGDYQTSYIEVKRGSKIGEKSAWMLNLSIDVPKIDKGVDPSIIGGIDVGVKSPLVCAINNAFSRYSISDNDLFHFNKKMFARRRILLKKNRHKRAGHGAKNKLKPITILTEKSERFRKKLIERWACEIADFFIKNKVGTVQMENLESMKRKEDSYFNIRLRGFWPYAEMQNKIEFKLKQYGIEIRKVAPNNTSKTCSKCGHLNNYFNFEYRKKNKFPHFKCEKCNFKENADYNAALNISNPKLKSTKEEP

SEQ ID NO: 259 - protein, 557 aa, synthetic construct
  source 1..557: note = Engineered CWCas12f (V271T)
MGEKSSRRRRNGKSGAWTAAITSCVGGKMAKNTITKTLKLRIVRPYNSAEVEKIVADEKNNREKIALEKNKDKVKEACSKHLKVAAYCTTQVERNACLFCKARKLDDKFYQKLRGQFPDAVFWQEISEIFRQLQKQAAEIYNQSLIELYYEIFIKGKGIANASSVEHYLSDVCYTRAAELFKNAAIASGLRSKIKSNFRLKELKNMKSGLPTTKSDNFPIPLVKQKGGQYTGFEISNHNSDFIIKIPFGRWQVKKEIDKYRPWEKFDFEQTQKSPKPISLLLSTQRRKRNKGWSKDEGTEAEIKKVMNGDYQTSYIEVKRGSKIGEKSAWMLNLSIDVPKIDKGVDPSIIGGIDVGVKSPLVCAINNAFSRYSISDNDLFHFNKKMFARRRILLKKNRHKRAGHGAKNKLKPITILTEKSERFRKKLIERWACEIADFFIKNKVGTVQMENLESMKRKEDSYFNIRLRGFWPYAEMQNKIEFKLKQYGIEIRKVAPNNTSKTCSKCGHLNNYFNFEYRKKNKFPHFKCEKCNFKENADYNAALNISNPKLKSTKEEP

SEQ ID NO: 260 - protein, 557 aa, synthetic construct
  source 1..557: note = Engineered CWCas12f (Q272C)
MGEKSSRRRRNGKSGAWTAAITSCVGGKMAKNTITKTLKLRIVRPYNSAEVEKIVADEKNNREKIALEKNKDKVKEACSKHLKVAAYCTTQVERNACLFCKARKLDDKFYQKLRGQFPDAVFWQEISEIFRQLQKQAAEIYNQSLIELYYEIFIKGKGIANASSVEHYLSDVCYTRAAELFKNAAIASGLRSKIKSNFRLKELKNMKSGLPTTKSDNFPIPLVKQKGGQYTGFEISNHNSDFIIKIPFGRWQVKKEIDKYRPWEKFDFEQVCKSPKPISLLLSTQRRKRNKGWSKDEGTEAEIKKVMNGDYQTSYIEVKRGSKIGEKSAWMLNLSIDVPKIDKGVDPSIIGGIDVGVKSPLVCAINNAFSRYSISDNDLFHFNKKMFARRRILLKKNRHKRAGHGAKNKLKPITILTEKSERFRKKLIERWACEIADFFIKNKVGTVQMENLESMKRKEDSYFNIRLRGFWPYAEMQNKIEFKLKQYGIEIRKVAPNNTSKTCSKCGHLNNYFNFEYRKKNKFPHFKCEKCNFKENADYNAALNISNPKLKSTKEEP

SEQ ID NO: 261 - protein, 557 aa, synthetic construct
  source 1..557: note = Engineered CWCas12f (Q272K)
MGEKSSRRRRNGKSGAWTAAITSCVGGKMAKNTITKTLKLRIVRPYNSAEVEKIVADEKNNREKIALEKNKDKVKEACSKHLKVAAYCTTQVERNACLFCKARKLDDKFYQKLRGQFPDAVFWQEISEIFRQLQKQAAEIYNQSLIELYYEIFIKGKGIANASSVEHYLSDVCYTRAAELFKNAAIASGLRSKIKSNFRLKELKNMKSGLPTTKSDNFPIPLVKQKGGQYTGFEISNHNSDFIIKIPFGRWQVKKEIDKYRPWEKFDFEQVKKSPKPISLLLSTQRRKRNKGWSKDEGTEAEIKKVMNGDYQTSYIEVKRGSKIGEKSAWMLNLSIDVPKIDKGVDPSIIGGIDVGVKSPLVCAINNAFSRYSISDNDLFHFNKKMFARRRILLKKNRHKRAGHGAKNKLKPITILTEKSERFRKKLIERWACEIADFFIKNKVGTVQMENLESMKRKEDSYFNIRLRGFWPYAEMQNKIEFKLKQYGIEIRKVAPNNTSKTCSKCGHLNNYFNFEYRKKNKFPHFKCEKCNFKENADYNAALNISNPKLKSTKEEP

SEQ ID NO: 262 - protein, 557 aa, synthetic construct
  source 1..557: note = Engineered CWCas12f (Q272R)
MGEKSSRRRRNGKSGAWTAAITSCVGGKMAKNTITKTLKLRIVRPYNSAEVEKIVADEKNNREKIALEKNKDKVKEACSKHLKVAAYCTTQVERNACLFCKARKLDDKFYQKLRGQFPDAVFWQEISEIFRQLQKQAAEIYNQSLIELYYEIFIKGKGIANASSVEHYLSDVCYTRAAELFKNAAIASGLRSKIKSNFRLKELKNMKSGLPTTKSDNFPIPLVKQKGGQYTGFEISNHNSDFIIKIPFGRWQVKKEIDKYRPWEKFDFEQVRKSPKPISLLLSTQRRKRNKGWSKDEGTEAEIKKVMNGDYQTSYIEVKRGSKIGEKSAWMLNLSIDVPKIDKGVDPSIIGGIDVGVKSPLVCAINNAFSRYSISDNDLFHFNKKMFARRRILLKKNRHKRAGHGAKNKLKPITILTEKSERFRKKLIERWACEIADFFIKNKVGTVQMENLESMKRKEDSYFNIRLRGFWPYAEMQNKIEFKLKQYGIEIRKVAPNNTSKTCSKCGHLNNYFNFEYRKKNKFPHFKCEKCNFKENADYNAALNISNPKLKSTKEEP

SEQ ID NO: 263 - protein, 557 aa, synthetic construct
  source 1..557: note = Engineered CWCas12f (S188Q/Q272K)
MGEKSSRRRRNGKSGAWTAAITSCVGGKMAKNTITKTLKLRIVRPYNSAEVEKIVADEKNNREKIALEKNKDKVKEACSKHLKVAAYCTTQVERNACLFCKARKLDDKFYQKLRGQFPDAVFWQEISEIFRQLQKQAAEIYNQSLIELYYEIFIKGKGIANASSVEHYLSDVCYTRAAELFKNAAIAQGLRSKIKSNFRLKELKNMKSGLPTTKSDNFPIPLVKQKGGQYTGFEISNHNSDFIIKIPFGRWQVKKEIDKYRPWEKFDFEQVKKSPKPISLLLSTQRRKRNKGWSKDEGTEAEIKKVMNGDYQTSYIEVKRGSKIGEKSAWMLNLSIDVPKIDKGVDPSIIGGIDVGVKSPLVCAINNAFSRYSISDNDLFHFNKKMFARRRILLKKNRHKRAGHGAKNKLKPITILTEKSERFRKKLIERWACEIADFFIKNKVGTVQMENLESMKRKEDSYFNIRLRGFWPYAEMQNKIEFKLKQYGIEIRKVAPNNTSKTCSKCGHLNNYFNFEYRKKNKFPHFKCEKCNFKENADYNAALNISNPKLKSTKEEP

SEQ ID NO: 264 - protein, 557 aa, synthetic construct
  source 1..557: note = Engineered CWCas12f (S188K/Q272K)
MGEKSSRRRRNGKSGAWTAAITSCVGGKMAKNTITKTLKLRIVRPYNSAEVEKIVADEKNNREKIALEKNKDKVKEACSKHLKVAAYCTTQVERNACLFCKARKLDDKFYQKLRGQFPDAVFWQEISEIFRQLQKQAAEIYNQSLIELYYEIFIKGKGIANASSVEHYLSDVCYTRAAELFKNAAIAKGLRSKIKSNFRLKELKNMKSGLPTTKSDNFPIPLVKQKGGQYTGFEISNHNSDFIIKIPFGRWQVKKEIDKYRPWEKFDFEQVKKSPKPISLLLSTQRRKRNKGWSKDEGTEAEIKKVMNGDYQTSYIEVKRGSKIGEKSAWMLNLSIDVPKIDKGVDPSIIGGIDVGVKSPLVCAINNAFSRYSISDNDLFHFNKKMFARRRILLKKNRHKRAGHGAKNKLKPITILTEKSERFRKKLIERWACEIADFFIKNKVGTVQMENLESMKRKEDSYFNIRLRGFWPYAEMQNKIEFKLKQYGIEIRKVAPNNTSKTCSKCGHLNNYFNFEYRKKNKFPHFKCEKCNFKENADYNAALNISNPKLKSTKEEP

SEQ ID NO: 265 - protein, 557 aa, synthetic construct
  source 1..557: note = Engineered CWCas12f (S188Q/R191K/Q272K)
MGEKSSRRRRNGKSGAWTAAITSCVGGKMAKNTITKTLKLRIVRPYNSAEVEKIVADEKNNREKIALEKNKDKVKEACSKHLKVAAYCTTQVERNACLFCKARKLDDKFYQKLRGQFPDAVFWQEISEIFRQLQKQAAEIYNQSLIELYYEIFIKGKGIANASSVEHYLSDVCYTRAAELFKNAAIAQGLKSKIKSNFRLKELKNMKSGLPTTKSDNFPIPLVKQKGGQYTGFEISNHNSDFIIKIPFGRWQVKKEIDKYRPWEKFDFEQVKKSPKPISLLLSTQRRKRNKGWSKDEGTEAEIKKVMNGDYQTSYIEVKRGSKIGEKSAWMLNLSIDVPKIDKGVDPSIIGGIDVGVKSPLVCAINNAFSRYSISDNDLFHFNKKMFARRRILLKKNRHKRAGHGAKNKLKPITILTEKSERFRKKLIERWACEIADFFIKNKVGTVQMENLESMKRKEDSYFNIRLRGFWPYAEMQNKIEFKLKQYGIEIRKVAPNNTSKTCSKCGHLNNYFNFEYRKKNKFPHFKCEKCNFKENADYNAALNISNPKLKSTKEEP

SEQ ID NO: 266 - DNA, 20 bp, unidentified
  source 1..20: mol_type = other DNA; note = LOC105370393 - protospacer
aagaaagctacaggaaagca

SEQ ID NO: 267 - DNA, 20 bp, synthetic construct
  source 1..20: mol_type = other DNA; note = LOC105370393 - forward primer
tgaccagggagttcctcaca

SEQ ID NO: 268 - DNA, 20 bp, synthetic construct
  source 1..20: mol_type = other DNA; note = LOC105370393 - reverse primer
gaagccgagctcagttaccc

SEQ ID NO: 269 - DNA, 20 bp, unidentified
  source 1..20: mol_type = other DNA; note = intergenic - protospacer
aagaggggaggttgactttg

SEQ ID NO: 270 - DNA, 20 bp, synthetic construct
  source 1..20: mol_type = other DNA; note = intergenic - forward primer
cctcccagatcccactcaga

SEQ ID NO: 271 - DNA, 20 bp, synthetic construct
  source 1..20: mol_type = other DNA; note = intergenic - reverse primer
cccaaagtcaacctcccctc

SEQ ID NO: 272 - DNA, 20 bp, unidentified
  source 1..20: mol_type = other DNA; note = ZNF10 - protospacer
aataagtcttaccacgtgtc

SEQ ID NO: 273 - DNA, 20 bp, synthetic construct
  source 1..20: mol_type = other DNA; note = ZNF10 - forward primer
gttcgtgccactgtactcca

SEQ ID NO: 274 - DNA, 20 bp, synthetic construct
  source 1..20: mol_type = other DNA; note = ZNF10 - reverse primer
ttctgcttccagccgagatg

SEQ ID NO: 275 - DNA, 20 bp, unidentified
  source 1..20: mol_type = other DNA; note = FUS - protospacer
acaaagaaaccagcagtggc

SEQ ID NO: 276 - DNA, 20 bp, synthetic construct
  source 1..20: mol_type = other DNA; note = FUS - forward primer
tacttcccctgccagcattg

SEQ ID NO: 277 - DNA, 20 bp, synthetic construct
  source 1..20: mol_type = other DNA; note = FUS - reverse primer
ggaagatccccccaaactgg

SEQ ID NO: 278 - DNA, 20 bp, unidentified
  source 1..20: mol_type = other DNA; note = OR4K17 - protospacer
acaagttcagaatcacctta

SEQ ID NO: 279 - DNA, 20 bp, synthetic construct
  source 1..20: mol_type = other DNA; note = OR4K17 - forward primer
tgaccagctcccaggatgta

SEQ ID NO: 280 - DNA, 20 bp, synthetic construct
  source 1..20: mol_type = other DNA; note = OR4K17 - reverse primer
gtgaaggagacccaagagcc

SEQ ID NO: 281 - DNA, 20 bp, unidentified
  source 1..20: mol_type = other DNA; note = POLRMT - protospacer
aggactatgtgtggccagtg

SEQ ID NO: 282 - DNA, 20 bp, synthetic construct
  source 1..20: mol_type = other DNA; note = POLRMT - forward primer
gagacggggtttcactgtgt

SEQ ID NO: 283 - DNA, 20 bp, synthetic construct
  source 1..20: mol_type = other DNA; note = POLRMT - reverse primer
ctctctgtctgttgcccagg

SEQ ID NO: 284 - DNA, 20 bp, unidentified
  source 1..20: mol_type = other DNA; note = LOC100128398 - protospacer
caaagaaatgtactgcctta

SEQ ID NO: 285 - DNA, 20 bp, synthetic construct
  source 1..20: mol_type = other DNA; note = LOC100128398 - forward primer
gggccactggtcaccatatt

SEQ ID NO: 286 - DNA, 20 bp, synthetic construct
  source 1..20: mol_type = other DNA; note = LOC100128398 - reverse primer
gcaccatgtcgtcccatttg

SEQ ID NO: 287 - DNA, 20 bp, unidentified
  source 1..20: mol_type = other DNA; note = CARS - protospacer
caacagcctcaccaggaaca

SEQ ID NO: 288 - DNA, 20 bp, synthetic construct
  source 1..20: mol_type = other DNA; note = CARS - forward primer
acaagccagggtgatccatg

SEQ ID NO: 289 - DNA, 20 bp, synthetic construct
  source 1..20: mol_type = other DNA; note = CARS - reverse primer
atcacaccactgcactctgg

SEQ ID NO: 290 - DNA, 20 bp, unidentified
  source 1..20: mol_type = other DNA; note = RPH3AL - protospacer
cacaagggatctgagacttg

SEQ ID NO: 291 - DNA, 20 bp, synthetic construct
  source 1..20: mol_type = other DNA; note = RPH3AL - forward primer
gcccctccgatcataagctc

SEQ ID NO: 292 - DNA, 20 bp, synthetic construct
  source 1..20: mol_type = other DNA; note = RPH3AL - reverse primer
gagggtgaagttgggtccag

SEQ ID NO: 293 - DNA, 20 bp, unidentified
  source 1..20: mol_type = other DNA; note = P2RX5-TAX1BP3 - protospacer
cacataggccattcagaaac

SEQ ID NO: 294 - DNA, 20 bp, synthetic construct
  source 1..20: mol_type = other DNA; note = P2RX5-TAX1BP3 - forward primer
gtctactgaaatgggggccc

SEQ ID NO: 295 - DNA, 20 bp, synthetic construct
  source 1..20: mol_type = other DNA; note = P2RX5-TAX1BP3 - reverse primer
ggccaggttggtcttgaact

SEQ ID NO: 296 - DNA, 20 bp, unidentified
  source 1..20: mol_type = other DNA; note = GAK - protospacer
cagagtcccgggaacaagcc

SEQ ID NO: 297 - DNA, 20 bp, synthetic construct
  source 1..20: mol_type = other DNA; note = GAK - forward primer
cagctcctcagaagagccag

SEQ ID NO: 298 - DNA, 20 bp, synthetic construct
  source 1..20: mol_type = other DNA; note = GAK - reverse primer
agtgagtgtgaggctccaga

SEQ ID NO: 299 - DNA, 20 bp, unidentified
  source 1..20: mol_type = other DNA; note = Intergene - protospacer
catacagggctctgtaccca

SEQ ID NO: 300 - DNA, 20 bp, synthetic construct
  source 1..20: mol_type = other DNA; note = Intergene - forward primer
ggcccagaaccttgctcttt

SEQ ID NO: 301 - DNA, 20 bp, synthetic construct
  source 1..20: mol_type = other DNA; note = Intergene - reverse primer
accaccctgcgtaacatagc

SEQ ID NO: 302 - DNA, 20 bp, unidentified
  source 1..20: mol_type = other DNA; note = Intergene - protospacer
ctgagatttgcgaagagtta

SEQ ID NO: 303 - DNA, 20 bp, synthetic construct
  source 1..20: mol_type = other DNA; note = Intergene - forward primer
gtggcagtggctgtattcct

SEQ ID NO: 304 - DNA, 20 bp, synthetic construct
  source 1..20: mol_type = other DNA; note = Intergene - reverse primer
gcttgaaagccaaagcctcc

SEQ ID NO: 305 - DNA, 20 bp, unidentified
  source 1..20: mol_type = other DNA; note = Intergene - protospacer
cttagtagtctcagaaccaa

SEQ ID NO: 306 - DNA, 20 bp, synthetic construct
  source 1..20: mol_type = other DNA; note = Intergene - forward primer
cttgctaaagggctggctct

SEQ ID NO: 307 - DNA, 20 bp, synthetic construct
  source 1..20: mol_type = other DNA; note = Intergene - reverse primer
gcccagctgattctaaggca

SEQ ID NO: 308 - DNA, 20 bp, unidentified
  source 1..20: mol_type = other DNA; note = Intergene - protospacer
gaaatatgactggaagtaaa

SEQ ID NO: 309 - DNA, 20 bp, synthetic construct
  source 1..20: mol_type = other DNA; note = Intergene - forward primer
cactctcgcttaccctgctc

SEQ ID NO: 310 - DNA, 20 bp, synthetic construct
  source 1..20: mol_type = other DNA; note = Intergene - reverse primer
acacagccaacacccctatg

SEQ ID NO: 311 - DNA, 20 bp, unidentified
  source 1..20: mol_type = other DNA; note = KLHL29 - protospacer
gagagaccgctcaggctgga

SEQ ID NO: 312 - DNA, 20 bp, synthetic construct
  source 1..20: mol_type = other DNA; note = KLHL29 - forward primer
gccgaaagcctacacctctt

SEQ ID NO: 313 - DNA, 20 bp, synthetic construct
  source 1..20: mol_type = other DNA; note = KLHL29 - reverse primer
agtgagaggagagaggctgg

SEQ ID NO: 314 - DNA, 20 bp, unidentified
  source 1..20: mol_type = other DNA; note = LOC105370393 - protospacer
gcagtacacctgagggaaca

SEQ ID NO: 315 - DNA, 20 bp, synthetic construct
  source 1..20: mol_type = other DNA; note = LOC105370393 - forward primer
tgaccagggagttcctcaca

SEQ ID NO: 316 - DNA, 20 bp, synthetic construct
  source 1..20: mol_type = other DNA; note = LOC105370393 - reverse primer
gaagccgagctcagttaccc

SEQ ID NO: 317 - DNA, 20 bp, unidentified
  source 1..20: mol_type = other DNA; note = OSBPL5 - protospacer
gcattaaggccagcgctggg

SEQ ID NO: 318 - DNA, 20 bp, synthetic construct
  source 1..20: mol_type = other DNA; note = OSBPL5 - forward primer
cagagtggccctaacctgtc

SEQ ID NO: 319 - DNA, 20 bp, synthetic construct
  source 1..20: mol_type = other DNA; note = OSBPL5 - reverse primer
cgatcctggttcctgctctg

SEQ ID NO: 320 - DNA, 20 bp, unidentified
  source 1..20: mol_type = other DNA; note = LOC105369597 - protospacer
gccatggtgaaggtgaaatc

SEQ ID NO: 321 - DNA, 20 bp, synthetic construct
  source 1..20: mol_type = other DNA; note = LOC105369597 - forward primer
actgtgctgctgagaggaac

SEQ ID NO: 322 - DNA, 20 bp, synthetic construct
  source 1..20: mol_type = other DNA; note = LOC105369597 - reverse primer
gaagcagggatgtcagtgct

SEQ ID NO: 323 - DNA, 20 bp, unidentified
  source 1..20: mol_type = other DNA; note = CCDC127 - protospacer
ggcaagggtcttgatgcatc

SEQ ID NO: 324 - DNA, 20 bp, synthetic construct
  source 1..20: mol_type = other DNA; note = CCDC127 - forward primer
caccagcttgaaggctctga

SEQ ID NO: 325 - DNA, 20 bp, synthetic construct
  source 1..20: mol_type = other DNA; note = CCDC127 - reverse primer
cctcctgggttcaagcgatt

SEQ ID NO: 326 - DNA, 20 bp, unidentified
  source 1..20: mol_type = other DNA; note = ZMYM2 - protospacer
gtaggctgctgttggacaga

SEQ ID NO: 327 - DNA, 20 bp, synthetic construct
  source 1..20: mol_type = other DNA; note = ZMYM2 - forward primer
gagctctgagttacccgaca

SEQ ID NO: 328 - DNA, 20 bp, synthetic construct
  source 1..20: mol_type = other DNA; note = ZMYM2 - reverse primer
caggcttgtgggagaaggaa

SEQ ID NO: 329 - DNA, 20 bp, unidentified
  source 1..20: mol_type = other DNA; note = Intergene - protospacer
gtcaaataaagaaaaatacg

SEQ ID NO: 330 - DNA, 20 bp, synthetic construct
  source 1..20: mol_type = other DNA; note = Intergene - forward primer
tggagagatgggatggctga

SEQ ID NO: 331 - DNA, 20 bp, synthetic construct
  source 1..20: mol_type = other DNA; note = Intergene - reverse primer
agcagagaaattgggaagca

SEQ ID NO: 332 - DNA, 20 bp, unidentified
  source 1..20: mol_type = other DNA; note = Intergene - protospacer
caaagacactcaccctgttg

SEQ ID NO: 333 - DNA, 20 bp, synthetic construct
  source 1..20: mol_type = other DNA; note = Intergene - forward primer
ggcccagaaccttgctcttt

SEQ ID NO: 334 - DNA, 20 bp, synthetic construct
  source 1..20: mol_type = other DNA; note = Intergene - reverse primer
accaccctgcgtaacatagc

SEQ ID NO: 335 - DNA, 20 bp, unidentified
  source 1..20: mol_type = other DNA; note = Intergene - protospacer
agaacacatacccctgggcc

SEQ ID NO: 336 - DNA, 20 bp, synthetic construct
  source 1..20: mol_type = other DNA; note = Intergene - forward primer
caccaccacacctggctaat

SEQ ID NO: 337 - DNA, 20 bp, synthetic construct
  source 1..20: mol_type = other DNA; note = Intergene - reverse primer
atgtccgagcaaggctttga

SEQ ID NO: 338 - DNA, 20 bp, unidentified
  source 1..20: mol_type = other DNA; note = INIP - protospacer
agagcagcgattgtaaggag

SEQ ID NO: 339 - DNA, 20 bp, synthetic construct
  source 1..20: mol_type = other DNA; note = INIP - forward primer
acagggccatcttgtgacag

SEQ ID NO: 340 - DNA, 20 bp, synthetic construct
  source 1..20: mol_type = other DNA; note = INIP - reverse primer
aagtgacgtctgcactgagg

SEQ ID NO: 341 - RNA, 10 nt, synthetic construct
  source 1..10: mol_type = other RNA; note = U-rich tail
tttttttttt

SEQ ID NO: 342 - RNA, 10 nt, synthetic construct
  source 1..10: mol_type = other RNA; note = U-rich tail
ttatttattt

SEQ ID NO: 343 - RNA, 10 nt, synthetic construct
  source 1..10: mol_type = other RNA; note = U-rich tail
tttctatttt

SEQ ID NO: 344 - RNA, 10 nt, synthetic construct
  source 1..10: mol_type = other RNA; note = U-rich tail
ttatgttttt

SEQ ID NO: 345 - protein, 557 aa, synthetic construct
  source 1..557: note = Engineered CWCas12f (Y174A)
MGEKSSRRRRNGKSGAWTAAITSCVGGKMAKNTITKTLKLRIVRPYNSAEVEKIVADEKNNREKIALEKNKDKVKEACSKHLKVAAYCTTQVERNACLFCKARKLDDKFYQKLRGQFPDAVFWQEISEIFRQLQKQAAEIYNQSLIELYYEIFIKGKGIANASSVEHYLSDVCATRAAELFKNAAIASGLRSKIKSNFRLKELKNMKSGLPTTKSDNFPIPLVKQKGGQYTGFEISNHNSDFIIKIPFGRWQVKKEIDKYRPWEKFDFEQVQKSPKPISLLLSTQRRKRNKGWSKDEGTEAEIKKVMNGDYQTSYIEVKRGSKIGEKSAWMLNLSIDVPKIDKGVDPSIIGGIDVGVKSPLVCAINNAFSRYSISDNDLFHFNKKMFARRRILLKKNRHKRAGHGAKNKLKPITILTEKSERFRKKLIERWACEIADFFIKNKVGTVQMENLESMKRKEDSYFNIRLRGFWPYAEMQNKIEFKLKQYGIEIRKVAPNNTSKTCSKCGHLNNYFNFEYRKKNKFPHFKCEKCNFKENADYNAALNISNPKLKSTKEEP

SEQ ID NO: 346 - protein, 557 aa, synthetic construct
  source 1..557: note = Engineered CWCas12f (Y174E)
MGEKSSRRRRNGKSGAWTAAITSCVGGKMAKNTITKTLKLRIVRPYNSAEVEKIVADEKNNREKIALEKNKDKVKEACSKHLKVAAYCTTQVERNACLFCKARKLDDKFYQKLRGQFPDAVFWQEISEIFRQLQKQAAEIYNQSLIELYYEIFIKGKGIANASSVEHYLSDVCETRAAELFKNAAIASGLRSKIKSNFRLKELKNMKSGLPTTKSDNFPIPLVKQKGGQYTGFEISNHNSDFIIKIPFGRWQVKKEIDKYRPWEKFDFEQVQKSPKPISLLLSTQRRKRNKGWSKDEGTEAEIKKVMNGDYQTSYIEVKRGSKIGEKSAWMLNLSIDVPKIDKGVDPSIIGGIDVGVKSPLVCAINNAFSRYSISDNDLFHFNKKMFARRRILLKKNRHKRAGHGAKNKLKPITILTEKSERFRKKLIERWACEIADFFIKNKVGTVQMENLESMKRKEDSYFNIRLRGFWPYAEMQNKIEFKLKQYGIEIRKVAPNNTSKTCSKCGHLNNYFNFEYRKKNKFPHFKCEKCNFKENADYNAALNISNPKLKSTKEEP

SEQ ID NO: 347 - protein, 557 aa, synthetic construct
  source 1..557: note = Engineered CWCas12f (Y174N)
MGEKSSRRRRNGKSGAWTAAITSCVGGKMAKNTITKTLKLRIVRPYNSAEVEKIVADEKNNREKIALEKNKDKVKEACSKHLKVAAYCTTQVERNACLFCKARKLDDKFYQKLRGQFPDAVFWQEISEIFRQLQKQAAEIYNQSLIELYYEIFIKGKGIANASSVEHYLSDVCNTRAAELFKNAAIASGLRSKIKSNFRLKELKNMKSGLPTTKSDNFPIPLVKQKGGQYTGFEISNHNSDFIIKIPFGRWQVKKEIDKYRPWEKFDFEQVQKSPKPISLLLSTQRRKRNKGWSKDEGTEAEIKKVMNGDYQTSYIEVKRGSKIGEKSAWMLNLSIDVPKIDKGVDPSIIGGIDVGVKSPLVCAINNAFSRYSISDNDLFHFNKKMFARRRILLKKNRHKRAGHGAKNKLKPITILTEKSERFRKKLIERWACEIADFFIKNKVGTVQMENLESMKRKEDSYFNIRLRGFWPYAEMQNKIEFKLKQYGIEIRKVAPNNTSKTCSKCGHLNNYFNFEYRKKNKFPHFKCEKCNFKENADYNAALNISNPKLKSTKEEP

SEQ ID NO: 348 - protein, 557 aa, synthetic construct
  source 1..557: note = Engineered CWCas12f (Y174R)
MGEKSSRRRRNGKSGAWTAAITSCVGGKMAKNTITKTLKLRIVRPYNSAEVEKIVADEKNNREKIALEKNKDKVKEACSKHLKVAAYCTTQVERNACLFCKARKLDDKFYQKLRGQFPDAVFWQEISEIFRQLQKQAAEIYNQSLIELYYEIFIKGKGIANASSVEHYLSDVCRTRAAELFKNAAIASGLRSKIKSNFRLKELKNMKSGLPTTKSDNFPIPLVKQKGGQYTGFEISNHNSDFIIKIPFGRWQVKKEIDKYRPWEKFDFEQVQKSPKPISLLLSTQRRKRNKGWSKDEGTEAEIKKVMNGDYQTSYIEVKRGSKIGEKSAWMLNLSIDVPKIDKGVDPSIIGGIDVGVKSPLVCAINNAFSRYSISDNDLFHFNKKMFARRRILLKKNRHKRAGHGAKNKLKPITILTEKSERFRKKLIERWACEIADFFIKNKVGTVQMENLESMKRKEDSYFNIRLRGFWPYAEMQNKIEFKLKQYGIEIRKVAPNNTSKTCSKCGHLNNYFNFEYRKKNKFPHFKCEKCNFKENADYNAALNISNPKLKSTKEEP

SEQ ID NO: 349 - protein, 557 aa, synthetic construct
  source 1..557: note = Engineered CWCas12f (A184T)
MGEKSSRRRRNGKSGAWTAAITSCVGGKMAKNTITKTLKLRIVRPYNSAEVEKIVADEKNNREKIALEKNKDKVKEACSKHLKVAAYCTTQVERNACLFCKARKLDDKFYQKLRGQFPDAVFWQEISEIFRQLQKQAAEIYNQSLIELYYEIFIKGKGIANASSVEHYLSDVCYTRAAELFKNTAIASGLRSKIKSNFRLKELKNMKSGLPTTKSDNFPIPLVKQKGGQYTGFEISNHNSDFIIKIPFGRWQVKKEIDKYRPWEKFDFEQVQKSPKPISLLLSTQRRKRNKGWSKDEGTEAEIKKVMNGDYQTSYIEVKRGSKIGEKSAWMLNLSIDVPKIDKGVDPSIIGGIDVGVKSPLVCAINNAFSRYSISDNDLFHFNKKMFARRRILLKKNRHKRAGHGAKNKLKPITILTEKSERFRKKLIERWACEIADFFIKNKVGTVQMENLESMKRKEDSYFNIRLRGFWPYAEMQNKIEFKLKQYGIEIRKVAPNNTSKTCSKCGHLNNYFNFEYRKKNKFPHFKCEKCNFKENADYNAALNISNPKLKSTKEEP

SEQ ID NO: 350 - protein, 557 aa, synthetic construct
  source 1..557: note = Engineered CWCas12f (S188G)
MGEKSSRRRRNGKSGAWTAAITSCVGGKMAKNTITKTLKLRIVRPYNSAEVEKIVADEKNNREKIALEKNKDKVKEACSKHLKVAAYCTTQVERNACLFCKARKLDDKFYQKLRGQFPDAVFWQEISEIFRQLQKQAAEIYNQSLIELYYEIFIKGKGIANASSVEHYLSDVCYTRAAELFKNAAIAGGLRSKIKSNFRLKELKNMKSGLPTTKSDNFPIPLVKQKGGQYTGFEISNHNSDFIIKIPFGRWQVKKEIDKYRPWEKFDFEQVQKSPKPISLLLSTQRRKRNKGWSKDEGTEAEIKKVMNGDYQTSYIEVKRGSKIGEKSAWMLNLSIDVPKIDKGVDPSIIGGIDVGVKSPLVCAINNAFSRYSISDNDLFHFNKKMFARRRILLKKNRHKRAGHGAKNKLKPITILTEKSERFRKKLIERWACEIADFFIKNKVGTVQMENLESMKRKEDSYFNIRLRGFWPYAEMQNKIEFKLKQYGIEIRKVAPNNTSKTCSKCGHLNNYFNFEYRKKNKFPHFKCEKCNFKENADYNAALNISNPKLKSTKEEP

SEQ ID NO: 351 - protein, 557 aa, synthetic construct; identical to SEQ ID NO: 1
  source 1..557: note = Engineered CWCas12f (S188S)

SEQ ID NO: 352 - protein, 557 aa, synthetic construct
  source 1..557: note = Engineered CWCas12f (S188T)
MGEKSSRRRRNGKSGAWTAAITSCVGGKMAKNTITKTLKLRIVRPYNSAEVEKIVADEKNNREKIALEKNKDKVKEACSKHLKVAAYCTTQVERNACLFCKARKLDDKFYQKLRGQFPDAVFWQEISEIFRQLQKQAAEIYNQSLIELYYEIFIKGKGIANASSVEHYLSDVCYTRAAELFKNAAIATGLRSKIKSNFRLKELKNMKSGLPTTKSDNFPIPLVKQKGGQYTGFEISNHNSDFIIKIPFGRWQVKKEIDKYRPWEKFDFEQVQKSPKPISLLLSTQRRKRNKGWSKDEGTEAEIKKVMNGDYQTSYIEVKRGSKIGEKSAWMLNLSIDVPKIDKGVDPSIIGGIDVGVKSPLVCAINNAFSRYSISDNDLFHFNKKMFARRRILLKKNRHKRAGHGAKNKLKPITILTEKSERFRKKLIERWACEIADFFIKNKVGTVQMENLESMKRKEDSYFNIRLRGFWPYAEMQNKIEFKLKQYGIEIRKVAPNNTSKTCSKCGHLNNYFNFEYRKKNKFPHFKCEKCNFKENADYNAALNISNPKLKSTKEEP

SEQ ID NO: 353 - protein, 557 aa, synthetic construct
  source 1..557: note = Engineered CWCas12f (S188V)
MGEKSSRRRRNGKSGAWTAAITSCVGGKMAKNTITKTLKLRIVRPYNSAEVEKIVADEKNNREKIALEKNKDKVKEACSKHLKVAAYCTTQVERNACLFCKARKLDDKFYQKLRGQFPDAVFWQEISEIFRQLQKQAAEIYNQSLIELYYEIFIKGKGIANASSVEHYLSDVCYTRAAELFKNAAIAVGLRSKIKSNFRLKELKNMKSGLPTTKSDNFPIPLVKQKGGQYTGFEISNHNSDFIIKIPFGRWQVKKEIDKYRPWEKFDFEQVQKSPKPISLLLSTQRRKRNKGWSKDEGTEAEIKKVMNGDYQTSYIEVKRGSKIGEKSAWMLNLSIDVPKIDKGVDPSIIGGIDVGVKSPLVCAINNAFSRYSISDNDLFHFNKKMFARRRILLKKNRHKRAGHGAKNKLKPITILTEKSERFRKKLIERWACEIADFFIKNKVGTVQMENLESMKRKEDSYFNIRLRGFWPYAEMQNKIEFKLKQYGIEIRKVAPNNTSKTCSKCGHLNNYFNFEYRKKNKFPHFKCEKCNFKENADYNAALNISNPKLKSTKEEP

SEQ ID NO: 354 - protein, 557 aa, synthetic construct
  source 1..557: note = Engineered CWCas12f (R191G)
MGEKSSRRRRNGKSGAWTAAITSCVGGKMAKNTITKTLKLRIVRPYNSAEVEKIVADEKNNREKIALEKNKDKVKEACSKHLKVAAYCTTQVERNACLFCKARKLDDKFYQKLRGQFPDAVFWQEISEIFRQLQKQAAEIYNQSLIELYYEIFIKGKGIANASSVEHYLSDVCYTRAAELFKNAAIASGLGSKIKSNFRLKELKNMKSGLPTTKSDNFPIPLVKQKGGQYTGFEISNHNSDFIIKIPFGRWQVKKEIDKYRPWEKFDFEQVQKSPKPISLLLSTQRRKRNKGWSKDEGTEAEIKKVMNGDYQTSYIEVKRGSKIGEKSAWMLNLSIDVPKIDKGVDPSIIGGIDVGVKSPLVCAINNAFSRYSISDNDLFHFNKKMFARRRILLKKNRHKRAGHGAKNKLKPITILTEKSERFRKKLIERWACEIADFFIKNKVGTVQMENLESMKRKEDSYFNIRLRGFWPYAEMQNKIEFKLKQYGIEIRKVAPNNTSKTCSKCGHLNNYFNFEYRKKNKFPHFKCEKCNFKENADYNAALNISNPKLKSTKEEP

SEQ ID NO: 355 - protein, 557 aa, synthetic construct
  source 1..557: note = Engineered CWCas12f (R191H)
MGEKSSRRRRNGKSGAWTAAITSCVGGKMAKNTITKTLKLRIVRPYNSAEVEKIVADEKNNREKIALEKNKDKVKEACSKHLKVAAYCTTQVERNACLFCKARKLDDKFYQKLRGQFPDAVFWQEISEIFRQLQKQAAEIYNQSLIELYYEIFIKGKGIANASSVEHYLSDVCYTRAAELFKNAAIASGLHSKIKSNFRLKELKNMKSGLPTTKSDNFPIPLVKQKGGQYTGFEISNHNSDFIIKIPFGRWQVKKEIDKYRPWEKFDFEQVQKSPKPISLLLSTQRRKRNKGWSKDEGTEAEIKKVMNGDYQTSYIEVKRGSKIGEKSAWMLNLSIDVPKIDKGVDPSIIGGIDVGVKSPLVCAINNAFSRYSISDNDLFHFNKKMFARRRILLKKNRHKRAGHGAKNKLKPITILTEKSERFRKKLIERWACEIADFFIKNKVGTVQMENLESMKRKEDSYFNIRLRGFWPYAEMQNKIEFKLKQYGIEIRKVAPNNTSKTCSKCGHLNNYFNFEYRKKNKFPHFKCEKCNFKENADYNAALNISNPKLKSTKEEP

SEQ ID NO: 356 - protein, 557 aa, synthetic construct
  source 1..557: note = Engineered CWCas12f (Y230A)
MGEKSSRRRRNGKSGAWTAAITSCVGGKMAKNTITKTLKLRIVRPYNSAEVEKIVADEKNNREKIALEKNKDKVKEACSKHLKVAAYCTTQVERNACLFCKARKLDDKFYQKLRGQFPDAVFWQEISEIFRQLQKQAAEIYNQSLIELYYEIFIKGKGIANASSVEHYLSDVCYTRAAELFKNAAIASGLRSKIKSNFRLKELKNMKSGLPTTKSDNFPIPLVKQKGGQATGFEISNHNSDFIIKIPFGRWQVKKEIDKYRPWEKFDFEQVQKSPKPISLLLSTQRRKRNKGWSKDEGTEAEIKKVMNGDYQTSYIEVKRGSKIGEKSAWMLNLSIDVPKIDKGVDPSIIGGIDVGVKSPLVCAINNAFSRYSISDNDLFHFNKKMFARRRILLKKNRHKRAGHGAKNKLKPITILTEKSERFRKKLIERWACEIADFFIKNKVGTVQMENLESMKRKEDSYFNIRLRGFWPYAEMQNKIEFKLKQYGIEIRKVAPNNTSKTCSKCGHLNNYFNFEYRKKNKFPHFKCEKCNFKENADYNAALNISNPKLKSTKEEP

SEQ ID NO: 357 - protein, 557 aa, synthetic construct
  source 1..557: note = Engineered CWCas12f (Y230I)
MGEKSSRRRRNGKSGAWTAAITSCVGGKMAKNTITKTLKLRIVRPYNSAEVEKIVADEKNNREKIALEKNKDKVKEACSKHLKVAAYCTTQVERNACLFCKARKLDDKFYQKLRGQFPDAVFWQEISEIFRQLQKQAAEIYNQSLIELYYEIFIKGKGIANASSVEHYLSDVCYTRAAELFKNAAIASGLRSKIKSNFRLKELKNMKSGLPTTKSDNFPIPLVKQKGGQITGFEISNHNSDFIIKIPFGRWQVKKEIDKYRPWEKFDFEQVQKSPKPISLLLSTQRRKRNKGWSKDEGTEAEIKKVMNGDYQTSYIEVKRGSKIGEKSAWMLNLSIDVPKIDKGVDPSIIGGIDVGVKSPLVCAINNAFSRYSISDNDLFHFNKKMFARRRILLKKNRHKRAGHGAKNKLKPITILTEKSERFRKKLIERWACEIADFFIKNKVGTVQMENLESMKRKEDSYFNIRLRGFWPYAEMQNKIEFKLKQYGIEIRKVAPNNTSKTCSKCGHLNNYFNFEYRKKNKFPHFKCEKCNFKENADYNAALNISNPKLKSTKEEP